European Patent Specification EP 3 423 563 B1, published May 24, 2023. Title: IMPROVED MUCONIC ACID PRODUCTION FROM GENETICALLY ENGINEERED MICROORGANISMS. Applicant: Myriant Corporation Sillers, Ryan Spencer, Michelle Yocum, R. Rogers Hermann, Theron. The sequence listing filed with the application follows.

SEQUENCE LISTING (94 sequences)

SEQ ID NO: 1 - DNA, 195 bp, Bacillus subtilis
  promoter (1)..(195): The P15 promoter from Bacillus subtilis phage SP01, with a stem and loop added just downstream from the transcription start site.
gctattgacgacagctatggttcactgtccaccaaccaaaactgtgctcagtaccgccaatatttctcccttgaggggtacaaagaggtgtccctagaagagatccacgctgtgtaaaaattttacaaaaaggtattgactttccctacagggtgtgtaataatttaattacaggcgggggcaaccccgcctgtt

SEQ ID NO: 2 - DNA, 164 bp, Bacillus subtilis
  promoter (1)..(164): The P26 promoter from Bacillus subtilis phage SP01
gcctacctagcttccaagaaagatatcctaacagcacaagagcggaaagatgttttgttctacatccagaacaacctctgctaaaattcctgaaaaattttgcaaaaagttgttgactttatctacaaggtgtggtataataatcttaacaacagcaggacgct

SEQ ID NO: 3 - DNA, 91 bp, Escherichia coli
  promoter (1)..(91): The PR promoter from Escherichia coli phage
acgttaaatctatcaccgcaagggataaatatctaacaccgtgcgtgttgactattttacctctggcggtgataatggttgcatgtacaag

SEQ ID NO: 4 - protein, 359 aa, Neurospora crassa
  PEPTIDE (1)..(359): Protein sequence of  3-dehydroshikimate dehydratase from Neurospora crassa encoded by the qa-4 gene.
MPSKLAISSMSLGRCFAGHSLDSKLDAAQRYGYLGIELFYEDLVDVAEHLSNERPSPEGPFVEAQIAAARHILQMCQARGLEVVCLQPFMHYDGLNDRAEHERRLEKLALWIELAHELHTDIIQIPANFLPANQVSDNLDLIVSDLCKVADIGAQALPPIRFAYESLCWSTRVDLWERCWDIVQRVDRPNFGICLDTFNILGRIYADPTSPSGRTPNAKEAVRKSIANLVSRVDVSKVFYVQVVDAERLSKPLLPGHPYYNPEQPARMSWSRNCRLFYGETEYGAYLPVKEVARALFHGIGFEGWVSLELFNRRMSEEGPEVPEELAMRGAISWAKLVQDLRIPVEGPLVTMPRVSASL

SEQ ID NO: 5 - DNA, 2160 bp, Neurospora crassa
  gene (1)..(2160): Genomic DNA sequence of the qa-4 gene from Neurospora crassa plus surrounding sequences.
gaattcgggaaatggaatcttacctgggaaccgaaatcacagtccgggtaggttatagagcatatagtgaactgtcaaagttctagacctggaccagccacttggagtcgttgttttagttatacctacattcactcactgttgactttcaatcatacttacttagacggagcaacgcgccagaatccaaattgttgcatagttgcggtatcaccaagtggcttcccataatagtttgccattcgatgagacagctaactggaagaccggtactcgcaggttgcacgattacacggaaggattcggtattccgtgtttcatctgtcaaagtccctttccatatgaatccgaggtactatgactggatctcgatacaagctggccagcgaggtgcctgccttgacaggctgtcaactgcgggacggccggctaagtgtttaacacgcaagggtggaagatgtctcgtcccgtcatccaagaccgtcaacattcgaggccatctgatcgttgaagagatgctaaatcttgtgaaacgctcataggtcgcttaccttcggcccacccgttaatgctttattccgctgagcaaacttcggcttccatcccgcggttcaccgtttacatcacttatcgttgcggttattggccgattcttcgcaaaccgaaacgatgacatcccgaatatctgcaatacaccgccacggccggcgtctttatcacacctcctatgggagacgaaagtgccttgatacccctagtcatttgaagattcaggatgggagacggctggccgcttgcggagttacgttcgagtcttggtcgcaggaacgcttgccgtattgaatgagaccccgagaaggtcaaatcaaatcttggaagaccccaactgcttcctcattgccttcactccccatatcaatggggcacatcctgtgactaccttggtgctttatttcctcaccatttggcgatacaagctcaaggacaccgaggtgatatacagttcttcaaggacactatctcacctcaatatcaagaaccagtctcatcatctcttatttctccaggatccccccaccaacaacatcggcttttttttttcccctattctcaagacccatcaagacgctcacttcgctgagcctttcgccatgccgtcaaagctagccattagttccatgtccctagggcgctgctttgccggccactctctggacagcaagcttgatgccgctcaacgatacggctatcttggtatcgagcttttttatgaggatctggtcgacgttgcagagcatttgtcgaacgagcgtccctctcccgaaggcccttttgtcgaagctcagatagccgccgctcgtcatattctccagatgtgtcaagccagggggcttgaggtcgtctgcctccagcctttcatgcactacgacggccttaacgacagggcagaacatgagcgtcgtctggagaagctagcactatggattgagctcgctcatgagcttcacaccgacatcattcagatcccagccaacttcctccctgccaaccaagtcagtgacaacctcgacctgattgtctcagatctttgcaaggtggccgatattggagctcaagctttgccccctatccgctttgcctacgagagtctttgctggagcacccgtgtcgacctctgggagcgctgctgggacatcgtacaacgcgttgaccgccccaactttggcatttgccttgacaccttcaacatcctcggccgcatctatgccgaccctacatctcctagcggtaggacacccaacgcaaaagaggcagtcaggaagtccatcgccaacttggtctcgcgcgtggatgtctccaaagtcttctacgtccaggtggttgacgccgagaggctgagcaagccactactgcccggtcacccgtattacaatccagagcagccggcgaggatgagctggtcgcgcaattgtagactgttctacggcgaaacagaatatggtgcgtatcttcccgtgaaggaggttgctcgagcccttttccacggcattggtttcgagggctgggtcagtttggagcttttcaaccgcagaatgtctgaggagggacctgaagtgccggaggaacttgccatgagaggcgctatctcgtgggccaagt

SEQ ID NO: 6 - protein, 348 aa, Aspergillus niger
  PEPTIDE (1)..(340): Protein sequence of 3dehydroshikimate dehydratase from Aspergillus nidulans. encoded by the qutC gene
MPANLKIGIPTVSLSKPGLHSLDHKLRSAAHGFAGIELFIDDLSHFASSSFNGSLTQAAKYISSLAKQLNLTFICLQPFGFYEGLVDTNQSTYLLTEKLPLWFAIARIIGTDLIQIPANFLQNDPVTGAARTSGDIRLIVSDLQTIADIGVKQGFRFVYEALCWSTHVDTWEAAWNVVKLVDRENFGICLDSFNTRTPLPSLGRRRMLSKPWPSPWRRSVLSSPVENWTSGKSSTSSLSMASGCRRRWTRSTPFMWRANPRRMSWSRNARLFPCEEERGGYLPVLEIARAFFEIGFEGWVSLELFSRTCNDPDVNTVGEHARRGMDRRRRVVAALGLDVEVPARNCEC

SEQ ID NO: 7 - DNA, 3298 bp, Aspergillus niger
  gene (1)..(3298): Genomic DNA sequence of the qutC gene from Aspergillus nidulans plus surrounding sequences
aagcttggtttcaagtgatgatatatagttatgaggatataatatgaaccgaaagacgatgtttcttgtgaatatttacgtgatagttgtctgtctaatatggtacagcagtagaacaactacatacggtcactacttacagccctagtcattccctccctcgattgcctaccatttatacactttgaacatccacaggcttgcctccctccatactctccctaacagcttgaacaactctgagcgccctcaccccatcttcaacgccacagccaactcctcgctcgccatcctcaccctttccactaacaacatcaacaaaatatccccactgcgcatcaaacggcctcacatcagcatccttcactgaaatctgctgcatcgccaactccgtattccagcctttctctttcccctgtccacaagaaacatggtcatagctccagcgcgtcatatcaggcacactgagactcgctctggttccaagaattcgataacagtcgcttgcactcttggaaggagcgggcggaatcgtaggattctcgcccgttcctgtttcaaagttcaacggcgaaggcgtcgcgtcgcagatgagaaatgtgcctactatcccagacgcaaagcgcagcgtcacagcacagccttcctcggcggtatgttccgggttctggcgcatgcgctgcaggagtgtaccctccgcgtagaccctactgacgggcccaaacagaaactgcagcacgtcgatatcgtggataagattaatccccagcacgccgcccttcttcttatctgcgcgccaagaaccgagcggcggcgcgaagtaagaggccggcttcagaagtgtccagaggccgttcactgcaacgacggtgccgagtgagtctgtctctaacaaagactttgtggtttggatgtacggattgaagcggcggtggtggccgatctggatgttgatcttcgcatccttgcctctcttctcatctttacatttctgttccttgacggtagcgaggaggtgctcggccgactccagatcgtcactgatcggtttctcaaggaggatattgcggattccgttctccagcagctggagcgtgacgtccacgtgcgtgtgattgggcgtgctcacgatcgccgcgtctggtttcccggttgtcttaccgacaacgtctaacatagacgtaatagaatcatagcaaggaacgccaaatgattctgcgaccgggattgcagagggtgaagggtcaacaaaagcgatcagctgggttcgtgggtgtcgttgcacggattgtgcgtgacggggcccaataagtccggcaccgacgatgacaatgaggatattcttgtccttttccttgctgcagggcaccattgtgcatgtcggtggctggaaataaacagaacagggatatggtcaagtcggagaatcggtgcaggatagaccggctacttgatgtaggacgacagtcgcgatctaccgagagcgtgagattcactgtgggactgatttatgtaatttgaggcgcagcagacttagggacttgaaatgtggctgtctgtggatgcatttgcggggtatggagtacagagtgcatacagctgtgtatatggagttccttacggagagggtgacctggtatggggagaacgggcaaaatgctcacccggcaacctctcaaagcgtttacccggtatactcctctgatatcaatatttccaatcagcacctatatcatcacgacgctctcctgaggattccgtagctaaccgccctggatcctacattaataaataagccatttgctttttctgctgcgagtgtgattctcaatacgattacgtatcacatgcagattgcctttacttcagctgcatttgatcagccacagctctaagagcaaacataccctacctacctacctacttcgcctagggtacataatcaccgccatctcctcctcgatcagtcttcaactcaatcagctcattcattctattcttaatataatatatacctttagatctccagcagagacccgaagagtcggcaattcaaaatgcccgcaaacctcaaaatcggtatcccaaccgtgtccctgtcaaaaccgggcctgcactctcttgaccataagctccgctcggccgctcatggcttcgcggggatcgagctgtttattgatgacctctcccatttcgcctcatcgtcattcaatggctccctcactcaagcggcaaagtatatctcctcgctcgccaagcaacttaacctcacatttatctgcctgcaaccattcggtttctacgagggtctggtggacacaaatcagtcgacgtacctgctcactgagaaactcccgctctggtttgcgatcgcccgcattataggcacagatctcatccaaatccccgcaaatttcctccagaatgaccctgtcaccggggctgcacgaacaagcggcgacataaggcttatcgtctcagatctgcagacgatcgcagatatcggtgtaaagcagggcttccgctttgtgtacgaggcgctctgctggtcgacgcatgtcgatacatgggaagcagcgtggaatgtcgtcaagctggttgatagagagaatttcgggatctgcctggatagcttcaacacgcggaccccgcttccgtcactgggaagacgccggatgctgagcaagccgtggccaagtccatggagacgctccgttctctcgtctccagtggagaactggacatcaggaaaatcttctacatccagcttgtcgatggcgagcggttgtcggcgccgctggacgagaagcacccctttcatgtggagggccaacccccgaagaatgagctggagtcgcaatgcgcggttattcccctgtgaagaggagaggggtgggtatcttcctgtgttggagatcgcgagggcgttctttgaaatcgggttcgaggggtgggtgagtctagagctgttttcaaggacgtgtaatgatcccgatgtgaacacggtgggggagcatgcgagacgtgggatggatagaaggaggagggttgttgcggcgctaggactcgatgttgaggtgccagcacgtaactgtgaatgttagcatgaacggcaaggagagggtggaggtgcaggtgcaggaggagctggctgttcagcatcggctgtaggtagtggtatcttgaaaggacgatagggtttgatctagagatttttattttgtctaattactggtaatgatggcctcatgcacgctgttgaacacgctgtacaacatcactgttgaagatgatacct

SEQ ID NO: 8 - protein, 502 aa, Klebsiella pneumoniae
  PEPTIDE (1)..(502): Protein sequence of protocatechuate decarboxylase (AroY) from Klebsiella pnemoniae ATCC25597
MTAPIQDLRDAIALLQQHDNQYLETDHPVDPNAELAGVYRHIGAGGTVKRPTRIGPAMMFNNIKGYPHSRILVGMHASRQRAALLLGCEASQLALEVGKAVKKPVAPVVVPASSAPCQEQIFLADDPDFDLRTLLPAHTNTPIDAGPFFCLGLALASDPVDASLTDVTIHRLCVQGRDELSMFLAAGRHIEVFRQKAEAAGKPLPITINMGLDPAIYIGACFEAPTTPFGYNELGVAGALRQRPVELVQGVSVPEKAIARAEIVIEGELLPGVRVREDQHTNSGHAMPEFPGYCGGANPSLPVIKVKAVTMRNNAILQTLVGPGEEHTTLAGLPTEASIWNAVEAAIPGFLQNVYAHTAGGGKFLGILQVKKRQPADEGRQGQAALLALATYSELKNIILVDEDVDIFDSDDILWAMTTRMQGDVSITTIPGIRGHQLDPSQTPEYSPSIRGNGISCKTIFDCTVPWALKSHFERAPFADVDPRPFAPEYFARLEKNQGSAK

SEQ ID NO: 9 - DNA, 5502 bp, Klebsiella pneumoniae
  gene (1)..(5502): DNA sequence of the aroY gene of Klebsiella pneumoniae 342 plus 2 kilobases of surrounding DNA sequences
gcgacgccgactgggcgatccgtgaactgctggcgcgtatgacccagcgtctgcagggctgtgaaaccatagaggatgtgattaaggtggcggagctgttcgcgccgaacatcgccccgacgatccccggtaaactgtatattctggataccgatccatggcagatgcgctgcgtggcgcagtggctgtcgcccgccggggagacgacgtcctttgctcccgacgactgctgggcgatacggcggggactcagccatccgccggtgcagggtgagcccgatatcacctgctatcatctgccggaggcgcacgccggccagtcgctctgcgtaccgctcatcgcccagggcgaagcgatcggtctgctgagctttcagaacgtcaccgccagtgacgccccttcccgggcttacctggagctgatggccgaagcgctggggctggcgctcgccaatcagcgtttacgcagcgccctgctggaaaaagcgttgttcgattcgctgaccggcctgcgtaaccgccatcatcttgatgaagcgctgcactcgcagatggcgctggcggtccatacccacaccccgctgagctgcctgatgatcgacatcgatcacttcaaagccatcaatgaccgctacggccatgaagccggggatctggtgattaagagcgtcgcgaccattgtgcagcgcgcggtgcgcgatatcggcatggctttccgctacggcggcgaggagtttttagtgctgctccccgggattgacgaagccggggcgcaccagtgcgccagcgagatctacacccaggtgcacaatatgacgctgcgcgatggcctgacggagataggccaggtggatgtgtcgattggcatcgccagctacccgcagcacacccaaagcgacagcctgctgcgcgcagcggacgccgcgctgtaccgggcgaaagagctgggccgttcaaggattgtcagctttggccgcctgaagacccgctaagcgggattattgctcagcggcattaagcagcgagataactttccgcaccaccgccgaacggaaatggcggtggtaaaccatgctcagctcactctccgccagccgatcctgaagatcgatatacaccacgttatcaaggcgtaaggccctcgccgagaccggcaccagcgccacccccaccccggcggagaccaggctaatcatcgaggtgacatcgttaattcgctgcaccacctgcggcgtaaaacccgcgacgcgacaggcgtcaataaatacctgctccagtccggtgccctgcggatcgtcaagcgagatccagttgtcagtgcgcaacgaggccagattgagcgcccccacgcctgccagcggatgctgttgataaagcgccaggcaaagtttttcccgcacaaatggcctgaccaccagcgcgtccggcggtgacgccagcggcgcgcggatgatggcgatatccagacgcagatccagcagcgcttcgtagagcatttgcacatccccctgcaccagcgacagctcaatccccggccagtcagcgcgcagctcgcgcaggagccccggcagtttgctgtcatacatcgcactggagacatagcccagatgcaatcgcccctgctcgcctcgtgcggtgcgctgggcgtccaggaccgcctgatcggccatctccagcgccagccgcgtcttctgcaagaaggcctcgcccgcggcggtgagggtcaggcgccggttagcgcgggagaagagcaccacgcccaggcgctgctcgagttgtttaatctgctggctgagggcgggctgggcgatatgtaaccgctctgccgcccgatgcatatgtagttcttcagcaacgaccacaaaatggcgtaacgctcgcaaggacatggccggactccgcggagtaaattgataataaaaatgttatcaataaagcatgaatgatgcaattgataaccattagcctgcgagcatactgtgcgcatcgacacgctaaggagaacatcatgaccgcaccgattcaggatctgcgcgacgctatcgcgctgctgcaacagcatgacaatcagtacctcgaaaccgatcatccggttgaccctaacgctgagctggccggcgtctatcgccacatcggcgcgggcggcaccgtgaagcgccccacgcgcatcggcccggcgatgatgtttaacaatattaagggctatccgcactcgcgcattctggtgggcatgcacgccagccgccagcgggccgcgctgctgctgggctgcgaagcctcacagctggcgctggaggtaggcaaagcggtgaaaaaaccggtcgcgccggtggtcgttccggccagcagcgccccctgtcaggaacaggtctttctggccgacgatccggattttgatttgcgcaccctgctcccggcgcccaccaacaccccgatcgacgccggtcccttcttctgcctgggcctggcgctggccagcgatcccgacgacgcctcgctcaccgacgtcaccatccaccgcttgtgcgtccagggccgggatgagctgtcgatgtttctcgccgctggccgccatatcgaagtgtttcgtcagaaagccgaggccgctggcaaaccgctgccgataaccatcaatatgggactcgatccggctatctatatcggcgcctgctttgaagcgccgaccacacgtttggctataacgaactgggcgtcgccggtgcgctgcgtcagcgtccggtagagctggtacagggcgtcagcgtcccggagaaagccatcgctcgcgccgagatcgttatcgaaggggaactgctgccgggggtacgcgtcagagaagatcagcacacaacagcggccatgcgatgccggaatttcctggttactgcggcggcgccaatccgtcgctgccggtcattaaagtcaaagcggtgaccatgcgaaacaatgcgattctgcagacgctggtagggccgggcgaagagcataccaccctcgccggattgccaacggaagccagtatctggaatgctgtcgaggctgctatcccgggctttttacaaaatgtctacgcccacaccgcgggcggcggtaaattcctcgggatcctgcaggtgaaaaaacgccagcccgccgacgaagggcgtcaggggcaggccgcgttgctggcgctggcgacctattccgagctgaaaaatatcattctggtcgatgaagatgtcgatatctttgacagcgacgatatcctgtgggccatgaccacccgcatgcagggggatgtcagcatcacgacgatcccaggcattcgtggtcaccagctggatccttcccagaccccggcctacagcccgtcgatccgcggagagggtatcagttgcaagacgattttcgattgcacggtgccgtgggcgctaaaatcacacttcgagcgcgcaccgtttgccgatgtcgatccgcgtccgtttgcgccggagtattttgcccggctggaaaaaaaccacggtcagtaaaatcaggtgatagccgccggagcacggcggcatcttccgggccagcatcacctgcagcgggtggctgacgcagggttagttgatcgcggcggagaggtcttttttcacctgctcacgctgctcgggggtcaacacctggctcacgtcgaagtagtatttcacacgataataccgcacctgctggtccagctggccaaaggcggccagctgctgtttgaccttagcgtcatcccatttcccggagtgaataacgtctgccagggcaccatcctgatagccgctgatttaatctggcttacattgttttcgaatccctgacgcagcgcctggattttggcgacctgctcttcactcagcttcaggtgctggacgaccggatcctgcgagacagacggtatatcggcggaggtcgacgcctggctggctgccgtaaagcaggtggtcagcgcaatggcgagcagggtgttacgcaagcgagtattcacagtgaatgatccttcaaaaaagaaaatgagaggcgattatcactgcgctaataaagactatctgtaacaaagggttaatttaaaactggataaaaaaaggatggtaagaaacagaaatcagatcccgggtcagcagcacagaaagatatattcatccttccagtaacggccctgtccaatgatatccccggcggcgctgattaactgtttttgcttttggtttcaatcccctcaacgatcacatggctggtcagggtatgaatagattgcaacagcccgggaaaagcggggtcgttttctttatcccagaagtaatctttatccactttgacgcaatcgaagcggaagcgctccagcagcgggaaggacgtcgtccgcggccaaaatcatccagccagaccgggcaaagcgccgccagcgtgctcagcgccgtcagctcacgtccggcgataaactcgtgaaagttctcatttatttccagagcaatgtgtttacaggagcgcaggaaatcacagagatagcgatccgtcagaataaagtggcttaataaatcatcaatattcagcgatatcggtttattatcgacccgggcgaaatcaaatacagaaagtaactcgatttgccgaataaatagagcaagcttatcgcgttcggtaagcgtggagaaagaaaacgtcgacgcagaggtggtattttgtgcgggtgctataatatctttagtaagcaactcccacgagtggtagctgccgtcatcgctaatagcgggctccagaacgaagcgataagaggtatttttcacgttttcttcaaccatttaaaaaataccaaaaataagaaagggttaagcatgtcatatattttccgccaacaaaaatagtttaaagtgatcgataataatcattcgatagttaaaaactatcaagatataatttattgatcggtaaattgaattaatataaattagccactgccgtaactccctctgaaaagtcaattaaaatattgtttcaaaccagccagttaccagagtattctgcgtaaagcctggtcgtctcacgctttgtgctgccaggtaaaaaaagagaggggtaataaaaatgaaaaatacaagccgccagttttagtcatatcattatgccgaatatgaataacgctgcgctgaggcgccgcttcgcctggcatgccatgagtcctcaacaaaaaagtgtgactcagtcgacaaaacgtcatattttcccgctatcctgcagcgaagaagagtgaagtggatgacaggcagtgaaaaaaataaacgtgattccgctggggctgatgctattcatgctcatcgccagcgcatggctgggccctgcgccgcggcacaccggcagcatgcagtgcgtttggtttgacggggcaatggtgagctgcctgccgaagcaacgactgggcgaaggctcgccgcatcatttactggtcagacgataaaccggtactcgccgggtggtgttgaacagattatcgctggc

SEQ ID NO: 10 - DNA, 4629 bp, Acinetobacter baylyi
  gene (1)..(4629): DNA sequence of the catA gene from Acinetobacter baylyi ADP1, including 410 bases of upstream sequence and two open reading frames downstream
atctgctcgaccatagtaatgatcacattatgagctaaatttactttttaaaatttaaatatattatatatatttgaattttattgttttattttaatttttagcttagaagtttttattaagatttatttttaaattagatgtcgaaaaaattagtataccaaaaaagcatgaaaacatactctcttaggaattggagtcgccatgagtttcagatacagttgatcagtatggaaggtatagaaacgactatcgaaataaataagtttgtggtgtgtgaagcaaggtaaagctcaaggctgaggcaaaccaagcaaaggttaattgaaccgatatgcacaacacattcaacgatagcgtcgacagataagtttatcaaatgatgttttggcgatttcaaggagaaagccatggaagttaaaatattcaatactcaggatgtgcaagattttttacgtgttgcaagcggacttgagcaagaaggtggcaatccgcgtgtaaagcagatcatccatcgtgtgctttcagatttatataaagccattgaagatttgaatatcacttcagatgaatactgggcaggtgtggcatatttaaatcagctaggtgccaatcaagaagctggtttactctcgccaggcttgggttttgaccattacctcgatatgcgtatggatgccgaagatgccgcactaggtattgaaaatgcgacaccacgtaccattgaaggcccgctatacgtggcaggtgcgcctgaatcggtaggttatgcgcgcatggatgacggaagtgatccaaatggtcataccctgattctacatggcacgatctttgatgcagatggaaaacctttacccaatgccaaagttgaaatctggcatgccaataccaaaggcttttattcacacttcgacccaacaggcgagcagcaggcgttcaatatgcgccgtagtattattaccgatgaaaacggtcagtatcgcgttcgtaccattttgcctgcgggttatggttgcccaccagaaggtccaacgcaacagttgctgaatcagttgggccgtcatggtaaccgccctgcgcacattcactattttgtttctgccgatggacaccgcaaactaactacgcaaattaatgtggctggcgatccgtacacctatgacgactttgcttatgcaacccgtgaaggcttggtggttgatgcagtggaacacaccgatcctgaagccattaaggccaatgatgttgaaggcccattcgctgaaatggttttcgatctaaaattgacgcgtttggttgatggtgtagataaccaagttgttgatcgtccacgtctagcggtgtaatacaccaaaatggttcaaaattatcaggcgagtgatcatgatcactggcctgtttttatttcagggaagggtggagacaattacgtggacaatcaaatcattcaggaaaccgtagataaaattttaagcgtattgccgaatcaggctgggcaattggcacgcttggttcgtctgatgcagtttgcttgtgaccccaccattaccgtcattggtaaatataatcatggtaaaagccgactactcaatgagctgatcgggacagatattttttctgttgccgataaacgagagacgattcaactggccgaacataaacaagatcaggtgcgttggttggatgcacccggactcgatgcagatgttgcggcagtggatgatcgtcatgcttttgaagcagtctggacacaggcagatattcgcctttttgtgcattcagtccgagaaggcgaactcgatgcaactgagcatcatcttttacaacaacttattgaagatgcagaccatagccggcgccaaaccatactggtcttgacccagatagatcagataccggatcagacaattttaacccagattaaaacctcaattgcacagcaggtacccaaactcgatatttgggctgtttcggccactcgccaccgtcagggtattgaaaatggaaaaaccttgctgatcgaaaaaagtggaatcggcgcgttacgacatacacttgagcaggcacttgctcaggttccatctgcacgaacgtatgaaaagaatagattgctgtctgacttgcatcatcaacttaagcagttattactcgatcaaaaacatgtacttcagcaactacaacagacacagcagcagcaattgcatgactttgatacaggactcatcaacatactcgataagattcgagtagatcttgagcccattgtaaatatagatggtcaagaccaagcactcaatccagattcatttgccacgatgtttaaaaatacagcagccaagcagcaacgtgccaaagtgcagattgcttactcacgtgcctgtatcgagatcaatagccatctcatacgtcacggtgtggtgggtttacccgcagagcaacaaaccacgataaaaagtattgatacggtcattgttgcggtttttggaatttcagtgaaatttcgcgatcagctacgtgcattgttttataccgataccgaacgacaacgcttgcaaagagagtttcgattttattttgaaaagtcagcaggccgaatgattttagctgccaagattgagcagacaatgcggcagcaagggtgtattcaaaatgcaatgatggcgttgcaacagatggagagtgcagcatgaccagcggcggacacattcaattgtttatcgaacacacccggcagattgcgactgcccaaggggatatacagttggcattgcaatcgatgcagcaatggcgcgaagcatttgctacagcattaaaacaaaatacctttgatttaacgggctggtcaccgcagacaaagatcgccaatcaactcaagcaatttaaccataagcttacaacgcatgtatcgaattgggataccgaatggcatacttttagtgctgctcaatcggttgcagaagtatttcatgatcgggtgatgttgcttgtattcggtaagtttaatgccggaaagagttcattgtgtaacttactggccgaatgctttcgttctcacgaacaaaccgtgcaatattttcatgttcaaaatgaacagatattttataccgaatctcacttacgcgaaggtgcaaccgagacgacagcgcaactacagggcgtatgtctgggtgaaaaacttattttgctagatacaccaggtttgcattctggtactcagaaaaatgcagcgctcacacaaaaatttatcgacagtgcagatggtgtgctgtggctcagtagcgcaacttcaccgggtcaggtgcaagagctagatgcactggggcgcgagttaaagcgtcataaacctttatttcctgttattacccgaagcgattttgtcgaagaagatgaaattgatggtgagctatgtacagtgctttgcaataaaaattcagaacaacgtgcgttgcaagagtctgatgtattgatgcgtgcgaaagaaaaactgcacatatgcaagtggatgtgagtttattaaagccgcccgtgtccgtttcaactcaaatggcgcgtgaagcagatatgaacccacaagccatgaacgaggctggttttgagcgattatttgcagcacttttggctcttattgagcctgctttgcgctataagcagcgtaaacctgccgaagtattgttgcattttttgcaagaacatatcattgaaggtttaaggttttacctgcaacccgatctagagcaaatacaacaggacctcaaacaggctcaagatgatttacgacagctacacaccgatttagccgaggcagtctggcgtagcgtattgcctgagctaccacaacttcttgagcaacatgcaagtacacaaaatattgatgccgtagtgaacagtttgaacgagtggataaacgtcgcattcgaacaacagcttgcaattcagcttgatgcttatggtttaaatttggattcgcttagcaagatcgaaaaaaccgaaaaaatgcagtatgaacgcattgcgggaatggtggtgcatgatggcttgtacacgactctcacgcagcagattcaacaagctgtcaaagcttctacgagtgaattgattgatcagtgtcaggctcaacttgagcagtcaatcaaacatgttcaaacactcgatgaaaccttcatcgattacagcgcagcactcgatcaactcagccaagcgctacgcattgaataaagagcagtaaatttttcagacatattttattcgatgagtggcctgatatggtgcgttgcaaacacctcctgtacacaggcgagaattttaggaatgtaattactgtggtccatatttcgcaccgcgagtgaaattgggctataggcatcatcatctaaaattggaatataaagtagattcttcaccccaatatccatggcagacgccggtacgatgcagacgccttcacctgctgccaccaagccgagtgccagttgaatttctcgaatttcggtgagtttggatggtactaggcctagttcggtaaagagtgactgaataaaggtcgcaaaattgggcttttgagagactgggtacagcagcatcggttcatcaataatttgagagagatgaacccctgttgctgcaaactga

SEQ ID NO: 11 - protein, 311 aa, Acinetobacter baylyi
  PEPTIDE (1)..(311): Protein sequence of CatA (catechol 1,2-dioxygenase) from Acinetobacter baylyi ADP1
MEVKIFNTQDVQDFLRVASGLEQEGGNPRVKQIIHRVLSDLYKAIEDLNITSDEYWAGVAYLNQLGANQEAGLLSPGLGFDHYLDMRMDAEDAALGIENATPRTIEGPLYVAGAPESVGYARMDDGSDPNGHTLILHGTIFDADGKPLPNAKVEIWHANTKGFYSHFDPTGEQQAFNMRRSIITDENGQYRVRTILPAGYGCPPEGPTQQLLNQLGRHGNRPAHIHYFVSADGHRKLTTQINVAGDPYTYDDFAYATREGLVVDAVEHTDPEAIKANDVEGPFAEMVFDLKLTRLVDGVDNQVVDRPRLAV

SEQ ID NO: 12 - DNA, 1461 bp, Acinetobacter sp. ADP1
  gene (1)..(1461): DNA sequence of the quiC (3-dehydroshikimate dehydratase)gene from Acinetobacter sp. ADP1
atgaaattaacttctttacgcgtatctttattggcgctgggcttggtaacatcaggttttgctgcggcagaaacttatactgtagatcgttatcaggatgatagtgaaaaaggctctttgcgttgggcaattgaacaatctaatgcaaatagcgcacaagagaatcagattctgattcaggctgttggtaaggcaccttatgtgatcaaggtggataaaccgttaccaccgattaaatcatctgtaaaaattattggtacagaatgggataaaacgggcgaatttattgcgattgatggttcaaactatatcaagggcgaaggcgaaaaagcatgtccaggtgcaaatccaggacaatatggtaccaatgttcgtaccatgactttaccaggtttggttctacaagatgtcaatggtgtgaccctgaaaggtcttgatgttcatcgcttctgtattggtgtactggtaaatcgttcaagcaataatttgattcagcataaccgtatttcaaataattacggtggcgctggtgtcatgatcacgggtgatgatggtaaaggtaacccaacgtctaccaccaccaataacaacaaagtattggataatgtgtttattgacaatggcgatggtcttgaactgacgcgtggagcagcattcaacctgattgctaacaatctgtttacatcgaccaaagccaatccagagccgtctcaaggcattgaaattctttgggggaatgacaatgcagtggtgggtaacaaatttgaaaactattcagatggtctacaaatcaactggggtaaacgtaattacatcgcttataacgaattgaccaataactctttgggtttcaatcttacaggtgatggaaacatcttcgatagtaacaaagtgcatggcaatcgtattggtatcgcaattcgttctgaaaaagatgcaaatgcacgtatcacacttaccaaaaatcagatttgggataatggtaaagatatcaaacgctgtgaggctggtggttcatgtgttccaaaccaacgtttaggtgcaattgtatttggtgttcctgcgcttgagcatgaaggttttgtaggctctcgtggtggcggtgtagtcattgaacctgcaaaattacaaaaaacatgtacacagccaaatcaacaaaactgtaatgccattccgaaccaaggtattcaggcacctaaactgactgtcagtaaaaaacaacttacagttgaagttaaaggaacaccaaaccagcgttacaacgtagaattttttggaaatcgtaatgcatcttcttccgaagctgagcaatatttaggttcaattgttgtagtgacagatcatcaaggtcttgcaaaagcaaactgggcaccaaaagtcagcatgccatctgttactgcgaatgtaactgatcacttgggcgccacttcagagttaagttctgcagtgaaaatgagataa

SEQ ID NO: 13 - DNA, 1461 bp, Acinetobacter sp. arc5
  gene (1)..(1461): Codon-optimized DNA sequence of the quiC (3-dehydroshikimate dehydratase)gene from Acinetobacter sp. ADP1
atgaaactgaccagcctgcgtgttagcctgctggcactgggtctggttaccagcggttttgcagcagcagaaacctataccgttgatcgttatcaggatgatagcgaaaaaggtagcctgcgttgggcaattgaacagagcaatgcaaatagcgcacaagaaaaccagattctgattcaggcagttggtaaagcaccgtatgttatcaaagttgataaaccgctgcctccgattaaaagcagcgttaaaatcattggcaccgagtgggataaaaccggtgaatttattgcaattgatggcagcaactatatcaaaggcgaaggtgaaaaagcatgtccgggtgcaaatccgggtcagtatggcaccaatgttcgtaccatgaccctgcctggtctggttctgcaagatgttaatggtgttaccctgaaaggtctggatgttcatcgtttttgtattggtgttctggttaatcgcagcagcaataacctgattcagcataatcgtatcagcaacaattatggtggtgccggtgttatgattaccggtgatgatggtaaaggtaatccgaccagcaccaccaccaataataacaaagttctggataacgtgttcatcgataatggtgatggtctggaactgacccgtggtgcagcatttaatctgattgcaaataacctgtttaccagcacaaaagccaatccggaaccgagccagggtattgaaattctgtggggtaatgataatgccgtggtgggtaacaaattcgaaaactattcagatggcctgcaaatcaattggggtaaacgtaactatatcgcctataacgaactgaccaataacagcctgggtttcaatctgacaggtgatggtaacattttcgacagcaataaagtgcatggtaaccgtattggtattgccattcgtagtgaaaaagatgccaatgcacgtattaccctgaccaaaaatcagatttgggataacggcaaagatatcaaacgttgtgaagccggtggtagctgtgttccgaatcagcgtctgggtgcaattgtttttggtgttccggcactggaacatgaaggttttgttggtagccgtggcggtggtgttgttattgaaccggcaaaactgcaaaaaacctgcacccagccgaaccagcagaattgtaatgcaattcctaatcagggtattcaggcaccgaaactgacagttagcaaaaaacagctgaccgttgaagttaaaggcacccctaatcagcgttataatgtggaattttttggcaatcgtaatgccagcagcagcgaagcagaacagtatctgggtagcattgttgttgttaccgatcatcagggtctggcaaaagcaaattgggctccgaaagttagcatgccgagcgttaccgcaaatgtgacagatcatctgggtgcgaccagcgaactgagcagcgcagttaaaatgcgttaa

SEQ ID NO: 14 - protein, 486 aa, Acinetobacter sp. arc5
  PEPTIDE (1)..(486): Protein sequence of QuiC (3-dehydroshikimate dehydrogenase from Acinetobacter sp. ADP1
MKLTSLRVSLLALGLVTSGFAAAETYTVDRYQDDSEKGSLRWAIEQSNANSAQENQILIQAVGKAPYVIKVDKPLPPIKSSVKIIGTEWDKTGEFIAIDGSNYIKGEGEKACPGANPGQYGTNVRTMTLPGLVLQDVNGVTLKGLDVHRFCIGVLVNRSSNNLIQHNRISNNYGGAGVMITGDDGKGNPTSTTTNNNKVLDNVFIDNGDGLELTRGAAFNLIANNLFTSTKANPEPSQGIEILWGNDNAVVGNKFENYSDGLQINWGKRNYIAYNELTNNSLGFNLTGDGNIFDSNKVHGNRIGIAIRSEKDANARITLTKNQIWDNGKDIKRCEAGGSCVPNQRLGAIVFGVPALEHEGFVGSRGGGVVIEPAKLQKTCTQPNQQNCNAIPNQGIQAPKLTVSKKQLTVEVKGTPNQRYNVEFFGNRNASSSEAEQYLGSIVVVTDHQGLAKANWAPKVSMPSVTANVTDHLGATSELSSAVKMR

SEQ ID NO: 15 - DNA, 9462 bp, Escherichia coli
  misc_feature (1)..(9462): DNA sequence of the plasmid pAC21
gttgacagtaagacgggtaagcctgttgatgataccgctgccttactgggtgcattagccagtctgaatgacctgtcacgggataatccgaagtggtcagactggaaaatcagagggcaggaactgctgaacagcaaaaagtcagatagcaccacatagcagacccgccataaaacgccctgagaagcccgtgacgggcttttcttgtattatgggtagtttccttgcatgaatccataaaaggcgcctgtagtgccatttacccccattcactgccagagccgtgagcgcagcgaactgaatgtcacgaaaaagacagcgactcaggtgcctgatggtcggagacaaaaggaatattcagcgatttgcccgagcttgcgagggtgctacttaagcctttagggttttaaggtctgttttgtagaggagcaaacagcgtttgcgacatccttttgtaatactgcggaactgactaaagtagtgagttatacacagggctgggatctattctttttatctttttttattctttctttattctataaattataaccacttgaatataaacaaaaaaaacacacaaaggtctagcggaatttacagagggtctagcagaatttacaagttttccagcaaaggtctagcagaatttacagatacccacaactcaaaggaaaaggactagtaattatcattgactagcccatctcaattggtatagtgattaaaatcacctagaccaattgagatgtatgtctgaattagttgttttcaaagcaaatgaactagcgattagtcgctatgacttaacggagcatgaaaccaagctaattttatgctgtgtggcactactcaaccccacgattgaaaaccctacaaggaaagaacggacggtatcgttcacttataaccaatacgctcagatgatgaacatcagtagggaaaatgcttatggtgtattagctaaagcaaccagagagctgatgacgagaactgtggaaatcaggaatcctttggttaaaggctttgagattttccagtggacaaactatgccaagttctcaagcgaaaaattagaattagtttttagtgaagagatattgccttatcttttccagttaaaaaaattcataaaatataatctggaacatgttaagtcttttgaaaacaaatactctatgaggatttatgagtggttattaaaagaactaacacaaaagaaaactcacaaggcaaatatagagattagccttgatgaatttaagttcatgttaatgcttgaaaataactaccatgagtttaaaaggcttaaccaatgggttttgaaaccaataagtaaagatttaaacacttacagcaatatgaaattggtggttgataagcgaggccgcccgactgatacgttgattttccaagttgaactagatagacaaatggatctcgtaaccgaacttgagaacaaccagataaaaatgaatggtgacaaaataccaacaaccattacatcagattcctacctacgtaacggactaagaaaaacactacacgatgctttaactgcaaaaattcagctcaccagttttgaggcaaaatttttgagtgacatgcaaagtaagcatgatctcaatggttcgttctcatggctcacgcaaaaacaacgaaccacactagagaacatactggctaaatacggaaggatctgaggttcttatggctcttgtatctatcagtgaagcatcaagactaacaaacaaaagtagaacaactgttcaccgttagatatcaaagggaaaactgtccatatgcacagatgaaaacggtgtaaaaaagatagatacatcagagcttttacgagtttttggtgcatttaaagctgttcaccatgaacagatcgacaatgtaacagatgaacagcatgtaacacctaatagaacaggtgaaaccagtaaaacaaagcaactagaacatgaaattgaacacctgagacaacttgttacagctcaacagtcacacatagacagcctgaaacaggcgatgctgcttatcgaatcaaagctgccgacaacacgggagccagtgacgcctcccgtggggaaaaaatcatggcaattctggaagaaatagcgctttcagccggcaaacctgaagccggatctgcgattctgataacaaactagcaacaccagaacagcccgtttgcgggcagcaaaacccgttatgcttgtaaaccgttttgtgaaaaaatttttaaaataaaaaaggggacctctagggtccccaattaattagtaatataatctattaaaggtcattcaaaaggtcatccaccggatcaattcccctgctcgcgcaggctgggtgccaagctctcgggtaacatcaaggcccgatccttggagcccttgccctcccgcacgatgatcgtgccgtgatcgaaatccagatccttgacccgcagttgcaaaccctcactgatccgcatgcccgttccatacagaagctgggcgaacaaacgatgctcgccttccagaaaaccgaggatgcgaaccacttcatccggggtcagcaccaccggcaagcgccgcgacggccgaggtcttccgatctcctgaagccagggcagatccgtgcacagcaccttgccgtagaagaacagcaaggccgccaatgcctgacgatgcgtggagaccgaaaccttgcgctcgttcgccagccaggacagaaatgcctcgacttcgctgctgcccaaggttgccgggtgacgcacaccgtggaaacggatgaaggcacgaacccagtggacataagcctgttcggttcgtaagctgtaatgcaagtagcgtatgcgctcacgcaactggtccagaaccttgaccgaacgcagcggtggtaacggcgcagtggcggttttcatggcttgttatgactgtttttttggggtacagtctatgcctcgggcatccaagcagcaagcgcgttacgccgtgggtcgatgtttgatgttatggagcagcaacgatgttacgcagcagggcagtcgccctaaaacaaagttaaacatcatgagggaagcggtgatcgccgaagtatcgactcaactatcagaggtagttggcgtcatcgagcgccatctcgaaccgacgttgctggccgtacatttgtacggctccgcagtggatggcggcctgaagccacacagtgatattgatttgctggttacggtgaccgtaaggcttgatgaaacaacgcggcgagctttgatcaacgaccttttggaaacttcggcttcccctggagagagcgagattctccgcgctgtagaagtcaccattgttgtgcacgacgacatcattccgtggcgttatccagctaagcgcgaactgcaatttggagaatggcagcgcaatgacattcttgcaggtatcttcgagccagccacgatcgacattgatctggctatcttgctgacaaaagcaagagaacatagcgttgccttggtaggtccagcggcggaggaactctttgatccggttcctgaacaggatctatttgaggcgctaaatgaaaccttaacgctatggaactcgccgcccgactgggctggcgatgagcgaaatgtagtgcttacgttgtcccgcatttggtacagcgcagtaaccggcaaaatcgcgccgaaggatgtcgctgccgactgggcaatggagcgcctgccggcccagtatcagcccgtcatacttgaagctagacaggcttatcttggacaagaagaagatcgcttggcctcgcgcgcagatcagttggaagaatttgtccactacgtgaaaggcgagatcaccaaggtagtcggcaaataatgtctaacaattcgttcaagccgacgccgcttcgcggcgcggcttaactcaagcgttagatgcactaagcacataattgctcacagccaaactatcaggtcaagtctgcttttattatttttaagcgtgcataataagccctacacaaattgggagatatatcatgaaaggctggctttttcttgttatcgcaatagttggcgaagtaatcgcaacatccgcattaaaatctagcgagggctttactaagctgatccggtggatgaccttttgaatgacctttaatagattatattactaattaattggggaccctagaggtccccttttttattttaaaaattttttcacaaaacggtttacaagcatacgttggccgattcattaatgcagctggcacgacaggtttcccgactggaaagcgggcagtgagcgcaacgcaattaatgtgagttagctcactcattaggcaccccaggctttacactttatgcttccggctcgtatgttgtgtggaattgtgagcggataacaatttcacacaggaaacagctatgaccatgattacgccaagcttgcatgcctgcaggtcgactctagaggatcccccccgccgccgacagagtaataggttttacttaatagctcttcctgtcccttccaggcagtgatccgcattccgttctcatggcgaggcaacatttcgggatggaagataatgttctttgctacaggaaaatcaacaatatgcgcaccagatgccactggcagccgcccgctgcgcgttactaactctataaatgcagggatctcatcaatgacaacatcctgcggactgtttcctgccagtcccatgatgatggcgacatccgtggcatggcctttgcccgtcagtgacaacgacccgtacagatcgaccacaatatggctcgtcgcggttaataagccgctactttccagccgatcaataaaactttttccggcattcattggccccacggtatgcgaactggagggaccaatcccaattttgaaaatatcgaatgcactaatcatgtgacggaagatcacttcgcagaataaataaatcctggtgtccctgttgataccgggaagccctgggccaacttttggcgaaaatgagacgttgatcggcacgtaagaggttccaactttcaccataatgaaataagatcactaccgggcgtattttttgagttatcgagattttcaggagctaaggaagctaaaatggagaaaaaaatcactggatataccaccgttgatatatcccaatggcatcgtaaagaacattttgaggcatttcagtcagttgctcaatgtacctataaccagaccgttcagctggatattacggcctttttaaagaccgtaaagaaaaataagcacaagttttatccggcctttattcacattcttgcccgcctgatgaatgctcatccggaattccgtatggcaatgaaagacggtgagctggtgatatgggatagtgttcacccttgttacaccgttttccatgagcaaactgaaacgttttcatcgctctggagtgaataccacgacgatttccggcagtttctacacatatattcgcaagatgtggcgtgttacggtgaaaacctggcctatttccctaaagggtttattgagaatatgtttttcgtctcagccaatccctgggtgagtttcaccagttttgatttaaacgtggccaatatggacaacttcttcgcccccgttttcaccatgggcaaatattatacgcaaggcgacaaggtgctgatgccgctggcgattcaggttcatcatgccgtttgtgatggcttccatgtcggcagaatgcttaatgaattacaacagtactgcgatgagtggcagggcggggcgtaatttttttaaggcagttattggtgcccttaaacgcctggtgctacgcctgaataagtgataataagcggatgaatggcagaaattcgaaagcaaattcgacccggtcgtcggttcagggcagggtcgttaaatagccgcttatgtctattgctggtttantcggtacccggggatcgcggccgcggaccggatcccatcacatatacctgccgttcactattatttagtgaaatgagatattatgatattttctgaattgtgattaaaaaggcaactttatgcccatgcaacagaaactataaaaaatacagagaatgaaaagaaacagatagattttttagttctttaggcccgtagtctgcaaatccttttatgattttctatcaaacaaaagaggaaaatagaccagttgcaatccaaacgagagtctaatagaatgaggtcgaaaagtaaatcgcgcgggtttgttactgataaagcaggcaagacctaaaatgtgtaaagggcaaagtgtatactttggcgtcaccccttacatattttaggtctttttttattgtgcgtaactaacttgccatcttcaaacaggagggctggaagaagcagaccgctaacacagtacataaaaaaggagacatgaacgatgaacatcaaaaagtttgcaaaacaagcaacagtattaacctttactaccgcactgctggcaggaggcgcaactcaagcgtttgcgaaagaaacgaaccaaaagccatataaggaaacatacggcatttcccatattacacgccatgatatgctgcaaatccctgaacagcaaaaaaatgaaaaatatcaagttcctgaattcgattcgtccacaattaaaaatatctcttctgcaaaaggcctggacgtttgggacagctggccattacaaaacgctgacggcactgtcgcaaactatcacggctaccacatcgtctttgcattagccggagatcctaaaaatgcggatgacacatcgatttacatgttctatcaaaaagtcggcgaaacttctattgacagctggaaaaacgctggccgcgtctttaaagacagcgacaaattcgatgcaaatgattctatcctaaaagaccaaacacaagaatggtcaggttcagccacatttacatctgacggaaaaatccgtttattctacactgatttctccggtaaacattacggcaaacaaacactgacaactgcacaagttaacgtatcagcatcagacagctctttgaacatcaacggtgtagaggattataaatcaatctttgacggtgacggaaaaacgtatcaaaatgtacagcagttcatcgatgaaggcaactacagctcaggcgacaaccatacgctgagagatcctcactacgtagaagataaaggccacaaatacttagtatttgaagcaaacactggaactgaagatggctaccaaggcgaagaatctttatttaacaaagcatactatggcaaaagcacatcattcttccgtcaagaaagtcaaaaacttctgcaaagcgataaaaaacgcacggctgagttagcaaacggcgctctcggtatgattgagctaaacgatgattacacactgaaaaaagtgatgaaaccgctgattgcatctaacacagtaacagatgaaattgaacgcgcgaacgtctttaaaatgaacggcaaatggtacctgttcactgactcccgcggatcaaaaatgacgattgacggcattacgtctaacgatatttacatgcttggttatgtttctaattctttaactggcccatacaagccgctgaacaaaactggccttgtgttaaaaatggatcttgatcctaacgatgtaacctttacttactcacacttcgctgtacctcaagcgaaaggaaacaatgtcgtgattacaagctatatgacaaacagaggattctacgcagacaaacaatcaacgtttgcgccgagcttcctgctgaacatcaaaggcaagaaaacatctgttgtcaaagacagcatccttgaacaaggacaattaacagttaacaaataaaaacgcaaaagaaaatgccaatatcctattggcattttcttttatttcttccatttaaatggatgcatgcgctagcggagtgtatactggcttactatgttggcactgatgagggtgtcagtgaagtgcttcagcctcgtgagcgggacggtcgtaaggtcgttccgctccacttcactgaacggcaatccgagggtgtggatccaattaaggccacgctgtcatttaaattccgtttttccagttcaaatgcaattgccttcaatgcaccttcgtagctgtggtgagccagcggtgctggctctcccccatttacggataagaatgcattttccgagttaataccgtcggcaatacctgacattaatacttcacagtcgctggcatcgagtacggaaaacttaatcgaagacgaaccacagttaataaccaaaacaaccggaaattcattcatctcttttctcatcctgagttacggattaaaacagtttgtatacgatgttcaggatggtcagcagaccaatcacggtaacaaacacgttatccagacgaccacggtatttcgccagagacggcgctttacggatggcatacatcggcaacaggcacagcagggatgcgataatcggtgcgcccatggcttcaatcaggtcgaggatgttcgggttggcgtaggcaacaacccaggtggagcccatgatgaagatcatgctgagagtattcagtttacccagcgacactttggttttgtcacctttataaccgaacttcagaatcagaccattcaagccttccagcgtccccagatagtgaccgaagaaagatttgaagatagccacgagtgcgatgatggaagccgcatattccagtgtaatcgcgaacgttgttttggtaccggtcatggacgcaaagtggttagccagataagaaagcactggaatattctgcgctttggcttccgccatgttggccggagacagagtaaacaggcagctaaaggcaaagaacatcaccactgcaaccatcagcatgctggcacgagaaatgatttgggaacatttacgttcggtgaagtcgcgaccgaagtctttctcatactcttcacgtttagaaaccacgaaggaagagacgattggcgagaagttaaaggagaaaaccatgatggaaatccccagccagacagtgatcaggataccgtcatgaccggttaacgacagcgaaccgaggtcaacctggtcgataactgcagagttccagtaagggatcagcgacaaagaaatcagcaccaggctggcgataaacggccataccaggtagctcagggtaccgagctcgaattcactggccgtcgttttacaacgtcgtgactgggaaaaccctggcgttacccaacttaatcgccttgcagcacatccccctttcgccagctggcgtaatagcgaagaggcccgcaccgatcgcccttcccaacagttgcgcagcctgaatggcgaatggcgcctgatgcggtattttctccttacgcatctgtgcggtatttcacaccgcatatggtgcactctcagtacaatctgctctgatgccgcatagttaagccagccccgacacccgccaacacccgctgacgaattc

SEQ ID NO: 16 - DNA, 9430 bp, Escherichia coli
  misc_feature (1)..(9430): DNA sequence of the plasmid pAC19
gttgacagtaagacgggtaagcctgttgatgataccgctgccttactgggtgcattagccagtctgaatgacctgtcacgggataatccgaagtggtcagactggaaaatcagagggcaggaactgctgaacagcaaaaagtcagatagcaccacatagcagacccgccataaaacgccctgagaagcccgtgacgggcttttcttgtattatgggtagtttccttgcatgaatccataaaaggcgcctgtagtgccatttacccccattcactgccagagccgtgagcgcagcgaactgaatgtcacgaaaaagacagcgactcaggtgcctgatggtcggagacaaaaggaatattcagcgatttgcccgagcttgcgagggtgctacttaagcctttagggttttaaggtctgttttgtagaggagcaaacagcgtttgcgacatccttttgtaatactgcggaactgactaaagtagtgagttatacacagggctgggatctattctttttatctttttttattctttctttattctataaattataaccacttgaatataaacaaaaaaaacacacaaaggtctagcggaatttacagagggtctagcagaatttacaagttttccagcaaaggtctagcagaatttacagatacccacaactcaaaggaaaaggactagtaattatcattgactagcccatctcaattggtatagtgattaaaatcacctagaccaattgagatgtatgtctgaattagttgttttcaaagcaaatgaactagcgattagtcgctatgacttaacggagcatgaaaccaagctaattttatgctgtgtggcactactcaaccccacgattgaaaaccctacaaggaaagaacggacggtatcgttcacttataaccaatacgctcagatgatgaacatcagtagggaaaatgcttatggtgtattagctaaagcaaccagagagctgatgacgagaactgtggaaatcaggaatcctttggttaaaggctttgagattttccagtggacaaactatgccaagttctcaagcgaaaaattagaattagtttttagtgaagagatattgccttatcttttccagttaaaaaaattcataaaatataatctggaacatgttaagtcttttgaaaacaaatactctatgaggatttatgagtggttattaaaagaactaacacaaaagaaaactcacaaggcaaatatagagattagccttgatgaatttaagttcatgttaatgcttgaaaataactaccatgagtttaaaaggcttaaccaatgggttttgaaaccaataagtaaagatttaaacacttacagcaatatgaaattggtggttgataagcgaggccgcccgactgatacgttgattttccaagttgaactagatagacaaatggatctcgtaaccgaacttgagaacaaccagataaaaatgaatggtgacaaaataccaacaaccattacatcagattcctacctacgtaacggactaagaaaaacactacacgatgctttaactgcaaaaattcagctcaccagttttgaggcaaaatttttgagtgacatgcaaagtaagcatgatctcaatggttcgttctcatggctcacgcaaaaacaacgaaccacactagagaacatactggctaaatacggaaggatctgaggttcttatggctcttgtatctatcagtgaagcatcaagactaacaaacaaaagtagaacaactgttcaccgttagatatcaaagggaaaactgtccatatgcacagatgaaaacggtgtaaaaaagatagatacatcagagcttttacgagtttttggtgcatttaaagctgttcaccatgaacagatcgacaatgtaacagatgaacagcatgtaacacctaatagaacaggtgaaaccagtaaaacaaagcaactagaacatgaaattgaacacctgagacaacttgttacagctcaacagtcacacatagacagcctgaaacaggcgatgctgcttatcgaatcaaagctgccgacaacacgggagccagtgacgcctcccgtggggaaaaaatcatggcaattctggaagaaatagcgctttcagccggcaaacctgaagccggatctgcgattctgataacaaactagcaacaccagaacagcccgtttgcgggcagcaaaacccgttatgcttgtaaaccgttttgtgaaaaaatttttaaaataaaaaaggggacctctagggtccccaattaattagtaatataatctattaaaggtcattcaaaaggtcatccaccggatcaattcccctgctcgcgcaggctgggtgccaagctctcgggtaacatcaaggcccgatccttggagcccttgccctcccgcacgatgatcgtgccgtgatcgaaatccagatccttgacccgcagttgcaaaccctcactgatccgcatgcccgttccatacagaagctgggcgaacaaacgatgctcgccttccagaaaaccgaggatgcgaaccacttcatccggggtcagcaccaccggcaagcgccgcgacggccgaggtcttccgatctcctgaagccagggcagatccgtgcacagcaccttgccgtagaagaacagcaaggccgccaatgcctgacgatgcgtggagaccgaaaccttgcgctcgttcgccagccaggacagaaatgcctcgacttcgctgctgcccaaggttgccgggtgacgcacaccgtggaaacggatgaaggcacgaacccagtggacataagcctgttcggttcgtaagctgtaatgcaagtagcgtatgcgctcacgcaactggtccagaaccttgaccgaacgcagcggtggtaacggcgcagtggcggttttcatggcttgttatgactgtttttttggggtacagtctatgcctcgggcatccaagcagcaagcgcgttacgccgtgggtcgatgtttgatgttatggagcagcaacgatgttacgcagcagggcagtcgccctaaaacaaagttaaacatcatgagggaagcggtgatcgccgaagtatcgactcaactatcagaggtagttggcgtcatcgagcgccatctcgaaccgacgttgctggccgtacatttgtacggctccgcagtggatggcggcctgaagccacacagtgatattgatttgctggttacggtgaccgtaaggcttgatgaaacaacgcggcgagctttgatcaacgaccttttggaaacttcggcttcccctggagagagcgagattctccgcgctgtagaagtcaccattgttgtgcacgacgacatcattccgtggcgttatccagctaagcgcgaactgcaatttggagaatggcagcgcaatgacattcttgcaggtatcttcgagccagccacgatcgacattgatctggctatcttgctgacaaaagcaagagaacatagcgttgccttggtaggtccagcggcggaggaactctttgatccggttcctgaacaggatctatttgaggcgctaaatgaaaccttaacgctatggaactcgccgcccgactgggctggcgatgagcgaaatgtagtgcttacgttgtcccgcatttggtacagcgcagtaaccggcaaaatcgcgccgaaggatgtcgctgccgactgggcaatggagcgcctgccggcccagtatcagcccgtcatacttgaagctagacaggcttatcttggacaagaagaagatcgcttggcctcgcgcgcagatcagttggaagaatttgtccactacgtgaaaggcgagatcaccaaggtagtcggcaaataatgtctaacaattcgttcaagccgacgccgcttcgcggcgcggcttaactcaagcgttagatgcactaagcacataattgctcacagccaaactatcaggtcaagtctgcttttattatttttaagcgtgcataataagccctacacaaattgggagatatatcatgaaaggctggctttttcttgttatcgcaatagttggcgaagtaatcgcaacatccgcattaaaatctagcgagggctttactaagctgatccggtggatgaccttttgaatgacctttaatagattatattactaattaattggggaccctagaggtccccttttttattttaaaaattttttcacaaaacggtttacaagcatacgttggccgattcattaatgcagctggcacgacaggtttcccgactggaaagcgggcagtgagcgcaacgcaattaatgtgagttagctcactcattaggcaccccaggctttacactttatgcttccggctcgtatgttgtgtggaattgtgagcggataacaatttcacacaggaaacagctatgaccatgattacgccaagcttgcatgcctgcaggtcgactctagaggatcccccccgccgccgacagagtaataggttttacttaatagctcttcctgtcccttccaggcagtgatccgcattccgttctcatggcgaggcaacatttcgggatggaagataatgttctttgctacaggaaaatcaacaatatgcgcaccagatgccactggcagccgcccgctgcgcgttactaactctataaatgcagggatctcatcaatgacaacatcctgcggactgtttcctgccagtcccatgatgatggcgacatccgtggcatggcctttgcccgtcagtgacaacgacccgtacagatcgaccacaatatggctcgtcgcggttaataagccgctactttccagccgatcaataaaactttttccggcattcattggccccacggtatgcgaactggagggaccaatcccaattttgaaaatatcgaatgcactaatcatatccacaccctcggattgccgttcagtgaagtggagcggaacgaccttacgaccgtcccgctcacgaggctttacgcactacgtactgcgatggcttcaatttccagcgggagggcggatccactaatacaaaatatatcaaaagttaataataatattattcttacttaagacttttttgtcttcattttttagtaaaaaatataaaaaaggccacctcccgattttatcggaaggcagcctcttaaattcagttcataatattaaaaaatattattcaacttcagaatatttgttggcataggcagctgccgcacccaacagtccaggctgcggataagtaatcaacttaaccggaatcttggacatgacgcgttcaaagcgtccttttgaaacaaagcgctgacggaaaccagattctggcaaatgggaagcgatacgaagaccgacaccaccgccaataacaacactggttgcaccctgtgccaaagcaagatcaccagcgatagcgccaaggctcaagcagaagcgatccaaagcggcttcagcaaggttgtctttaccttccaaagccatctgccataatttaatatcatccagcaagctgaacggaacgccttcaatggcagccagtgcttcgtagatattaccaagacccgggccagaaataatgcgttcgatagaaacgcggcggaaacgttcacgtaaacgtgccagaattttgtcttcaagtctgtcaagcggagcaaagtcgatatgaccgccttcagtttcgatgacgaaataacggccttcagtccgcaacagatgggcaacacccaagcccgttcccggaccaagaatagtgataacaccatcgctaggaagcgcttcatcaggaccacaaatatgatccagataagaagaatccatatgcgcaaccgcgtgggcaaccgcgccgaagtcattgatcagaacatgcgtatcgatgtccagcttttcattcagagtagctggtcttaatacccaagggttattggtaagttttaaaacttcaccatgaaccgggccagcccatgcaatagctgcggcacgtggcagaggacgacccagtttttcaccgaaacgttcccaagctaactgcaagctagcatgttctgccgttttaaaagttgtttcttctccaagagaaagaacccgaccattgcttacttccgcaatagagaaacgcgcatgcgttccaccgatgtcaatcgcaacaatttccataataattcctttctgaaatcagaaggctacccaacaggtaaaataagtccgcccgctttataccatcgttgtaaacaaaaagtataattggttaagacttatctaaaaaagacaaaaggattcagccaaagcaagtttaactacttctgggagcgccacatctcctcgatttcatccaggctccgacctttggtttccggcacgaagcgagcaacaatcaagccacctaagatacttaatgctgcgaaaacgagataggagaaaccgtggttgaaagtctgattcaatgctggagaaccatcggcaaccttaaacaggaagttaaccaagatattagctaaccattgtccggtaacagcgataggcatagctgcgcccttgatggaactcgggaacatttctgacagaacaacccagcagacagggccccatgacataccaaagactgcaatataaagaagcacagaagccaaaggcaaaacaccaccgactttgaaccagaaacagcagcctaaaacagccatcattgcagccataccgagagcaccccaaataagcagaggtttacggccgaagcggtcaacaacacgggaagcaatcatggtgaagatgaagttcacaacaccgatagagatggtctgcaataatgccgtatcagctccaaaacctaaattctggaacatctgcggtgcataatacagcacggcgttaataccgactaactgctggaaggcagcaacggatacaccggcaaaaacaacggtgataccaaaagcaaacaaacctgcgctgcttttgtccatggctttatcaaagccagctttaatcttttgaatcgtcagattaggatcggcttgcggttccagacgagcaaggattttgctagcctcggaatgacgtcccttcatcaccaaccaatgcggcgtatccggtgcggttaacagcagcaataagaaggcaataccgatcaggccttctgaagccggagaccagcaccaaccactggcattaacccaatcgatagaaccgaaatgagccagtaaccaggtaaagatataaccggttaaagcacccgtcacaatggccatctgctgaccagaaaccatctgaccacgtttgtctggcggagcaatttcagcaatataggttggggtcaaggttgaaacgacaccgatacctaaaccggcaagaaaccggaaaaagcaaaaaatttgtaaagccgaaccaccggttccaaataatttttcggttaacgcagcaccaaaaccggcggcgacgaaacaaatggaactcatcaacaatccgccgcgacgaccgaagcgaataccaatccagccagacagcaaagaaccggtaacacaaccgaccaaaacagcaacaacgaccatcccagaaagggaagccgcagccgtagcagacaggtgacgaggggcaataaaatggatatcaaccggtgtaccgattgcagcgataaccgctgaatcgtaaccgaaaagcaagccgcctatagcagcgattagggctagtcgcgtgactagaccctgactactttcagaactcatggcgattcctctccctctagagcgtcctgctgttgttaagattattataccacaccttgtagataaagtcaacaactttttgcaaaatttttcaggaattttagcagaggttgttctggatgtagaacaaaacatctttccgctcttgtgctgttaggatatctttcttggaagctaggtaggcctcgagttatggcagttggttaaaaggaaacaaaaagaccgttttcacacaaaacggtctttttcgatttctttttacagtcacagccacttttgcaccaattaaggccacgctgtcatttaaactccgtttttccagttcaaatgcaattgccttcaatgcaccttcgtagctgtggtgagccagcggtgctggctctcccccatttacggataagaatgcattttccgagttaataccgtcggcaatacctgacattaatacttcacagtcgctggcatcgagtacggaaaacttaatcgaagacgaaccacagttaataaccaaaacaaccggaaattcattcatctcttttctcatcctgagttacggattaaaacagtttgtatacgatgttcaggatggtcagcagaccaatcacggtaacaaacacgttatccagacgaccacggtatttcgccagagacggcgctttacggatggcatacatcggcaacaggcacagcagggatgcgataatcggtgcgcccatggcttcaatcaggtcgaggatgttcgggttggcgtaggcaacaacccaggtggagcccatgatgaagatcatgctgagagtattcagtttacccagcgacactttggttttgtcacctttataaccgaacttcagaatcagaccattcaagccttccagcgtccccagatagtgaccgaagaaagatttgaagatagccacgagtgcgatgatggaagccgcatattccagtgtaatcgcgaacgttgttttggtaccggtcatggacgcaaagtggttagccagataagaaagcactggaatattctgcgctttggcttccgccatgttggccggagacagagtaaacaggcagctaaaggcaaagaacatcaccactgcaaccatcagcatgctggcacgagaaatgatttgggaacatttacgttcggtgaagtcgcgaccgaagtctttctcatactcttcacgtttagaaaccacgaaggaagagacgattggcgagaagttaaaggagaaaaccatgatggaaatccccagccagacagtgatcaggataccgtcatgaccggttaacgacagcgaaccgaggtcaacctggtcgataactgcagagttccagtaagggatcagcgacaaagaaatcagcaccaggctggcgataaacggccataccaggtagctcagggtaccgagctcgaattcactggccgtcgttttacaacgtcgtgactgggaaaaccctggcgttacccaacttaatcgccttgcagcacatccccctttcgccagctggcgtaatagcgaagaggcccgcaccgatcgcccttcccaacagttgcgcagcctgaatggcgaatggcgcctgatgcggtattttctccttacgcatctgtgcggtatttcacaccgcatatggtgcactctcagtacaatctgctctgatgccgcatagttaagccagccccgacacccgccaacacccgctgacgaattc

SEQ ID NO: 17 - DNA, 5768 bp, Escherichia coli
  misc_feature (1)..(5768): DNA sequence of the plasmid pMH17F
gttgacagtaagacgggtaagcctgttgatgataccgctgccttactgggtgcattagccagtctgaatgacctgtcacgggataatccgaagtggtcagactggaaaatcagagggcaggaactgctgaacagcaaaaagtcagatagcaccacatagcagacccgccataaaacgccctgagaagcccgtgacgggcttttcttgtattatgggtagtttccttgcatgaatccataaaaggcgcctgtagtgccatttacccccattcactgccagagccgtgagcgcagcgaactgaatgtcacgaaaaagacagcgactcaggtgcctgatggtcggagacaaaaggaatattcagcgatttgcccgagcttgcgagggtgctacttaagcctttagggttttaaggtctgttttgtagaggagcaaacagcgtttgcgacatccttttgtaatactgcggaactgactaaagtagtgagttatacacagggctgggatctattctttttatctttttttattctttctttattctataaattataaccacttgaatataaacaaaaaaaacacacaaaggtctagcggaatttacagagggtctagcagaatttacaagttttccagcaaaggtctagcagaatttacagatacccacaactcaaaggaaaaggactagtaattatcattgactagcccatctcaattggtatagtgattaaaatcacctagaccaattgagatgtatgtctgaattagttgttttcaaagcaaatgaactagcgattagtcgctatgacttaacggagcatgaaaccaagctaattttatgctgtgtggcactactcaaccccacgattgaaaaccctacaaggaaagaacggacggtatcgttcacttataaccaatacgctcagatgatgaacatcagtagggaaaatgcttatggtgtattagctaaagcaaccagagagctgatgacgagaactgtggaaatcaggaatcctttggttaaaggctttgagattttccagtggacaaactatgccaagttctcaagcgaaaaattagaattagtttttagtgaagagatattgccttatcttttccagttaaaaaaattcataaaatataatctggaacatgttaagtcttttgaaaacaaatactctatgaggatttatgagtggttattaaaagaactaacacaaaagaaaactcacaaggcaaatatagagattagccttgatgaatttaagttcatgttaatgcttgaaaataactaccatgagtttaaaaggcttaaccaatgggttttgaaaccaataagtaaagatttaaacacttacagcaatatgaaattggtggttgataagcgaggccgcccgactgatacgttgattttccaagttgaactagatagacaaatggatctcgtaaccgaacttgagaacaaccagataaaaatgaatggtgacaaaataccaacaaccattacatcagattcctacctacgtaacggactaagaaaaacactacacgatgctttaactgcaaaaattcagctcaccagttttgaggcaaaatttttgagtgacatgcaaagtaagcatgatctcaatggttcgttctcatggctcacgcaaaaacaacgaaccacactagagaacatactggctaaatacggaaggatctgaggttcttatggctcttgtatctatcagtgaagcatcaagactaacaaacaaaagtagaacaactgttcaccgttagatatcaaagggaaaactgtccatatgcacagatgaaaacggtgtaaaaaagatagatacatcagagcttttacgagtttttggtgcatttaaagctgttcaccatgaacagatcgacaatgtaacagatgaacagcatgtaacacctaatagaacaggtgaaaccagtaaaacaaagcaactagaacatgaaattgaacacctgagacaacttgttacagctcaacagtcacacatagacagcctgaaacaggcgatgctgcttatcgaatcaaagctgccgacaacacgggagccagtgacgcctcccgtggggaaaaaatcatggcaattctggaagaaatagcgctttcagccggcaaacctgaagccggatctgcgattctgataacaaactagcaacaccagaacagcccgtttgcgggcagcaaaacccgttatgcttgtaaaccgttttgtgaaaaaatttttaaaataaaaaaggggacctctagggtccccaattaattagtaatataatctattaaaggtcattcaaaaggtcatccaccggatcaattcccctgctcgcgcaggctgggtgccaagctctcgggtaacatcaaggcccgatccttggagcccttgccctcccgcacgatgatcgtgccgtgatcgaaatccagatccttgacccgcagttgcaaaccctcactgatccgcatgcccgttccatacagaagctgggcgaacaaacgatgctcgccttccagaaaaccgaggatgcgaaccacttcatccggggtcagcaccaccggcaagcgccgcgacggccgaggtcttccgatctcctgaagccagggcagatccgtgcacagcaccttgccgtagaagaacagcaaggccgccaatgcctgacgatgcgtggagaccgaaaccttgcgctcgttcgccagccaggacagaaatgcctcgacttcgctgctgcccaaggttgccgggtgacgcacaccgtggaaacggatgaaggcacgaacccagtggacataagcctgttcggttcgtaagctgtaatgcaagtagcgtatgcgctcacgcaactggtccagaaccttgaccgaacgcagcggtggtaacggcgcagtggcggttttcatggcttgttatgactgtttttttggggtacagtctatgcctcgggcatccaagcagcaagcgcgttacgccgtgggtcgatgtttgatgttatggagcagcaacgatgttacgcagcagggcagtcgccctaaaacaaagttaaacatcatgagggaagcggtgatcgccgaagtatcgactcaactatcagaggtagttggcgtcatcgagcgccatctcgaaccgacgttgctggccgtacatttgtacggctccgcagtggatggcggcctgaagccacacagtgatattgatttgctggttacggtgaccgtaaggcttgatgaaacaacgcggcgagctttgatcaacgaccttttggaaacttcggcttcccctggagagagcgagattctccgcgctgtagaagtcaccattgttgtgcacgacgacatcattccgtggcgttatccagctaagcgcgaactgcaatttggagaatggcagcgcaatgacattcttgcaggtatcttcgagccagccacgatcgacattgatctggctatcttgctgacaaaagcaagagaacatagcgttgccttggtaggtccagcggcggaggaactctttgatccggttcctgaacaggatctatttgaggcgctaaatgaaaccttaacgctatggaactcgccgcccgactgggctggcgatgagcgaaatgtagtgcttacgttgtcccgcatttggtacagcgcagtaaccggcaaaatcgcgccgaaggatgtcgctgccgactgggcaatggagcgcctgccggcccagtatcagcccgtcatacttgaagctagacaggcttatcttggacaagaagaagatcgcttggcctcgcgcgcagatcagttggaagaatttgtccactacgtgaaaggcgagatcaccaaggtagtcggcaaataatgtctaacaattcgttcaagccgacgccgcttcgcggcgcggcttaactcaagcgttagatgcactaagcacataattgctcacagccaaactatcaggtcaagtctgcttttattatttttaagcgtgcataataagccctacacaaattgggagatatatcatgaaaggctggctttttcttgttatcgcaatagttggcgaagtaatcgcaacatccgcattaaaatctagcgagggctttactaagctgatccggtggatgaccttttgaatgacctttaatagattatattactaattaattggggaccctagaggtccccttttttattttaaaaattttttcacaaaacggtttacaagcatacgttggccgattcattaatgcagctggcacgacaggtttcccgactggaaagcgggcagtgagcgcaacgcaattaatgtgagttagctcactcattaggcaccccaggctttacactttatgcttccggctcgtatgttgtgtggaattgtgagttacctagagagggtgagaattgccgaacatgcgcataagtttcccggacagatttcaggtggtcagcagcaacgcgttgccattgcgcgttcgctgtgtatgaagccgaaaattatgttgtttgatgagccaacgtcggcgctcgatcctgagatggtgaaagaggtgctggatacgatgattgggctggcgcagtcgggtatgacaatgttgtgtgtaacacatgagatggggtttgcacgaaccgtcgctgaccgggtaatttttatggatcgtggggaaatagtggagcaagctgcacctgatgaattttttgcgcatcctaaatcagagcgtacgagggcatttttatcgcaggtaatccattaattgaatgttagttcgaaaagcaaaaaggccatcctttcggatggcctttcgcttgatttgatgtctggcagtttatggcgggcgtcctgcccgccaccctccgggccgttgcttcgcaacgttcaaatccgctcccggcggatttgtcctactcgggagagtgttcaccgacaaacaacagataaaacaaaaggcccagtcttccgactgagccttttgttttatttgatgtctggcagttccctactctcgcatggggagaccccacactaccatcggcgctacggcggtttcacttctgagttcggcatggggtcaggtgggaccaccgcgctactgccgccagacaaattcttttctaatctgccgaactttaacctaaaaagtggtgctgatacccagagtcgaactggggacctcacccttaccaagggtgcgctctaccaactgagccatatcagcacgctaaatttgatgcctggcagttccctactctcgcatggggagaccccacactaccatcggcgctacggcgtttcacttctgagttcggcatggggtcaggtgggaccaccgcgctacggccgccaggcaaattctgttttatcagaccgcttctgcgttctgatttaatctgtatcaggctgaaaatcttctctcatccggataacaatttcacacaggaaacagctatgaccatgattacgccaagctcgagctcgaattcactggccgtcgttttacaacgtcgtgactgggaaaaccctggcgttacccaacttaatcgccttgcagcacatccccctttcgccagctggcgtaatagcgaagaggcccgcaccgatcgcccttcccaacagttgcgcagcctgaatggcgaatggcgcctgatgcggtattttctccttacgcatctgtgcggtatttcacaccgcatatggtgcactctcagtacaatctgctctgatgccgcatagttaagccagccccgacacccgccaacacccgctgacgaattc

SEQ ID NO: 18 - DNA, 1053 bp, Escherichia coli
  gene (1)..(1053): DNA sequence of the coding region of the wild type aroG gene
atgaattatcagaacgacgatttacgcatcaaagaaatcaaagagttacttcctcctgtcgcattgctggaaaaattccccgctactgaaaatgccgcgaatacggttgcccatgcccgaaaagcgatccataagatcctgaaaggtaatgatgatcgcctgttggttgtgattggcccatgctcaattcatgatcctgtcgcggcaaaagagtatgccactcgcttgctggcgctgcgtgaagagctgaaagatgagctggaaatcgtaatgcgcgtctattttgaaaagccgcgtaccacggtgggctggaaagggctgattaacgatccgcatatggataatagcttccagatcaacgacggtctgcgtatagcccgtaaattgctgcttgatattaacgacagcggtctgccagcggcaggtgagtttctcgatatgatcaccccacaatatctcgctgacctgatgagctggggcgcaattggcgcacgtaccaccgaatcgcaggtgcaccgcgaactggcatcagggctttcttgtccggtcggcttcaaaaatggcaccgacggtacgattaaagtggctatcgatgccattaatgccgccggtgcgccgcactgcttcctgtccgtaacgaaatgggggcattcggcgattgtgaataccagcggtaacggcgattgccatatcattctgcgcggcggtaaagagcctaactacagcgcgaagcacgttgctgaagtgaaagaagggctgaacaaagcaggcctgccagcacaggtgatgatcgatttcagccatgctaactcgtccaaacaattcaaaaagcagatggatgtttgtgctgacgtttgccagcagattgccggtggcgaaaaggccattattggcgtgatggtggaaagccatctggtggaaggcaatcagagcctcgagagcggggagccgctggcctacggtaagagcatcaccgatgcctgcatcggctgggaagataccgatgctctgttacgtcaactggcgaatgcagtaaaagcgcgtcgcgggtaa

SEQ ID NO: 19 - DNA, 8820 bp, Escherichia coli
  misc_feature (1)..(8820): DNA sequence of the plasmid pMH28F
gttgacagtaagacgggtaagcctgttgatgataccgctgccttactgggtgcattagccagtctgaatgacctgtcacgggataatccgaagtggtcagactggaaaatcagagggcaggaactgctgaacagcaaaaagtcagatagcaccacatagcagacccgccataaaacgccctgagaagcccgtgacgggcttttcttgtattatgggtagtttccttgcatgaatccataaaaggcgcctgtagtgccatttacccccattcactgccagagccgtgagcgcagcgaactgaatgtcacgaaaaagacagcgactcaggtgcctgatggtcggagacaaaaggaatattcagcgatttgcccgagcttgcgagggtgctacttaagcctttagggttttaaggtctgttttgtagaggagcaaacagcgtttgcgacatccttttgtaatactgcggaactgactaaagtagtgagttatacacagggctgggatctattctttttatctttttttattctttctttattctataaattataaccacttgaatataaacaaaaaaaacacacaaaggtctagcggaatttacagagggtctagcagaatttacaagttttccagcaaaggtctagcagaatttacagatacccacaactcaaaggaaaaggactagtaattatcattgactagcccatctcaattggtatagtgattaaaatcacctagaccaattgagatgtatgtctgaattagttgttttcaaagcaaatgaactagcgattagtcgctatgacttaacggagcatgaaaccaagctaattttatgctgtgtggcactactcaaccccacgattgaaaaccctacaaggaaagaacggacggtatcgttcacttataaccaatacgctcagatgatgaacatcagtagggaaaatgcttatggtgtattagctaaagcaaccagagagctgatgacgagaactgtggaaatcaggaatcctttggttaaaggctttgagattttccagtggacaaactatgccaagttctcaagcgaaaaattagaattagtttttagtgaagagatattgccttatcttttccagttaaaaaaattcataaaatataatctggaacatgttaagtcttttgaaaacaaatactctatgaggatttatgagtggttattaaaagaactaacacaaaagaaaactcacaaggcaaatatagagattagccttgatgaatttaagttcatgttaatgcttgaaaataactaccatgagtttaaaaggcttaaccaatgggttttgaaaccaataagtaaagatttaaacacttacagcaatatgaaattggtggttgataagcgaggccgcccgactgatacgttgattttccaagttgaactagatagacaaatggatctcgtaaccgaacttgagaacaaccagataaaaatgaatggtgacaaaataccaacaaccattacatcagattcctacctacgtaacggactaagaaaaacactacacgatgctttaactgcaaaaattcagctcaccagttttgaggcaaaatttttgagtgacatgcaaagtaagcatgatctcaatggttcgttctcatggctcacgcaaaaacaacgaaccacactagagaacatactggctaaatacggaaggatctgaggttcttatggctcttgtatctatcagtgaagcatcaagactaacaaacaaaagtagaacaactgttcaccgttagatatcaaagggaaaactgtccatatgcacagatgaaaacggtgtaaaaaagatagatacatcagagcttttacgagtttttggtgcatttaaagctgttcaccatgaacagatcgacaatgtaacagatgaacagcatgtaacacctaatagaacaggtgaaaccagtaaaacaaagcaactagaacatgaaattgaacacctgagacaacttgttacagctcaacagtcacacatagacagcctgaaacaggcgatgctgcttatcgaatcaaagctgccgacaacacgggagccagtgacgcctcccgtggggaaaaaatcatggcaattctggaagaaatagcgctttcagccggcaaacctgaagccggatctgcgattctgataacaaactagcaacaccagaacagcccgtttgcgggcagcaaaacccgttatgcttgtaaaccgttttgtgaaaaaatttttaaaataaaaaaggggacctctagggtccccaattaattagtaatataatctattaaaggtcattcaaaaggtcatccaccggatcaattcccctgctcgcgcaggctgggtgccaagctctcgggtaacatcaaggcccgatccttggagcccttgccctcccgcacgatgatcgtgccgtgatcgaaatccagatccttgacccgcagttgcaaaccctcactgatccgcatgcccgttccatacagaagctgggcgaacaaacgatgctcgccttccagaaaaccgaggatgcgaaccacttcatccggggtcagcaccaccggcaagcgccgcgacggccgaggtcttccgatctcctgaagccagggcagatccgtgcacagcaccttgccgtagaagaacagcaaggccgccaatgcctgacgatgcgtggagaccgaaaccttgcgctcgttcgccagccaggacagaaatgcctcgacttcgctgctgcccaaggttgccgggtgacgcacaccgtggaaacggatgaaggcacgaacccagtggacataagcctgttcggttcgtaagctgtaatgcaagtagcgtatgcgctcacgcaactggtccagaaccttgaccgaacgcagcggtggtaacggcgcagtggcggttttcatggcttgttatgactgtttttttggggtacagtctatgcctcgggcatccaagcagcaagcgcgttacgccgtgggtcgatgtttgatgttatggagcagcaacgatgttacgcagcagggcagtcgccctaaaacaaagttaaacatcatgagggaagcggtgatcgccgaagtatcgactcaactatcagaggtagttggcgtcatcgagcgccatctcgaaccgacgttgctggccgtacatttgtacggctccgcagtggatggcggcctgaagccacacagtgatattgatttgctggttacggtgaccgtaaggcttgatgaaacaacgcggcgagctttgatcaacgaccttttggaaacttcggcttcccctggagagagcgagattctccgcgctgtagaagtcaccattgttgtgcacgacgacatcattccgtggcgttatccagctaagcgcgaactgcaatttggagaatggcagcgcaatgacattcttgcaggtatcttcgagccagccacgatcgacattgatctggctatcttgctgacaaaagcaagagaacatagcgttgccttggtaggtccagcggcggaggaactctttgatccggttcctgaacaggatctatttgaggcgctaaatgaaaccttaacgctatggaactcgccgcccgactgggctggcgatgagcgaaatgtagtgcttacgttgtcccgcatttggtacagcgcagtaaccggcaaaatcgcgccgaaggatgtcgctgccgactgggcaatggagcgcctgccggcccagtatcagcccgtcatacttgaagctagacaggcttatcttggacaagaagaagatcgcttggcctcgcgcgcagatcagttggaagaatttgtccactacgtgaaaggcgagatcaccaaggtagtcggcaaataatgtctaacaattcgttcaagccgacgccgcttcgcggcgcggcttaactcaagcgttagatgcactaagcacataattgctcacagccaaactatcaggtcaagtctgcttttattatttttaagcgtgcataataagccctacacaaattgggagatatatcatgaaaggctggctttttcttgttatcgcaatagttggcgaagtaatcgcaacatccgcattaaaatctagcgagggctttactaagctgatccggtggatgaccttttgaatgacctttaatagattatattactaattaattggggaccctagaggtccccttttttattttaaaaattttttcacaaaacggtttacaagcatacgttggccgattcattaatgcagctggcacgacaggtttcccgactggaaagcgggcagtgagcgcaacgcaattaatgtgagttagctcactcattaggcaccccaggctttacactttatgcttccggctcgtatgttgtgtggaattgtgagttacctagagagggtgagaattgccgaacatgcgcataagtttcccggacagatttcaggtggtcagcagcaacgcgttgccattgcgcgttcgctgtgtatgaagccgaaaattatgttgtttgatgagccaacgtcggcgctcgatcctgagatggtgaaagaggtgctggatacgatgattgggctggcgcagtcgggtatgacaatgttgtgtgtaacacatgagatggggtttgcacgaaccgtcgctgaccgggtaatttttatggatcgtggggaaatagtggagcaagctgcacctgatgaattttttgcgcatcctaaatcagagcgtacgagggcatttttatcgcaggtaatccattaattgaatgttagttcgaaaagcaaaaaggccatcctttcggatggcctttcgcttgatttgatgtctggcagtttatggcgggcgtcctgcccgccaccctccgggccgttgcttcgcaacgttcaaatccggtgacggaagatcacttcgcagaataaataaatcctggtgtccctgttgataccgggaagccctgggccaacttttggcgaaaatgagacgttgatcggcacgtaagaggttccaactttcaccataatgaaataagatcactaccgggcgtattttttgagttatcgagattttcaggagctaaggaagctaaaatggagaaaaaaatcactggatataccaccgttgatatatcccaatggcatcgtaaagaacattttgaggcatttcagtcagttgctcaatgtacctataaccagaccgttcagctggatattacggcctttttaaagaccgtaaagaaaaataagcacaagttttatccggcctttattcacattcttgcccgcctgatgaatgctcatccggaattccgtatggcaatgaaagacggtgagctggtgatatgggatagtgttcacccttgttacaccgttttccatgagcaaactgaaacgttttcatcgctctggagtgaataccacgacgatttccggcagtttctacacatatattcgcaagatgtggcgtgttacggtgaaaacctggcctatttccctaaagggtttattgagaatatgtttttcgtctcagccaatccctgggtgagtttcaccagttttgatttaaacgtggccaatatggacaacttcttcgcccccgttttcaccatgggcaaatattatacgcaaggcgacaaggtgctgatgccgctggcgattcaggttcatcatgccgtttgtgatggcttccatgtcggcagaatgcttaatgaattacaacagtactgcgatgagtggcagggcggggcgtaatttttttaaggcagttattggtgcccttaaacgcctggtgctacgcctgaataagtgataataagcggatgaatggcagaaattcgaaagcaaattcgacccggtcgtcggttcagggcagggtcgttaaatagccgcttatgtctattgctggtttantcggtacccggggatcgcggccgcggaccggatcccatcacatatacctgccgttcactattatttagtgaaatgagatattatgatattttctgaattgtgattaaaaaggcaactttatgcccatgcaacagaaactataaaaaatacagagaatgaaaagaaacagatagattttttagttctttaggcccgtagtctgcaaatccttttatgattttctatcaaacaaaagaggaaaatagaccagttgcaatccaaacgagagtctaatagaatgaggtcgaaaagtaaatcgcgcgggtttgttactgataaagcaggcaagacctaaaatgtgtaaagggcaaagtgtatactttggcgtcaccccttacatattttaggtctttttttattgtgcgtaactaacttgccatcttcaaacaggagggctggaagaagcagaccgctaacacagtacataaaaaaggagacatgaacgatgaacatcaaaaagtttgcaaaacaagcaacagtattaacctttactaccgcactgctggcaggaggcgcaactcaagcgtttgcgaaagaaacgaaccaaaagccatataaggaaacatacggcatttcccatattacacgccatgatatgctgcaaatccctgaacagcaaaaaaatgaaaaatatcaagttcctgaattcgattcgtccacaattaaaaatatctcttctgcaaaaggcctggacgtttgggacagctggccattacaaaacgctgacggcactgtcgcaaactatcacggctaccacatcgtctttgcattagccggagatcctaaaaatgcggatgacacatcgatttacatgttctatcaaaaagtcggcgaaacttctattgacagctggaaaaacgctggccgcgtctttaaagacagcgacaaattcgatgcaaatgattctatcctaaaagaccaaacacaagaatggtcaggttcagccacatttacatctgacggaaaaatccgtttattctacactgatttctccggtaaacattacggcaaacaaacactgacaactgcacaagttaacgtatcagcatcagacagctctttgaacatcaacggtgtagaggattataaatcaatctttgacggtgacggaaaaacgtatcaaaatgtacagcagttcatcgatgaaggcaactacagctcaggcgacaaccatacgctgagagatcctcactacgtagaagataaaggccacaaatacttagtatttgaagcaaacactggaactgaagatggctaccaaggcgaagaatctttatttaacaaagcatactatggcaaaagcacatcattcttccgtcaagaaagtcaaaaacttctgcaaagcgataaaaaacgcacggctgagttagcaaacggcgctctcggtatgattgagctaaacgatgattacacactgaaaaaagtgatgaaaccgctgattgcatctaacacagtaacagatgaaattgaacgcgcgaacgtctttaaaatgaacggcaaatggtacctgttcactgactcccgcggatcaaaaatgacgattgacggcattacgtctaacgatatttacatgcttggttatgtttctaattctttaactggcccatacaagccgctgaacaaaactggccttgtgttaaaaatggatcttgatcctaacgatgtaacctttacttactcacacttcgctgtacctcaagcgaaaggaaacaatgtcgtgattacaagctatatgacaaacagaggattctacgcagacaaacaatcaacgtttgcgccgagcttcctgctgaacatcaaaggcaagaaaacatctgttgtcaaagacagcatccttgaacaaggacaattaacagttaacaaataaaaacgcaaaagaaaatgccaatatcctattggcattttcttttatttcttccatttaaatggatgcatgcgctagcggagtgtatactggcttactatgttggcactgatgagggtgtcagtgaagtgcttcctcccggcggatttgtcctactcgggagagtgttcaccgacaaacaacagataaaacaaaaggcccagtcttccgactgagccttttgttttatttgatgtctggcagttccctactctcgcatggggagaccccacactaccatcggcgctacggcggtttcacttctgagttcggcatggggtcaggtgggaccaccgcgctactgccgccagacaaattcttttctaatctgccgaactttaacctaaaaagtggtgctgatacccagagtcgaactggggacctcacccttaccaagggtgcgctctaccaactgagccatatcagcacgctaaatttgatgcctggcagttccctactctcgcatggggagaccccacactaccatcggcgctacggcgtttcacttctgagttcggcatggggtcaggtgggaccaccgcgctacggccgccaggcaaattctgttttatcagaccgcttctgcgttctgatttaatctgtatcaggctgaaaatcttctctcatccggataacaatttcacacaggaaacagctatgaccatgattacgccaagctcgagctcgaattcactggccgtcgttttacaacgtcgtgactgggaaaaccctggcgttacccaacttaatcgccttgcagcacatccccctttcgccagctggcgtaatagcgaagaggcccgcaccgatcgcccttcccaacagttgcgcagcctgaatggcgaatggcgcctgatgcggtattttctccttacgcatctgtgcggtatttcacaccgcatatggtgcactctcagtacaatctgctctgatgccgcatagttaagccagccccgacacccgccaacacccgctgacgaattc

SEQ ID NO: 20 - DNA, 4774 bp, Escherichia coli
  misc_feature (1)..(4774)
gttgacagtaagacgggtaagcctgttgatgataccgctgccttactgggtgcattagccagtctgaatgacctgtcacgggataatccgaagtggtcagactggaaaatcagagggcaggaactgctgaacagcaaaaagtcagatagcaccacatagcagacccgccataaaacgccctgagaagcccgtgacgggcttttcttgtattatgggtagtttccttgcatgaatccataaaaggcgcctgtagtgccatttacccccattcactgccagagccgtgagcgcagcgaactgaatgtcacgaaaaagacagcgactcaggtgcctgatggtcggagacaaaaggaatattcagcgatttgcccgagcttgcgagggtgctacttaagcctttagggttttaaggtctgttttgtagaggagcaaacagcgtttgcgacatccttttgtaatactgcggaactgactaaagtagtgagttatacacagggctgggatctattctttttatctttttttattctttctttattctataaattataaccacttgaatataaacaaaaaaaacacacaaaggtctagcggaatttacagagggtctagcagaatttacaagttttccagcaaaggtctagcagaatttacagatacccacaactcaaaggaaaaggactagtaattatcattgactagcccatctcaattggtatagtgattaaaatcacctagaccaattgagatgtatgtctgaattagttgttttcaaagcaaatgaactagcgattagtcgctatgacttaacggagcatgaaaccaagctaattttatgctgtgtggcactactcaaccccacgattgaaaaccctacaaggaaagaacggacggtatcgttcacttataaccaatacgctcagatgatgaacatcagtagggaaaatgcttatggtgtattagctaaagcaaccagagagctgatgacgagaactgtggaaatcaggaatcctttggttaaaggctttgagattttccagtggacaaactatgccaagttctcaagcgaaaaattagaattagtttttagtgaagagatattgccttatcttttccagttaaaaaaattcataaaatataatctggaacatgttaagtcttttgaaaacaaatactctatgaggatttatgagtggttattaaaagaactaacacaaaagaaaactcacaaggcaaatatagagattagccttgatgaatttaagttcatgttaatgcttgaaaataactaccatgagtttaaaaggcttaaccaatgggttttgaaaccaataagtaaagatttaaacacttacagcaatatgaaattggtggttgataagcgaggccgcccgactgatacgttgattttccaagttgaactagatagacaaatggatctcgtaaccgaacttgagaacaaccagataaaaatgaatggtgacaaaataccaacaaccattacatcagattcctacctacgtaacggactaagaaaaacactacacgatgctttaactgcaaaaattcagctcaccagttttgaggcaaaatttttgagtgacatgcaaagtaagcatgatctcaatggttcgttctcatggctcacgcaaaaacaacgaaccacactagagaacatactggctaaatacggaaggatctgaggttcttatggctcttgtatctatcagtgaagcatcaagactaacaaacaaaagtagaacaactgttcaccgttagatatcaaagggaaaactgtccatatgcacagatgaaaacggtgtaaaaaagatagatacatcagagcttttacgagtttttggtgcatttaaagctgttcaccatgaacagatcgacaatgtaacagatgaacagcatgtaacacctaatagaacaggtgaaaccagtaaaacaaagcaactagaacatgaaattgaacacctgagacaacttgttacagctcaacagtcacacatagacagcctgaaacaggcgatgctgcttatcgaatcaaagctgccgacaacacgggagccagtgacgcctcccgtggggaaaaaatcatggcaattctggaagaaatagcgctttcagccggcaaacctgaagccggatctgcgattctgataacaaactagcaacaccagaacagcccgtttgcgggcagcaaaacccgttatgcttgtaaaccgttttgtgaaaaaatttttaaaataaaaaaggggacctctagggtccccaattaattagtaatataatctattaaaggtcattcaaaaggtcatccaccggatcaattcccctgctcgcgcaggctgggtgccaagctctcgggtaacatcaaggcccgatccttggagcccttgccctcccgcacgatgatcgtgccgtgatcgaaatccagatccttgacccgcagttgcaaaccctcactgatccgcatgcccgttccatacagaagctgggcgaacaaacgatgctcgccttccagaaaaccgaggatgcgaaccacttcatccggggtcagcaccaccggcaagcgccgcgacggccgaggtcttccgatctcctgaagccagggcagatccgtgcacagcaccttgccgtagaagaacagcaaggccgccaatgcctgacgatgcgtggagaccgaaaccttgcgctcgttcgccagccaggacagaaatgcctcgacttcgctgctgcccaaggttgccgggtgacgcacaccgtggaaacggatgaaggcacgaacccagtggacataagcctgttcggttcgtaagctgtaatgcaagtagcgtatgcgctcacgcaactggtccagaaccttgaccgaacgcagcggtggtaacggcgcagtggcggttttcatggcttgttatgactgtttttttggggtacagtctatgcctcgggcatccaagcagcaagcgcgttacgccgtgggtcgatgtttgatgttatggagcagcaacgatgttacgcagcagggcagtcgccctaaaacaaagttaaacatcatgagggaagcggtgatcgccgaagtatcgactcaactatcagaggtagttggcgtcatcgagcgccatctcgaaccgacgttgctggccgtacatttgtacggctccgcagtggatggcggcctgaagccacacagtgatattgatttgctggttacggtgaccgtaaggcttgatgaaacaacgcggcgagctttgatcaacgaccttttggaaacttcggcttcccctggagagagcgagattctccgcgctgtagaagtcaccattgttgtgcacgacgacatcattccgtggcgttatccagctaagcgcgaactgcaatttggagaatggcagcgcaatgacattcttgcaggtatcttcgagccagccacgatcgacattgatctggctatcttgctgacaaaagcaagagaacatagcgttgccttggtaggtccagcggcggaggaactctttgatccggttcctgaacaggatctatttgaggcgctaaatgaaaccttaacgctatggaactcgccgcccgactgggctggcgatgagcgaaatgtagtgcttacgttgtcccgcatttggtacagcgcagtaaccggcaaaatcgcgccgaaggatgtcgctgccgactgggcaatggagcgcctgccggcccagtatcagcccgtcatacttgaagctagacaggcttatcttggacaagaagaagatcgcttggcctcgcgcgcagatcagttggaagaatttgtccactacgtgaaaggcgagatcaccaaggtagtcggcaaataatgtctaacaattcgttcaagccgacgccgcttcgcggcgcggcttaactcaagcgttagatgcactaagcacataattgctcacagccaaactatcaggtcaagtctgcttttattatttttaagcgtgcataataagccctacacaaattgggagatatatcatgaaaggctggctttttcttgttatcgcaatagttggcgaagtaatcgcaacatccgcattaaaatctagcgagggctttactaagctgatccggtggatgaccttttgaatgacctttaatagattatattactaattaattggggaccctagaggtccccttttttattttaaaaattttttcacaaaacggtttacaagcatacgttggccgattcattaatgcagctggcacgacaggtttcccgactggaaagcgggcagtgagcgcaacgcaattaatgtgagttagctcactcattaggcaccccaggctttacactttatgcttccggctcgtatgttgtgtggaattgtgagcggataacaatttcacacaggaaacagctatgaccatgattacgccaagcttgcatgcctgcaggtcgactctagaggatccccgggtaccgagctcgaattcactggccgtcgttttacaacgtcgtgactgggaaaaccctggcgttacccaacttaatcgccttgcagcacatccccctttcgccagctggcgtaatagcgaagaggcccgcaccgatcgcccttcccaacagttgcgcagcctgaatggcgaatggcgcctgatgcggtattttctccttacgcatctgtgcggtatttcacaccgcatatggtgcactctcagtacaatctgctctgatgccgcatagttaagccagccccgacacccgccaacacccgctgacgaattc

SEQ ID NO: 21 - DNA, 6432 bp, Escherichia coli
  misc_feature (1)..(6432): DNA sequence of the plasmid  pMG27
gttgacagtaagacgggtaagcctgttgatgataccgctgccttactgggtgcattagccagtctgaatgacctgtcacgggataatccgaagtggtcagactggaaaatcagagggcaggaactgctgaacagcaaaaagtcagatagcaccacatagcagacccgccataaaacgccctgagaagcccgtgacgggcttttcttgtattatgggtagtttccttgcatgaatccataaaaggcgcctgtagtgccatttacccccattcactgccagagccgtgagcgcagcgaactgaatgtcacgaaaaagacagcgactcaggtgcctgatggtcggagacaaaaggaatattcagcgatttgcccgagcttgcgagggtgctacttaagcctttagggttttaaggtctgttttgtagaggagcaaacagcgtttgcgacatccttttgtaatactgcggaactgactaaagtagtgagttatacacagggctgggatctattctttttatctttttttattctttctttattctataaattataaccacttgaatataaacaaaaaaaacacacaaaggtctagcggaatttacagagggtctagcagaatttacaagttttccagcaaaggtctagcagaatttacagatacccacaactcaaaggaaaaggactagtaattatcattgactagcccatctcaattggtatagtgattaaaatcacctagaccaattgagatgtatgtctgaattagttgttttcaaagcaaatgaactagcgattagtcgctatgacttaacggagcatgaaaccaagctaattttatgctgtgtggcactactcaaccccacgattgaaaaccctacaaggaaagaacggacggtatcgttcacttataaccaatacgctcagatgatgaacatcagtagggaaaatgcttatggtgtattagctaaagcaaccagagagctgatgacgagaactgtggaaatcaggaatcctttggttaaaggctttgagattttccagtggacaaactatgccaagttctcaagcgaaaaattagaattagtttttagtgaagagatattgccttatcttttccagttaaaaaaattcataaaatataatctggaacatgttaagtcttttgaaaacaaatactctatgaggatttatgagtggttattaaaagaactaacacaaaagaaaactcacaaggcaaatatagagattagccttgatgaatttaagttcatgttaatgcttgaaaataactaccatgagtttaaaaggcttaaccaatgggttttgaaaccaataagtaaagatttaaacacttacagcaatatgaaattggtggttgataagcgaggccgcccgactgatacgttgattttccaagttgaactagatagacaaatggatctcgtaaccgaacttgagaacaaccagataaaaatgaatggtgacaaaataccaacaaccattacatcagattcctacctacgtaacggactaagaaaaacactacacgatgctttaactgcaaaaattcagctcaccagttttgaggcaaaatttttgagtgacatgcaaagtaagcatgatctcaatggttcgttctcatggctcacgcaaaaacaacgaaccacactagagaacatactggctaaatacggaaggatctgaggttcttatggctcttgtatctatcagtgaagcatcaagactaacaaacaaaagtagaacaactgttcaccgttagatatcaaagggaaaactgtccatatgcacagatgaaaacggtgtaaaaaagatagatacatcagagcttttacgagtttttggtgcatttaaagctgttcaccatgaacagatcgacaatgtaacagatgaacagcatgtaacacctaatagaacaggtgaaaccagtaaaacaaagcaactagaacatgaaattgaacacctgagacaacttgttacagctcaacagtcacacatagacagcctgaaacaggcgatgctgcttatcgaatcaaagctgccgacaacacgggagccagtgacgcctcccgtggggaaaaaatcatggcaattctggaagaaatagcgctttcagccggcaaacctgaagccggatctgcgattctgataacaaactagcaacaccagaacagcccgtttgcgggcagcaaaacccgttatgcttgtaaaccgttttgtgaaaaaatttttaaaataaaaaaggggacctctagggtccccaattaattagtaatataatctattaaaggtcattcaaaaggtcatccaccggatcaattcccctgctcgcgcaggctgggtgccaagctctcgggtaacatcaaggcccgatccttggagcccttgccctcccgcacgatgatcgtgccgtgatcgaaatccagatccttgacccgcagttgcaaaccctcactgatccgcatgcccgttccatacagaagctgggcgaacaaacgatgctcgccttccagaaaaccgaggatgcgaaccacttcatccggggtcagcaccaccggcaagcgccgcgacggccgaggtcttccgatctcctgaagccagggcagatccgtgcacagcaccttgccgtagaagaacagcaaggccgccaatgcctgacgatgcgtggagaccgaaaccttgcgctcgttcgccagccaggacagaaatgcctcgacttcgctgctgcccaaggttgccgggtgacgcacaccgtggaaacggatgaaggcacgaacccagtggacataagcctgttcggttcgtaagctgtaatgcaagtagcgtatgcgctcacgcaactggtccagaaccttgaccgaacgcagcggtggtaacggcgcagtggcggttttcatggcttgttatgactgtttttttggggtacagtctatgcctcgggcatccaagcagcaagcgcgttacgccgtgggtcgatgtttgatgttatggagcagcaacgatgttacgcagcagggcagtcgccctaaaacaaagttaaacatcatgagggaagcggtgatcgccgaagtatcgactcaactatcagaggtagttggcgtcatcgagcgccatctcgaaccgacgttgctggccgtacatttgtacggctccgcagtggatggcggcctgaagccacacagtgatattgatttgctggttacggtgaccgtaaggcttgatgaaacaacgcggcgagctttgatcaacgaccttttggaaacttcggcttcccctggagagagcgagattctccgcgctgtagaagtcaccattgttgtgcacgacgacatcattccgtggcgttatccagctaagcgcgaactgcaatttggagaatggcagcgcaatgacattcttgcaggtatcttcgagccagccacgatcgacattgatctggctatcttgctgacaaaagcaagagaacatagcgttgccttggtaggtccagcggcggaggaactctttgatccggttcctgaacaggatctatttgaggcgctaaatgaaaccttaacgctatggaactcgccgcccgactgggctggcgatgagcgaaatgtagtgcttacgttgtcccgcatttggtacagcgcagtaaccggcaaaatcgcgccgaaggatgtcgctgccgactgggcaatggagcgcctgccggcccagtatcagcccgtcatacttgaagctagacaggcttatcttggacaagaagaagatcgcttggcctcgcgcgcagatcagttggaagaatttgtccactacgtgaaaggcgagatcaccaaggtagtcggcaaataatgtctaacaattcgttcaagccgacgccgcttcgcggcgcggcttaactcaagcgttagatgcactaagcacataattgctcacagccaaactatcaggtcaagtctgcttttattatttttaagcgtgcataataagccctacacaaattgggagatatatcatgaaaggctggctttttcttgttatcgcaatagttggcgaagtaatcgcaacatccgcattaaaatctagcgagggctttactaagctgatccggtggatgaccttttgaatgacctttaatagattatattactaattaattggggaccctagaggtccccttttttattttaaaaattttttcacaaaacggtttacaagcatacgttggccgattcattaatgcagctggcacgacaggtttcccgactggaaagcgggcagtgagcgcaacgcaattaatgtgagttagctcactcattaggcaccccaggctttacactttatgcttccggctcgtatgttgtgtggaattgtgagcggataacaatttcacacaggaaacagctatgaccatgattacgccaagcttgcatgcctgcaggtcgaccgttaaatctatcaccgcaagggataaatatctaacaccgtgcgtgttgactattttacctctggcggtgataatggttgcatgtactaatctagataaggaatatagccatgaccgcaccgattcaggatctgcgtgatgcaattgccctgctgcaacagcatgataatcagtatctggaaaccgatcatccggttgatccgaatgcagaactggcaggcgtttatcgtcatattggtgccggtggcaccgttaaacgtccgacccgtattggtccggcaatgatgtttaataacattaaaggttatccgcacagccgtattctggttggtatgcatgcaagccgtcagcgtgcagcactgctgctgggttgtgaagcaagtcagctggcactggaagttggtaaagcagttaaaaaaccggttgcaccggtggttgttccggcaagcagcgcaccgtgtcaagagcagatttttctggcagatgatccggattttgatctgcgtaccctgctgcctgcacataccaataccccgattgatgcaggtccgtttttttgtctgggtctggccctggcaagcgatccggtggatgcaagcctgaccgatgttaccattcatcgtctgtgtgttcagggtcgtgatgaactgagcatgttcctggcagcaggtcgccatattgaagtttttcgtcagaaagcagaagcagcaggtaaaccgctgccgattaccattaatatgggtctggacccagcaatctatattggcgcatgttttgaagcaccgaccaccccgtttggttataatgaactgggtgttgccggtgcactgcgtcagcgtccggttgaactggttcagggtgttagcgttccggaaaaagcaattgcacgtgccgaaattgttattgaaggtgaactgctgcctggtgttcgtgttcgtgaagatcagcataccaattcaggtcatgcaatgccggaatttccgggttattgtggtggtgcaaatccgagcctgccggttattaaagttaaagccgttaccatgcgcaataacgcaattctgcaaaccctggttggtccgggtgaagaacataccaccctggcaggtctgccgaccgaagcaagcatttggaatgcagttgaagcagcaattccgggttttctgcaaaatgtttatgcccataccgcaggcggtggtaaatttctgggtattctgcaagtgaaaaaacgtcagcctgccgatgaaggtcgtcagggtcaggcagccctgctggcgctggcaacctatagcgaactgaaaaatatcattctggtggatgaggatgtggacatttttgatagtgatgatattctgtgggcaatgaccacccgtatgcagggtgatgttagcattaccaccattccgggtattcgcggtcatcagctggacccgagccagacaccggaatattcaccgagcattcgtggtaatggtattagctgcaaaaccatctttgattgtaccgttccgtgggcactgaaaagccattttgaacgtgcaccgtttgcagatgttgatccgcgtccgtttgcacctgaatattttgcacgtctggaaaaaaatcagggcagcgcaaaataagctaataacaggcctgctggtaatcgcaggaatttttatttggatggatccccgggtaccgagctcgaattcactggccgtcgttttacaacgtcgtgactgggaaaaccctggcgttacccaacttaatcgccttgcagcacatccccctttcgccagctggcgtaatagcgaagaggcccgcaccgatcgcccttcccaacagttgcgcagcctgaatggcgaatggcgcctgatgcggtattttctccttacgcatctgtgcggtatttcacaccgcatatggtgcactctcagtacaatctgctctgatgccgcatagttaagccagccccgacacccgccaacacccgctgacgaattc

SEQ ID NO: 22 - DNA, 7294 bp, Escherichia coli
  misc_feature (1)..(7294): DNA sequence of the plasmid pMG31
gttgacagtaagacgggtaagcctgttgatgataccgctgccttactgggtgcattagccagtctgaatgacctgtcacgggataatccgaagtggtcagactggaaaatcagagggcaggaactgctgaacagcaaaaagtcagatagcaccacatagcagacccgccataaaacgccctgagaagcccgtgacgggcttttcttgtattatgggtagtttccttgcatgaatccataaaaggcgcctgtagtgccatttacccccattcactgccagagccgtgagcgcagcgaactgaatgtcacgaaaaagacagcgactcaggtgcctgatggtcggagacaaaaggaatattcagcgatttgcccgagcttgcgagggtgctacttaagcctttagggttttaaggtctgttttgtagaggagcaaacagcgtttgcgacatccttttgtaatactgcggaactgactaaagtagtgagttatacacagggctgggatctattctttttatctttttttattctttctttattctataaattataaccacttgaatataaacaaaaaaaacacacaaaggtctagcggaatttacagagggtctagcagaatttacaagttttccagcaaaggtctagcagaatttacagatacccacaactcaaaggaaaaggactagtaattatcattgactagcccatctcaattggtatagtgattaaaatcacctagaccaattgagatgtatgtctgaattagttgttttcaaagcaaatgaactagcgattagtcgctatgacttaacggagcatgaaaccaagctaattttatgctgtgtggcactactcaaccccacgattgaaaaccctacaaggaaagaacggacggtatcgttcacttataaccaatacgctcagatgatgaacatcagtagggaaaatgcttatggtgtattagctaaagcaaccagagagctgatgacgagaactgtggaaatcaggaatcctttggttaaaggctttgagattttccagtggacaaactatgccaagttctcaagcgaaaaattagaattagtttttagtgaagagatattgccttatcttttccagttaaaaaaattcataaaatataatctggaacatgttaagtcttttgaaaacaaatactctatgaggatttatgagtggttattaaaagaactaacacaaaagaaaactcacaaggcaaatatagagattagccttgatgaatttaagttcatgttaatgcttgaaaataactaccatgagtttaaaaggcttaaccaatgggttttgaaaccaataagtaaagatttaaacacttacagcaatatgaaattggtggttgataagcgaggccgcccgactgatacgttgattttccaagttgaactagatagacaaatggatctcgtaaccgaacttgagaacaaccagataaaaatgaatggtgacaaaataccaacaaccattacatcagattcctacctacgtaacggactaagaaaaacactacacgatgctttaactgcaaaaattcagctcaccagttttgaggcaaaatttttgagtgacatgcaaagtaagcatgatctcaatggttcgttctcatggctcacgcaaaaacaacgaaccacactagagaacatactggctaaatacggaaggatctgaggttcttatggctcttgtatctatcagtgaagcatcaagactaacaaacaaaagtagaacaactgttcaccgttagatatcaaagggaaaactgtccatatgcacagatgaaaacggtgtaaaaaagatagatacatcagagcttttacgagtttttggtgcatttaaagctgttcaccatgaacagatcgacaatgtaacagatgaacagcatgtaacacctaatagaacaggtgaaaccagtaaaacaaagcaactagaacatgaaattgaacacctgagacaacttgttacagctcaacagtcacacatagacagcctgaaacaggcgatgctgcttatcgaatcaaagctgccgacaacacgggagccagtgacgcctcccgtggggaaaaaatcatggcaattctggaagaaatagcgctttcagccggcaaacctgaagccggatctgcgattctgataacaaactagcaacaccagaacagcccgtttgcgggcagcaaaacccgttatgcttgtaaaccgttttgtgaaaaaatttttaaaataaaaaaggggacctctagggtccccaattaattagtaatataatctattaaaggtcattcaaaaggtcatccaccggatcaattcccctgctcgcgcaggctgggtgccaagctctcgggtaacatcaaggcccgatccttggagcccttgccctcccgcacgatgatcgtgccgtgatcgaaatccagatccttgacccgcagttgcaaaccctcactgatccgcatgcccgttccatacagaagctgggcgaacaaacgatgctcgccttccagaaaaccgaggatgcgaaccacttcatccggggtcagcaccaccggcaagcgccgcgacggccgaggtcttccgatctcctgaagccagggcagatccgtgcacagcaccttgccgtagaagaacagcaaggccgccaatgcctgacgatgcgtggagaccgaaaccttgcgctcgttcgccagccaggacagaaatgcctcgacttcgctgctgcccaaggttgccgggtgacgcacaccgtggaaacggatgaaggcacgaacccagtggacataagcctgttcggttcgtaagctgtaatgcaagtagcgtatgcgctcacgcaactggtccagaaccttgaccgaacgcagcggtggtaacggcgcagtggcggttttcatggcttgttatgactgtttttttggggtacagtctatgcctcgggcatccaagcagcaagcgcgttacgccgtgggtcgatgtttgatgttatggagcagcaacgatgttacgcagcagggcagtcgccctaaaacaaagttaaacatcatgagggaagcggtgatcgccgaagtatcgactcaactatcagaggtagttggcgtcatcgagcgccatctcgaaccgacgttgctggccgtacatttgtacggctccgcagtggatggcggcctgaagccacacagtgatattgatttgctggttacggtgaccgtaaggcttgatgaaacaacgcggcgagctttgatcaacgaccttttggaaacttcggcttcccctggagagagcgagattctccgcgctgtagaagtcaccattgttgtgcacgacgacatcattccgtggcgttatccagctaagcgcgaactgcaatttggagaatggcagcgcaatgacattcttgcaggtatcttcgagccagccacgatcgacattgatctggctatcttgctgacaaaagcaagagaacatagcgttgccttggtaggtccagcggcggaggaactctttgatccggttcctgaacaggatctatttgaggcgctaaatgaaaccttaacgctatggaactcgccgcccgactgggctggcgatgagcgaaatgtagtgcttacgttgtcccgcatttggtacagcgcagtaaccggcaaaatcgcgccgaaggatgtcgctgccgactgggcaatggagcgcctgccggcccagtatcagcccgtcatacttgaagctagacaggcttatcttggacaagaagaagatcgcttggcctcgcgcgcagatcagttggaagaatttgtccactacgtgaaaggcgagatcaccaaggtagtcggcaaataatgtctaacaattcgttcaagccgacgccgcttcgcggcgcggcttaactcaagcgttagatgcactaagcacataattgctcacagccaaactatcaggtcaagtctgcttttattatttttaagcgtgcataataagccctacacaaattgggagatatatcatgaaaggctggctttttcttgttatcgcaatagttggcgaagtaatcgcaacatccgcattaaaatctagcgagggctttactaagctgatccggtggatgaccttttgaatgacctttaatagattatattactaattaattggggaccctagaggtccccttttttattttaaaaattttttcacaaaacggtttacaagcatacgttggccgattcattaatgcagctggcacgacaggtttcccgactggaaagcgggcagtgagcgcaacgcaattaatgtgagttagctcactcattaggcaccccaggctttacactttatgcttccggctcgtatgttgtgtggaattgtgagcggataacaatttcacacaggaaacagctatgaccatgattacgccaagcttgctattgacgacagctatggttcactgtccaccaaccaaaactgtgctcagtaccgccaatatttctcccttgaggggtacaaagaggtgtccctagaagagatccacgctgtgtaaaaattttacaaaaaggtattgactttccctacagggtgtgtaataatttaattacaggcgggggcaaccccgcctgttctgcagaggaggaatatagccatggaagtgaaaatcttcaacacccaggatgttcaggattttctgcgtgttgcaagcggtctggaacaagagggtggtaatccgcgtgttaaacaaattattcatcgtgttctgagcgacctgtataaagcaattgaagatctgaatatcaccagcgacgaatattgggcaggcgttgcatatctgaatcagctgggtgcaaatcaagaagcaggtctgctgagtccgggtctgggttttgatcattatctggatatgcgtatggatgcagaagatgcagcactgggtattgaaaatgcaacaccgcgtaccattgaaggtccgctgtatgttgcgggtgcaccggaaagcgttggttatgcacgcatggatgatggtagcgatccgaatggtcataccctgattctgcatggcaccatttttgatgcagatggtaaaccgctgccgaatgcaaaagttgaaatttggcatgcaaacaccaaaggcttttatagccattttgatccgaccggtgaacagcaggcctttaatatgcgtcgtagcattattaccgatgagaatggtcagtatcgtgttcgtaccattctgcctgccggttatggttgtcctccggaaggtccgacccagcaactgctgaaccaactgggtcgtcatggtaatcgtccggcacatattcattattttgttagcgcagatggtcaccgtaaactgaccacccagattaatgttgccggtgatccgtatacctatgatgattttgcatatgccacccgtgaaggtctggttgttgatgcagttgaacataccgatccggaagcaattaaagccaatgatgtggaaggtccttttgccgaaatggtgtttgatctgaaactgacccgtctggttgatggtgttgataatcaggttgtggatcgtccgcgtctggcagtttaatacaccaaaatggttcaaaattatcaggcgagtgatcatgatcactggcctgtttttatttcagggaagggtggagacaattacgtggataatcagatcatccaagaaaccgtggataaaattctgagcgttctgccgaatcaggcaggtcagctggcacgtctggtgcgtctgatgcaatttgcatgcgatccgaccattaccgttattggcaaatataaccatggtaaaagccgtctgctgaatgaactgattggcaccgatatctttagcgttgcagataaacgtgaaaccattcagctggccgaacataaacaggatcaggttcgttggctggatgcacctggtctggatgccgatgttgcagcagttgatgatcgtcatgcatttgaagcagtttggacccaggcagatattcgtctgtttgttcatagcgttcgtgaaggtgaactggatgcaaccgaacaccatctgctgcaacagctgattgaagatgccgatcatagccgtcgtcagaccattctggttctgacccagattgatcagattccggatcagaccatcctgacacagattaaaaccagcattgcacagcaggttccgaaactggatatttgggcagttagcgcaacccgtcatcgtcagggcattgaaaacggtaaaaccctgctgatcgaaaaaagcggtattggtgcactgcgccataccctggaacaggcactggcacaggtgccgagcgcacgtacctatgaaaaaaatcgtctgctgtcagatctgcaccatcagctgaaacaactgctgctggatcagaaacatgttctgcaacaactgcaacagacacagcaacagcagctgcatgattttgataccggtctgattaacattctggacaaaattcgtgttgatctggaaccgattgtgaatattgatggtcaggatcaagcactgaatccggatagctttgcaaccatgtttaaaaacaccgcagcaaaacagcagcgtgccaaagttcagattgcatatagccgtgcatgcattgaaatcaacagccatctgattcgccatggtgttgttggtctgcctgcggaacagcagaccaccattaaaagcattgataccgtgattgttgccgtgtttggtatcagcgttaaatttcgtgatcagctgcgtgccctgttttataccgataccgaacgtcagcgtctgcaacgtgaatttcgtttctattttgaaaaaagtgccggtcgcatgattctggcagcaaaaattgaacagaccatgcgtcagcagggctgtattcagaatgccatgatggcactgcaacaaatggaaagcgcagcataaaaacacggacgccgcaaacggcgtccgaatttcttggtcgactctagaggatccccgggtaccgagctcgaattcactggccgtcgttttacaacgtcgtgactgggaaaaccctggcgttacccaacttaatcgccttgcagcacatccccctttcgccagctggcgtaatagcgaagaggcccgcaccgatcgcccttcccaacagttgcgcagcctgaatggcgaatggcgcctgatgcggtattttctccttacgcatctgtgcggtatttcacaccgcatatggtgcactctcagtacaatctgctctgatgccgcatagttaagccagccccgacacccgccaacacccgctgacgaattc

SEQ ID NO: 23 - DNA, 8952 bp, Escherichia coli
  misc_feature (1)..(8952): DNA sequence of the plasmid pMG33
gttgacagtaagacgggtaagcctgttgatgataccgctgccttactgggtgcattagccagtctgaatgacctgtcacgggataatccgaagtggtcagactggaaaatcagagggcaggaactgctgaacagcaaaaagtcagatagcaccacatagcagacccgccataaaacgccctgagaagcccgtgacgggcttttcttgtattatgggtagtttccttgcatgaatccataaaaggcgcctgtagtgccatttacccccattcactgccagagccgtgagcgcagcgaactgaatgtcacgaaaaagacagcgactcaggtgcctgatggtcggagacaaaaggaatattcagcgatttgcccgagcttgcgagggtgctacttaagcctttagggttttaaggtctgttttgtagaggagcaaacagcgtttgcgacatccttttgtaatactgcggaactgactaaagtagtgagttatacacagggctgggatctattctttttatctttttttattctttctttattctataaattataaccacttgaatataaacaaaaaaaacacacaaaggtctagcggaatttacagagggtctagcagaatttacaagttttccagcaaaggtctagcagaatttacagatacccacaactcaaaggaaaaggactagtaattatcattgactagcccatctcaattggtatagtgattaaaatcacctagaccaattgagatgtatgtctgaattagttgttttcaaagcaaatgaactagcgattagtcgctatgacttaacggagcatgaaaccaagctaattttatgctgtgtggcactactcaaccccacgattgaaaaccctacaaggaaagaacggacggtatcgttcacttataaccaatacgctcagatgatgaacatcagtagggaaaatgcttatggtgtattagctaaagcaaccagagagctgatgacgagaactgtggaaatcaggaatcctttggttaaaggctttgagattttccagtggacaaactatgccaagttctcaagcgaaaaattagaattagtttttagtgaagagatattgccttatcttttccagttaaaaaaattcataaaatataatctggaacatgttaagtcttttgaaaacaaatactctatgaggatttatgagtggttattaaaagaactaacacaaaagaaaactcacaaggcaaatatagagattagccttgatgaatttaagttcatgttaatgcttgaaaataactaccatgagtttaaaaggcttaaccaatgggttttgaaaccaataagtaaagatttaaacacttacagcaatatgaaattggtggttgataagcgaggccgcccgactgatacgttgattttccaagttgaactagatagacaaatggatctcgtaaccgaacttgagaacaaccagataaaaatgaatggtgacaaaataccaacaaccattacatcagattcctacctacgtaacggactaagaaaaacactacacgatgctttaactgcaaaaattcagctcaccagttttgaggcaaaatttttgagtgacatgcaaagtaagcatgatctcaatggttcgttctcatggctcacgcaaaaacaacgaaccacactagagaacatactggctaaatacggaaggatctgaggttcttatggctcttgtatctatcagtgaagcatcaagactaacaaacaaaagtagaacaactgttcaccgttagatatcaaagggaaaactgtccatatgcacagatgaaaacggtgtaaaaaagatagatacatcagagcttttacgagtttttggtgcatttaaagctgttcaccatgaacagatcgacaatgtaacagatgaacagcatgtaacacctaatagaacaggtgaaaccagtaaaacaaagcaactagaacatgaaattgaacacctgagacaacttgttacagctcaacagtcacacatagacagcctgaaacaggcgatgctgcttatcgaatcaaagctgccgacaacacgggagccagtgacgcctcccgtggggaaaaaatcatggcaattctggaagaaatagcgctttcagccggcaaacctgaagccggatctgcgattctgataacaaactagcaacaccagaacagcccgtttgcgggcagcaaaacccgttatgcttgtaaaccgttttgtgaaaaaatttttaaaataaaaaaggggacctctagggtccccaattaattagtaatataatctattaaaggtcattcaaaaggtcatccaccggatcaattcccctgctcgcgcaggctgggtgccaagctctcgggtaacatcaaggcccgatccttggagcccttgccctcccgcacgatgatcgtgccgtgatcgaaatccagatccttgacccgcagttgcaaaccctcactgatccgcatgcccgttccatacagaagctgggcgaacaaacgatgctcgccttccagaaaaccgaggatgcgaaccacttcatccggggtcagcaccaccggcaagcgccgcgacggccgaggtcttccgatctcctgaagccagggcagatccgtgcacagcaccttgccgtagaagaacagcaaggccgccaatgcctgacgatgcgtggagaccgaaaccttgcgctcgttcgccagccaggacagaaatgcctcgacttcgctgctgcccaaggttgccgggtgacgcacaccgtggaaacggatgaaggcacgaacccagtggacataagcctgttcggttcgtaagctgtaatgcaagtagcgtatgcgctcacgcaactggtccagaaccttgaccgaacgcagcggtggtaacggcgcagtggcggttttcatggcttgttatgactgtttttttggggtacagtctatgcctcgggcatccaagcagcaagcgcgttacgccgtgggtcgatgtttgatgttatggagcagcaacgatgttacgcagcagggcagtcgccctaaaacaaagttaaacatcatgagggaagcggtgatcgccgaagtatcgactcaactatcagaggtagttggcgtcatcgagcgccatctcgaaccgacgttgctggccgtacatttgtacggctccgcagtggatggcggcctgaagccacacagtgatattgatttgctggttacggtgaccgtaaggcttgatgaaacaacgcggcgagctttgatcaacgaccttttggaaacttcggcttcccctggagagagcgagattctccgcgctgtagaagtcaccattgttgtgcacgacgacatcattccgtggcgttatccagctaagcgcgaactgcaatttggagaatggcagcgcaatgacattcttgcaggtatcttcgagccagccacgatcgacattgatctggctatcttgctgacaaaagcaagagaacatagcgttgccttggtaggtccagcggcggaggaactctttgatccggttcctgaacaggatctatttgaggcgctaaatgaaaccttaacgctatggaactcgccgcccgactgggctggcgatgagcgaaatgtagtgcttacgttgtcccgcatttggtacagcgcagtaaccggcaaaatcgcgccgaaggatgtcgctgccgactgggcaatggagcgcctgccggcccagtatcagcccgtcatacttgaagctagacaggcttatcttggacaagaagaagatcgcttggcctcgcgcgcagatcagttggaagaatttgtccactacgtgaaaggcgagatcaccaaggtagtcggcaaataatgtctaacaattcgttcaagccgacgccgcttcgcggcgcggcttaactcaagcgttagatgcactaagcacataattgctcacagccaaactatcaggtcaagtctgcttttattatttttaagcgtgcataataagccctacacaaattgggagatatatcatgaaaggctggctttttcttgttatcgcaatagttggcgaagtaatcgcaacatccgcattaaaatctagcgagggctttactaagctgatccggtggatgaccttttgaatgacctttaatagattatattactaattaattggggaccctagaggtccccttttttattttaaaaattttttcacaaaacggtttacaagcatacgttggccgattcattaatgcagctggcacgacaggtttcccgactggaaagcgggcagtgagcgcaacgcaattaatgtgagttagctcactcattaggcaccccaggctttacactttatgcttccggctcgtatgttgtgtggaattgtgagcggataacaatttcacacaggaaacagctatgaccatgattacgccaagcttgctattgacgacagctatggttcactgtccaccaaccaaaactgtgctcagtaccgccaatatttctcccttgaggggtacaaagaggtgtccctagaagagatccacgctgtgtaaaaattttacaaaaaggtattgactttccctacagggtgtgtaataatttaattacaggcgggggcaaccccgcctgttctgcagaggaggaatatagccatggaagtgaaaatcttcaacacccaggatgttcaggattttctgcgtgttgcaagcggtctggaacaagagggtggtaatccgcgtgttaaacaaattattcatcgtgttctgagcgacctgtataaagcaattgaagatctgaatatcaccagcgacgaatattgggcaggcgttgcatatctgaatcagctgggtgcaaatcaagaagcaggtctgctgagtccgggtctgggttttgatcattatctggatatgcgtatggatgcagaagatgcagcactgggtattgaaaatgcaacaccgcgtaccattgaaggtccgctgtatgttgcgggtgcaccggaaagcgttggttatgcacgcatggatgatggtagcgatccgaatggtcataccctgattctgcatggcaccatttttgatgcagatggtaaaccgctgccgaatgcaaaagttgaaatttggcatgcaaacaccaaaggcttttatagccattttgatccgaccggtgaacagcaggcctttaatatgcgtcgtagcattattaccgatgagaatggtcagtatcgtgttcgtaccattctgcctgccggttatggttgtcctccggaaggtccgacccagcaactgctgaaccaactgggtcgtcatggtaatcgtccggcacatattcattattttgttagcgcagatggtcaccgtaaactgaccacccagattaatgttgccggtgatccgtatacctatgatgattttgcatatgccacccgtgaaggtctggttgttgatgcagttgaacataccgatccggaagcaattaaagccaatgatgtggaaggtccttttgccgaaatggtgtttgatctgaaactgacccgtctggttgatggtgttgataatcaggttgtggatcgtccgcgtctggcagtttaatacaccaaaatggttcaaaattatcaggcgagtgatcatgatcactggcctgtttttatttcagggaagggtggagacaattacgtggataatcagatcatccaagaaaccgtggataaaattctgagcgttctgccgaatcaggcaggtcagctggcacgtctggtgcgtctgatgcaatttgcatgcgatccgaccattaccgttattggcaaatataaccatggtaaaagccgtctgctgaatgaactgattggcaccgatatctttagcgttgcagataaacgtgaaaccattcagctggccgaacataaacaggatcaggttcgttggctggatgcacctggtctggatgccgatgttgcagcagttgatgatcgtcatgcatttgaagcagtttggacccaggcagatattcgtctgtttgttcatagcgttcgtgaaggtgaactggatgcaaccgaacaccatctgctgcaacagctgattgaagatgccgatcatagccgtcgtcagaccattctggttctgacccagattgatcagattccggatcagaccatcctgacacagattaaaaccagcattgcacagcaggttccgaaactggatatttgggcagttagcgcaacccgtcatcgtcagggcattgaaaacggtaaaaccctgctgatcgaaaaaagcggtattggtgcactgcgccataccctggaacaggcactggcacaggtgccgagcgcacgtacctatgaaaaaaatcgtctgctgtcagatctgcaccatcagctgaaacaactgctgctggatcagaaacatgttctgcaacaactgcaacagacacagcaacagcagctgcatgattttgataccggtctgattaacattctggacaaaattcgtgttgatctggaaccgattgtgaatattgatggtcaggatcaagcactgaatccggatagctttgcaaccatgtttaaaaacaccgcagcaaaacagcagcgtgccaaagttcagattgcatatagccgtgcatgcattgaaatcaacagccatctgattcgccatggtgttgttggtctgcctgcggaacagcagaccaccattaaaagcattgataccgtgattgttgccgtgtttggtatcagcgttaaatttcgtgatcagctgcgtgccctgttttataccgataccgaacgtcagcgtctgcaacgtgaatttcgtttctattttgaaaaaagtgccggtcgcatgattctggcagcaaaaattgaacagaccatgcgtcagcagggctgtattcagaatgccatgatggcactgcaacaaatggaaagcgcagcataaaaacacggacgccgcaaacggcgtccgaatttcttggtcgaccgttaaatctatcaccgcaagggataaatatctaacaccgtgcgtgttgactattttacctctggcggtgataatggttgcatgtactaatctagataaggaatatagccatgaccgcaccgattcaggatctgcgtgatgcaattgccctgctgcaacagcatgataatcagtatctggaaaccgatcatccggttgatccgaatgcagaactggcaggcgtttatcgtcatattggtgccggtggcaccgttaaacgtccgacccgtattggtccggcaatgatgtttaataacattaaaggttatccgcacagccgtattctggttggtatgcatgcaagccgtcagcgtgcagcactgctgctgggttgtgaagcaagtcagctggcactggaagttggtaaagcagttaaaaaaccggttgcaccggtggttgttccggcaagcagcgcaccgtgtcaagagcagatttttctggcagatgatccggattttgatctgcgtaccctgctgcctgcacataccaataccccgattgatgcaggtccgtttttttgtctgggtctggccctggcaagcgatccggtggatgcaagcctgaccgatgttaccattcatcgtctgtgtgttcagggtcgtgatgaactgagcatgttcctggcagcaggtcgccatattgaagtttttcgtcagaaagcagaagcagcaggtaaaccgctgccgattaccattaatatgggtctggacccagcaatctatattggcgcatgttttgaagcaccgaccaccccgtttggttataatgaactgggtgttgccggtgcactgcgtcagcgtccggttgaactggttcagggtgttagcgttccggaaaaagcaattgcacgtgccgaaattgttattgaaggtgaactgctgcctggtgttcgtgttcgtgaagatcagcataccaattcaggtcatgcaatgccggaatttccgggttattgtggtggtgcaaatccgagcctgccggttattaaagttaaagccgttaccatgcgcaataacgcaattctgcaaaccctggttggtccgggtgaagaacataccaccctggcaggtctgccgaccgaagcaagcatttggaatgcagttgaagcagcaattccgggttttctgcaaaatgtttatgcccataccgcaggcggtggtaaatttctgggtattctgcaagtgaaaaaacgtcagcctgccgatgaaggtcgtcagggtcaggcagccctgctggcgctggcaacctatagcgaactgaaaaatatcattctggtggatgaggatgtggacatttttgatagtgatgatattctgtgggcaatgaccacccgtatgcagggtgatgttagcattaccaccattccgggtattcgcggtcatcagctggacccgagccagacaccggaatattcaccgagcattcgtggtaatggtattagctgcaaaaccatctttgattgtaccgttccgtgggcactgaaaagccattttgaacgtgcaccgtttgcagatgttgatccgcgtccgtttgcacctgaatattttgcacgtctggaaaaaaatcagggcagcgcaaaataagctaataacaggcctgctggtaatcgcaggaatttttatttggatggatccccgggtaccgagctcgaattcactggccgtcgttttacaacgtcgtgactgggaaaaccctggcgttacccaacttaatcgccttgcagcacatccccctttcgccagctggcgtaatagcgaagaggcccgcaccgatcgcccttcccaacagttgcgcagcctgaatggcgaatggcgcctgatgcggtattttctccttacgcatctgtgcggtatttcacaccgcatatggtgcactctcagtacaatctgctctgatgccgcatagttaagccagccccgacacccgccaacacccgctgacgaattc

SEQ ID NO: 24 - DNA, 10630 bp, Escherichia coli
  misc_feature (1)..(10630): DNA sequence of the plasmid pMG37
gttgacagtaagacgggtaagcctgttgatgataccgctgccttactgggtgcattagccagtctgaatgacctgtcacgggataatccgaagtggtcagactggaaaatcagagggcaggaactgctgaacagcaaaaagtcagatagcaccacatagcagacccgccataaaacgccctgagaagcccgtgacgggcttttcttgtattatgggtagtttccttgcatgaatccataaaaggcgcctgtagtgccatttacccccattcactgccagagccgtgagcgcagcgaactgaatgtcacgaaaaagacagcgactcaggtgcctgatggtcggagacaaaaggaatattcagcgatttgcccgagcttgcgagggtgctacttaagcctttagggttttaaggtctgttttgtagaggagcaaacagcgtttgcgacatccttttgtaatactgcggaactgactaaagtagtgagttatacacagggctgggatctattctttttatctttttttattctttctttattctataaattataaccacttgaatataaacaaaaaaaacacacaaaggtctagcggaatttacagagggtctagcagaatttacaagttttccagcaaaggtctagcagaatttacagatacccacaactcaaaggaaaaggactagtaattatcattgactagcccatctcaattggtatagtgattaaaatcacctagaccaattgagatgtatgtctgaattagttgttttcaaagcaaatgaactagcgattagtcgctatgacttaacggagcatgaaaccaagctaattttatgctgtgtggcactactcaaccccacgattgaaaaccctacaaggaaagaacggacggtatcgttcacttataaccaatacgctcagatgatgaacatcagtagggaaaatgcttatggtgtattagctaaagcaaccagagagctgatgacgagaactgtggaaatcaggaatcctttggttaaaggctttgagattttccagtggacaaactatgccaagttctcaagcgaaaaattagaattagtttttagtgaagagatattgccttatcttttccagttaaaaaaattcataaaatataatctggaacatgttaagtcttttgaaaacaaatactctatgaggatttatgagtggttattaaaagaactaacacaaaagaaaactcacaaggcaaatatagagattagccttgatgaatttaagttcatgttaatgcttgaaaataactaccatgagtttaaaaggcttaaccaatgggttttgaaaccaataagtaaagatttaaacacttacagcaatatgaaattggtggttgataagcgaggccgcccgactgatacgttgattttccaagttgaactagatagacaaatggatctcgtaaccgaacttgagaacaaccagataaaaatgaatggtgacaaaataccaacaaccattacatcagattcctacctacgtaacggactaagaaaaacactacacgatgctttaactgcaaaaattcagctcaccagttttgaggcaaaatttttgagtgacatgcaaagtaagcatgatctcaatggttcgttctcatggctcacgcaaaaacaacgaaccacactagagaacatactggctaaatacggaaggatctgaggttcttatggctcttgtatctatcagtgaagcatcaagactaacaaacaaaagtagaacaactgttcaccgttagatatcaaagggaaaactgtccatatgcacagatgaaaacggtgtaaaaaagatagatacatcagagcttttacgagtttttggtgcatttaaagctgttcaccatgaacagatcgacaatgtaacagatgaacagcatgtaacacctaatagaacaggtgaaaccagtaaaacaaagcaactagaacatgaaattgaacacctgagacaacttgttacagctcaacagtcacacatagacagcctgaaacaggcgatgctgcttatcgaatcaaagctgccgacaacacgggagccagtgacgcctcccgtggggaaaaaatcatggcaattctggaagaaatagcgctttcagccggcaaacctgaagccggatctgcgattctgataacaaactagcaacaccagaacagcccgtttgcgggcagcaaaacccgttatgcttgtaaaccgttttgtgaaaaaatttttaaaataaaaaaggggacctctagggtccccaattaattagtaatataatctattaaaggtcattcaaaaggtcatccaccggatcaattcccctgctcgcgcaggctgggtgccaagctctcgggtaacatcaaggcccgatccttggagcccttgccctcccgcacgatgatcgtgccgtgatcgaaatccagatccttgacccgcagttgcaaaccctcactgatccgcatgcccgttccatacagaagctgggcgaacaaacgatgctcgccttccagaaaaccgaggatgcgaaccacttcatccggggtcagcaccaccggcaagcgccgcgacggccgaggtcttccgatctcctgaagccagggcagatccgtgcacagcaccttgccgtagaagaacagcaaggccgccaatgcctgacgatgcgtggagaccgaaaccttgcgctcgttcgccagccaggacagaaatgcctcgacttcgctgctgcccaaggttgccgggtgacgcacaccgtggaaacggatgaaggcacgaacccagtggacataagcctgttcggttcgtaagctgtaatgcaagtagcgtatgcgctcacgcaactggtccagaaccttgaccgaacgcagcggtggtaacggcgcagtggcggttttcatggcttgttatgactgtttttttggggtacagtctatgcctcgggcatccaagcagcaagcgcgttacgccgtgggtcgatgtttgatgttatggagcagcaacgatgttacgcagcagggcagtcgccctaaaacaaagttaaacatcatgagggaagcggtgatcgccgaagtatcgactcaactatcagaggtagttggcgtcatcgagcgccatctcgaaccgacgttgctggccgtacatttgtacggctccgcagtggatggcggcctgaagccacacagtgatattgatttgctggttacggtgaccgtaaggcttgatgaaacaacgcggcgagctttgatcaacgaccttttggaaacttcggcttcccctggagagagcgagattctccgcgctgtagaagtcaccattgttgtgcacgacgacatcattccgtggcgttatccagctaagcgcgaactgcaatttggagaatggcagcgcaatgacattcttgcaggtatcttcgagccagccacgatcgacattgatctggctatcttgctgacaaaagcaagagaacatagcgttgccttggtaggtccagcggcggaggaactctttgatccggttcctgaacaggatctatttgaggcgctaaatgaaaccttaacgctatggaactcgccgcccgactgggctggcgatgagcgaaatgtagtgcttacgttgtcccgcatttggtacagcgcagtaaccggcaaaatcgcgccgaaggatgtcgctgccgactgggcaatggagcgcctgccggcccagtatcagcccgtcatacttgaagctagacaggcttatcttggacaagaagaagatcgcttggcctcgcgcgcagatcagttggaagaatttgtccactacgtgaaaggcgagatcaccaaggtagtcggcaaataatgtctaacaattcgttcaagccgacgccgcttcgcggcgcggcttaactcaagcgttagatgcactaagcacataattgctcacagccaaactatcaggtcaagtctgcttttattatttttaagcgtgcataataagccctacacaaattgggagatatatcatgaaaggctggctttttcttgttatcgcaatagttggcgaagtaatcgcaacatccgcattaaaatctagcgagggctttactaagctgatccggtggatgaccttttgaatgacctttaatagattatattactaattaattggggaccctagaggtccccttttttattttaaaaattttttcacaaaacggtttacaagcatacgttggccgattcattaatgcagctggcacgacaggtttcccgactggaaagcgggcagtgagcgcaacgcaattaatgtgagttagctcactcattaggcaccccaggctttacactttatgcttccggctcgtatgttgtgtggaattgtgagcggataacaatttcacacaggaaacagctatgaccatgattacgccaagcttgctattgacgacagctatggttcactgtccaccaaccaaaactgtgctcagtaccgccaatatttctcccttgaggggtacaaagaggtgtccctagaagagatccacgctgtgtaaaaattttacaaaaaggtattgactttccctacagggtgtgtaataatttaattacaggcgggggcaaccccgcctgttctgcagaggaggaatatagccatggaagtgaaaatcttcaacacccaggatgttcaggattttctgcgtgttgcaagcggtctggaacaagagggtggtaatccgcgtgttaaacaaattattcatcgtgttctgagcgacctgtataaagcaattgaagatctgaatatcaccagcgacgaatattgggcaggcgttgcatatctgaatcagctgggtgcaaatcaagaagcaggtctgctgagtccgggtctgggttttgatcattatctggatatgcgtatggatgcagaagatgcagcactgggtattgaaaatgcaacaccgcgtaccattgaaggtccgctgtatgttgcgggtgcaccggaaagcgttggttatgcacgcatggatgatggtagcgatccgaatggtcataccctgattctgcatggcaccatttttgatgcagatggtaaaccgctgccgaatgcaaaagttgaaatttggcatgcaaacaccaaaggcttttatagccattttgatccgaccggtgaacagcaggcctttaatatgcgtcgtagcattattaccgatgagaatggtcagtatcgtgttcgtaccattctgcctgccggttatggttgtcctccggaaggtccgacccagcaactgctgaaccaactgggtcgtcatggtaatcgtccggcacatattcattattttgttagcgcagatggtcaccgtaaactgaccacccagattaatgttgccggtgatccgtatacctatgatgattttgcatatgccacccgtgaaggtctggttgttgatgcagttgaacataccgatccggaagcaattaaagccaatgatgtggaaggtccttttgccgaaatggtgtttgatctgaaactgacccgtctggttgatggtgttgataatcaggttgtggatcgtccgcgtctggcagtttaatacaccaaaatggttcaaaattatcaggcgagtgatcatgatcactggcctgtttttatttcagggaagggtggagacaattacgtggataatcagatcatccaagaaaccgtggataaaattctgagcgttctgccgaatcaggcaggtcagctggcacgtctggtgcgtctgatgcaatttgcatgcgatccgaccattaccgttattggcaaatataaccatggtaaaagccgtctgctgaatgaactgattggcaccgatatctttagcgttgcagataaacgtgaaaccattcagctggccgaacataaacaggatcaggttcgttggctggatgcacctggtctggatgccgatgttgcagcagttgatgatcgtcatgcatttgaagcagtttggacccaggcagatattcgtctgtttgttcatagcgttcgtgaaggtgaactggatgcaaccgaacaccatctgctgcaacagctgattgaagatgccgatcatagccgtcgtcagaccattctggttctgacccagattgatcagattccggatcagaccatcctgacacagattaaaaccagcattgcacagcaggttccgaaactggatatttgggcagttagcgcaacccgtcatcgtcagggcattgaaaacggtaaaaccctgctgatcgaaaaaagcggtattggtgcactgcgccataccctggaacaggcactggcacaggtgccgagcgcacgtacctatgaaaaaaatcgtctgctgtcagatctgcaccatcagctgaaacaactgctgctggatcagaaacatgttctgcaacaactgcaacagacacagcaacagcagctgcatgattttgataccggtctgattaacattctggacaaaattcgtgttgatctggaaccgattgtgaatattgatggtcaggatcaagcactgaatccggatagctttgcaaccatgtttaaaaacaccgcagcaaaacagcagcgtgccaaagttcagattgcatatagccgtgcatgcattgaaatcaacagccatctgattcgccatggtgttgttggtctgcctgcggaacagcagaccaccattaaaagcattgataccgtgattgttgccgtgtttggtatcagcgttaaatttcgtgatcagctgcgtgccctgttttataccgataccgaacgtcagcgtctgcaacgtgaatttcgtttctattttgaaaaaagtgccggtcgcatgattctggcagcaaaaattgaacagaccatgcgtcagcagggctgtattcagaatgccatgatggcactgcaacaaatggaaagcgcagcataaaaacacggacgccgcaaacggcgtccgaatttcttggtcgaccgttaaatctatcaccgcaagggataaatatctaacaccgtgcgtgttgactattttacctctggcggtgataatggttgcatgtactaatctagataaggaatatagccatgaccgcaccgattcaggatctgcgtgatgcaattgccctgctgcaacagcatgataatcagtatctggaaaccgatcatccggttgatccgaatgcagaactggcaggcgtttatcgtcatattggtgccggtggcaccgttaaacgtccgacccgtattggtccggcaatgatgtttaataacattaaaggttatccgcacagccgtattctggttggtatgcatgcaagccgtcagcgtgcagcactgctgctgggttgtgaagcaagtcagctggcactggaagttggtaaagcagttaaaaaaccggttgcaccggtggttgttccggcaagcagcgcaccgtgtcaagagcagatttttctggcagatgatccggattttgatctgcgtaccctgctgcctgcacataccaataccccgattgatgcaggtccgtttttttgtctgggtctggccctggcaagcgatccggtggatgcaagcctgaccgatgttaccattcatcgtctgtgtgttcagggtcgtgatgaactgagcatgttcctggcagcaggtcgccatattgaagtttttcgtcagaaagcagaagcagcaggtaaaccgctgccgattaccattaatatgggtctggacccagcaatctatattggcgcatgttttgaagcaccgaccaccccgtttggttataatgaactgggtgttgccggtgcactgcgtcagcgtccggttgaactggttcagggtgttagcgttccggaaaaagcaattgcacgtgccgaaattgttattgaaggtgaactgctgcctggtgttcgtgttcgtgaagatcagcataccaattcaggtcatgcaatgccggaatttccgggttattgtggtggtgcaaatccgagcctgccggttattaaagttaaagccgttaccatgcgcaataacgcaattctgcaaaccctggttggtccgggtgaagaacataccaccctggcaggtctgccgaccgaagcaagcatttggaatgcagttgaagcagcaattccgggttttctgcaaaatgtttatgcccataccgcaggcggtggtaaatttctgggtattctgcaagtgaaaaaacgtcagcctgccgatgaaggtcgtcagggtcaggcagccctgctggcgctggcaacctatagcgaactgaaaaatatcattctggtggatgaggatgtggacatttttgatagtgatgatattctgtgggcaatgaccacccgtatgcagggtgatgttagcattaccaccattccgggtattcgcggtcatcagctggacccgagccagacaccggaatattcaccgagcattcgtggtaatggtattagctgcaaaaccatctttgattgtaccgttccgtgggcactgaaaagccattttgaacgtgcaccgtttgcagatgttgatccgcgtccgtttgcacctgaatattttgcacgtctggaaaaaaatcagggcagcgcaaaataagctaataacaggcctgctggtaatcgcaggaatttttatttggatggatccgcctacctagcttccaagaaagatatcctaacagcacaagagcggaaagatgttttgttctacatccagaacaacctctgctaaaattcctgaaaaattttgcaaaaagttgttgactttatctacaaggtgtggtataataatcttaacaacagcaggacgctcccgggttgaggaaaacctaatgaaactgaccagcctgcgtgttagcctgctggcactgggtctggttaccagcggttttgcagcagcagaaacctataccgttgatcgttatcaggatgatagcgaaaaaggtagcctgcgttgggcaattgaacagagcaatgcaaatagcgcacaagaaaaccagattctgattcaggcagttggtaaagcaccgtatgttatcaaagttgataaaccgctgcctccgattaaaagcagcgttaaaatcattggcaccgagtgggataaaaccggtgaatttattgcaattgatggcagcaactatatcaaaggcgaaggtgaaaaagcatgtccgggtgcaaatccgggtcagtatggcaccaatgttcgtaccatgaccctgcctggtctggttctgcaagatgttaatggtgttaccctgaaaggtctggatgttcatcgtttttgtattggtgttctggttaatcgcagcagcaataacctgattcagcataatcgtatcagcaacaattatggtggtgccggtgttatgattaccggtgatgatggtaaaggtaatccgaccagcaccaccaccaataataacaaagttctggataacgtgttcatcgataatggtgatggtctggaactgacccgtggtgcagcatttaatctgattgcaaataacctgtttaccagcacaaaagccaatccggaaccgagccagggtattgaaattctgtggggtaatgataatgccgtggtgggtaacaaattcgaaaactattcagatggcctgcaaatcaattggggtaaacgtaactatatcgcctataacgaactgaccaataacagcctgggtttcaatctgacaggtgatggtaacattttcgacagcaataaagtgcatggtaaccgtattggtattgccattcgtagtgaaaaagatgccaatgcacgtattaccctgaccaaaaatcagatttgggataacggcaaagatatcaaacgttgtgaagccggtggtagctgtgttccgaatcagcgtctgggtgcaattgtttttggtgttccggcactggaacatgaaggttttgttggtagccgtggcggtggtgttgttattgaaccggcaaaactgcaaaaaacctgcacccagccgaaccagcagaattgtaatgcaattcctaatcagggtattcaggcaccgaaactgacagttagcaaaaaacagctgaccgttgaagttaaaggcacccctaatcagcgttataatgtggaattttttggcaatcgtaatgccagcagcagcgaagcagaacagtatctgggtagcattgttgttgttaccgatcatcagggtctggcaaaagcaaattgggctccgaaagttagcatgccgagcgttaccgcaaatgtgacagatcatctgggtgcgaccagcgaactgagcagcgcagttaaaatgcgttaaatgcatgcgcgccgcgttcgcgcggcgcttttttttggtaccgagctcgaattcactggccgtcgttttacaacgtcgtgactgggaaaaccctggcgttacccaacttaatcgccttgcagcacatccccctttcgccagctggcgtaatagcgaagaggcccgcaccgatcgcccttcccaacagttgcgcagcctgaatggcgaatggcgcctgatgcggtattttctccttacgcatctgtgcggtatttcacaccgcatatggtgcactctcagtacaatctgctctgatgccgcatagttaagccagccccgacacccgccaacacccgctgacgaattc

SEQ ID NO: 25 - DNA, 6452 bp, Escherichia coli
  misc_feature (1)..(6452): DNA sequence of the plasmid pMG39
gttgacagtaagacgggtaagcctgttgatgataccgctgccttactgggtgcattagccagtctgaatgacctgtcacgggataatccgaagtggtcagactggaaaatcagagggcaggaactgctgaacagcaaaaagtcagatagcaccacatagcagacccgccataaaacgccctgagaagcccgtgacgggcttttcttgtattatgggtagtttccttgcatgaatccataaaaggcgcctgtagtgccatttacccccattcactgccagagccgtgagcgcagcgaactgaatgtcacgaaaaagacagcgactcaggtgcctgatggtcggagacaaaaggaatattcagcgatttgcccgagcttgcgagggtgctacttaagcctttagggttttaaggtctgttttgtagaggagcaaacagcgtttgcgacatccttttgtaatactgcggaactgactaaagtagtgagttatacacagggctgggatctattctttttatctttttttattctttctttattctataaattataaccacttgaatataaacaaaaaaaacacacaaaggtctagcggaatttacagagggtctagcagaatttacaagttttccagcaaaggtctagcagaatttacagatacccacaactcaaaggaaaaggactagtaattatcattgactagcccatctcaattggtatagtgattaaaatcacctagaccaattgagatgtatgtctgaattagttgttttcaaagcaaatgaactagcgattagtcgctatgacttaacggagcatgaaaccaagctaattttatgctgtgtggcactactcaaccccacgattgaaaaccctacaaggaaagaacggacggtatcgttcacttataaccaatacgctcagatgatgaacatcagtagggaaaatgcttatggtgtattagctaaagcaaccagagagctgatgacgagaactgtggaaatcaggaatcctttggttaaaggctttgagattttccagtggacaaactatgccaagttctcaagcgaaaaattagaattagtttttagtgaagagatattgccttatcttttccagttaaaaaaattcataaaatataatctggaacatgttaagtcttttgaaaacaaatactctatgaggatttatgagtggttattaaaagaactaacacaaaagaaaactcacaaggcaaatatagagattagccttgatgaatttaagttcatgttaatgcttgaaaataactaccatgagtttaaaaggcttaaccaatgggttttgaaaccaataagtaaagatttaaacacttacagcaatatgaaattggtggttgataagcgaggccgcccgactgatacgttgattttccaagttgaactagatagacaaatggatctcgtaaccgaacttgagaacaaccagataaaaatgaatggtgacaaaataccaacaaccattacatcagattcctacctacgtaacggactaagaaaaacactacacgatgctttaactgcaaaaattcagctcaccagttttgaggcaaaatttttgagtgacatgcaaagtaagcatgatctcaatggttcgttctcatggctcacgcaaaaacaacgaaccacactagagaacatactggctaaatacggaaggatctgaggttcttatggctcttgtatctatcagtgaagcatcaagactaacaaacaaaagtagaacaactgttcaccgttagatatcaaagggaaaactgtccatatgcacagatgaaaacggtgtaaaaaagatagatacatcagagcttttacgagtttttggtgcatttaaagctgttcaccatgaacagatcgacaatgtaacagatgaacagcatgtaacacctaatagaacaggtgaaaccagtaaaacaaagcaactagaacatgaaattgaacacctgagacaacttgttacagctcaacagtcacacatagacagcctgaaacaggcgatgctgcttatcgaatcaaagctgccgacaacacgggagccagtgacgcctcccgtggggaaaaaatcatggcaattctggaagaaatagcgctttcagccggcaaacctgaagccggatctgcgattctgataacaaactagcaacaccagaacagcccgtttgcgggcagcaaaacccgttatgcttgtaaaccgttttgtgaaaaaatttttaaaataaaaaaggggacctctagggtccccaattaattagtaatataatctattaaaggtcattcaaaaggtcatccaccggatcaattcccctgctcgcgcaggctgggtgccaagctctcgggtaacatcaaggcccgatccttggagcccttgccctcccgcacgatgatcgtgccgtgatcgaaatccagatccttgacccgcagttgcaaaccctcactgatccgcatgcccgttccatacagaagctgggcgaacaaacgatgctcgccttccagaaaaccgaggatgcgaaccacttcatccggggtcagcaccaccggcaagcgccgcgacggccgaggtcttccgatctcctgaagccagggcagatccgtgcacagcaccttgccgtagaagaacagcaaggccgccaatgcctgacgatgcgtggagaccgaaaccttgcgctcgttcgccagccaggacagaaatgcctcgacttcgctgctgcccaaggttgccgggtgacgcacaccgtggaaacggatgaaggcacgaacccagtggacataagcctgttcggttcgtaagctgtaatgcaagtagcgtatgcgctcacgcaactggtccagaaccttgaccgaacgcagcggtggtaacggcgcagtggcggttttcatggcttgttatgactgtttttttggggtacagtctatgcctcgggcatccaagcagcaagcgcgttacgccgtgggtcgatgtttgatgttatggagcagcaacgatgttacgcagcagggcagtcgccctaaaacaaagttaaacatcatgagggaagcggtgatcgccgaagtatcgactcaactatcagaggtagttggcgtcatcgagcgccatctcgaaccgacgttgctggccgtacatttgtacggctccgcagtggatggcggcctgaagccacacagtgatattgatttgctggttacggtgaccgtaaggcttgatgaaacaacgcggcgagctttgatcaacgaccttttggaaacttcggcttcccctggagagagcgagattctccgcgctgtagaagtcaccattgttgtgcacgacgacatcattccgtggcgttatccagctaagcgcgaactgcaatttggagaatggcagcgcaatgacattcttgcaggtatcttcgagccagccacgatcgacattgatctggctatcttgctgacaaaagcaagagaacatagcgttgccttggtaggtccagcggcggaggaactctttgatccggttcctgaacaggatctatttgaggcgctaaatgaaaccttaacgctatggaactcgccgcccgactgggctggcgatgagcgaaatgtagtgcttacgttgtcccgcatttggtacagcgcagtaaccggcaaaatcgcgccgaaggatgtcgctgccgactgggcaatggagcgcctgccggcccagtatcagcccgtcatacttgaagctagacaggcttatcttggacaagaagaagatcgcttggcctcgcgcgcagatcagttggaagaatttgtccactacgtgaaaggcgagatcaccaaggtagtcggcaaataatgtctaacaattcgttcaagccgacgccgcttcgcggcgcggcttaactcaagcgttagatgcactaagcacataattgctcacagccaaactatcaggtcaagtctgcttttattatttttaagcgtgcataataagccctacacaaattgggagatatatcatgaaaggctggctttttcttgttatcgcaatagttggcgaagtaatcgcaacatccgcattaaaatctagcgagggctttactaagctgatccggtggatgaccttttgaatgacctttaatagattatattactaattaattggggaccctagaggtccccttttttattttaaaaattttttcacaaaacggtttacaagcatacgttggccgattcattaatgcagctggcacgacaggtttcccgactggaaagcgggcagtgagcgcaacgcaattaatgtgagttagctcactcattaggcaccccaggctttacactttatgcttccggctcgtatgttgtgtggaattgtgagcggataacaatttcacacaggaaacagctatgaccatgattacgccaagcttgcatgcctgcaggtcgactctagaggatccgcctacctagcttccaagaaagatatcctaacagcacaagagcggaaagatgttttgttctacatccagaacaacctctgctaaaattcctgaaaaattttgcaaaaagttgttgactttatctacaaggtgtggtataataatcttaacaacagcaggacgctcccgggttgaggaaaacctaatgaaactgaccagcctgcgtgttagcctgctggcactgggtctggttaccagcggttttgcagcagcagaaacctataccgttgatcgttatcaggatgatagcgaaaaaggtagcctgcgttgggcaattgaacagagcaatgcaaatagcgcacaagaaaaccagattctgattcaggcagttggtaaagcaccgtatgttatcaaagttgataaaccgctgcctccgattaaaagcagcgttaaaatcattggcaccgagtgggataaaaccggtgaatttattgcaattgatggcagcaactatatcaaaggcgaaggtgaaaaagcatgtccgggtgcaaatccgggtcagtatggcaccaatgttcgtaccatgaccctgcctggtctggttctgcaagatgttaatggtgttaccctgaaaggtctggatgttcatcgtttttgtattggtgttctggttaatcgcagcagcaataacctgattcagcataatcgtatcagcaacaattatggtggtgccggtgttatgattaccggtgatgatggtaaaggtaatccgaccagcaccaccaccaataataacaaagttctggataacgtgttcatcgataatggtgatggtctggaactgacccgtggtgcagcatttaatctgattgcaaataacctgtttaccagcacaaaagccaatccggaaccgagccagggtattgaaattctgtggggtaatgataatgccgtggtgggtaacaaattcgaaaactattcagatggcctgcaaatcaattggggtaaacgtaactatatcgcctataacgaactgaccaataacagcctgggtttcaatctgacaggtgatggtaacattttcgacagcaataaagtgcatggtaaccgtattggtattgccattcgtagtgaaaaagatgccaatgcacgtattaccctgaccaaaaatcagatttgggataacggcaaagatatcaaacgttgtgaagccggtggtagctgtgttccgaatcagcgtctgggtgcaattgtttttggtgttccggcactggaacatgaaggttttgttggtagccgtggcggtggtgttgttattgaaccggcaaaactgcaaaaaacctgcacccagccgaaccagcagaattgtaatgcaattcctaatcagggtattcaggcaccgaaactgacagttagcaaaaaacagctgaccgttgaagttaaaggcacccctaatcagcgttataatgtggaattttttggcaatcgtaatgccagcagcagcgaagcagaacagtatctgggtagcattgttgttgttaccgatcatcagggtctggcaaaagcaaattgggctccgaaagttagcatgccgagcgttaccgcaaatgtgacagatcatctgggtgcgaccagcgaactgagcagcgcagttaaaatgcgttaaatgcatgcgcgccgcgttcgcgcggcgcttttttttggtaccgagctcgaattcactggccgtcgttttacaacgtcgtgactgggaaaaccctggcgttacccaacttaatcgccttgcagcacatccccctttcgccagctggcgtaatagcgaagaggcccgcaccgatcgcccttcccaacagttgcgcagcctgaatggcgaatggcgcctgatgcggtattttctccttacgcatctgtgcggtatttcacaccgcatatggtgcactctcagtacaatctgctctgatgccgcatagttaagccagccccgacacccgccaacacccgctgacgaattc

SEQ ID NO: 26 - DNA, 10012 bp, Escherichia coli
  misc_feature (1)..(10012): DNA sequence of the plasmid pMG47
gttgacagtaagacgggtaagcctgttgatgataccgctgccttactgggtgcattagccagtctgaatgacctgtcacgggataatccgaagtggtcagactggaaaatcagagggcaggaactgctgaacagcaaaaagtcagatagcaccacatagcagacccgccataaaacgccctgagaagcccgtgacgggcttttcttgtattatgggtagtttccttgcatgaatccataaaaggcgcctgtagtgccatttacccccattcactgccagagccgtgagcgcagcgaactgaatgtcacgaaaaagacagcgactcaggtgcctgatggtcggagacaaaaggaatattcagcgatttgcccgagcttgcgagggtgctacttaagcctttagggttttaaggtctgttttgtagaggagcaaacagcgtttgcgacatccttttgtaatactgcggaactgactaaagtagtgagttatacacagggctgggatctattctttttatctttttttattctttctttattctataaattataaccacttgaatataaacaaaaaaaacacacaaaggtctagcggaatttacagagggtctagcagaatttacaagttttccagcaaaggtctagcagaatttacagatacccacaactcaaaggaaaaggactagtaattatcattgactagcccatctcaattggtatagtgattaaaatcacctagaccaattgagatgtatgtctgaattagttgttttcaaagcaaatgaactagcgattagtcgctatgacttaacggagcatgaaaccaagctaattttatgctgtgtggcactactcaaccccacgattgaaaaccctacaaggaaagaacggacggtatcgttcacttataaccaatacgctcagatgatgaacatcagtagggaaaatgcttatggtgtattagctaaagcaaccagagagctgatgacgagaactgtggaaatcaggaatcctttggttaaaggctttgagattttccagtggacaaactatgccaagttctcaagcgaaaaattagaattagtttttagtgaagagatattgccttatcttttccagttaaaaaaattcataaaatataatctggaacatgttaagtcttttgaaaacaaatactctatgaggatttatgagtggttattaaaagaactaacacaaaagaaaactcacaaggcaaatatagagattagccttgatgaatttaagttcatgttaatgcttgaaaataactaccatgagtttaaaaggcttaaccaatgggttttgaaaccaataagtaaagatttaaacacttacagcaatatgaaattggtggttgataagcgaggccgcccgactgatacgttgattttccaagttgaactagatagacaaatggatctcgtaaccgaacttgagaacaaccagataaaaatgaatggtgacaaaataccaacaaccattacatcagattcctacctacgtaacggactaagaaaaacactacacgatgctttaactgcaaaaattcagctcaccagttttgaggcaaaatttttgagtgacatgcaaagtaagcatgatctcaatggttcgttctcatggctcacgcaaaaacaacgaaccacactagagaacatactggctaaatacggaaggatctgaggttcttatggctcttgtatctatcagtgaagcatcaagactaacaaacaaaagtagaacaactgttcaccgttagatatcaaagggaaaactgtccatatgcacagatgaaaacggtgtaaaaaagatagatacatcagagcttttacgagtttttggtgcatttaaagctgttcaccatgaacagatcgacaatgtaacagatgaacagcatgtaacacctaatagaacaggtgaaaccagtaaaacaaagcaactagaacatgaaattgaacacctgagacaacttgttacagctcaacagtcacacatagacagcctgaaacaggcgatgctgcttatcgaatcaaagctgccgacaacacgggagccagtgacgcctcccgtggggaaaaaatcatggcaattctggaagaaatagcgctttcagccggcaaacctgaagccggatctgcgattctgataacaaactagcaacaccagaacagcccgtttgcgggcagcaaaacccgttatgcttgtaaaccgttttgtgaaaaaatttttaaaataaaaaaggggacctctagggtccccaattaattagtaatataatctattaaaggtcattcaaaaggtcatccaccggatcaattcccctgctcgcgcaggctgggtgccaagctctcgggtaacatcaaggcccgatccttggagcccttgccctcccgcacgatgatcgtgccgtgatcgaaatccagatccttgacccgcagttgcaaaccctcactgatccgcatgcccgttccatacagaagctgggcgaacaaacgatgctcgccttccagaaaaccgaggatgcgaaccacttcatccggggtcagcaccaccggcaagcgccgcgacggccgaggtcttccgatctcctgaagccagggcagatccgtgcacagcaccttgccgtagaagaacagcaaggccgccaatgcctgacgatgcgtggagaccgaaaccttgcgctcgttcgccagccaggacagaaatgcctcgacttcgctgctgcccaaggttgccgggtgacgcacaccgtggaaacggatgaaggcacgaacccagtggacataagcctgttcggttcgtaagctgtaatgcaagtagcgtatgcgctcacgcaactggtccagaaccttgaccgaacgcagcggtggtaacggcgcagtggcggttttcatggcttgttatgactgtttttttggggtacagtctatgcctcgggcatccaagcagcaagcgcgttacgccgtgggtcgatgtttgatgttatggagcagcaacgatgttacgcagcagggcagtcgccctaaaacaaagttaaacatcatgagggaagcggtgatcgccgaagtatcgactcaactatcagaggtagttggcgtcatcgagcgccatctcgaaccgacgttgctggccgtacatttgtacggctccgcagtggatggcggcctgaagccacacagtgatattgatttgctggttacggtgaccgtaaggcttgatgaaacaacgcggcgagctttgatcaacgaccttttggaaacttcggcttcccctggagagagcgagattctccgcgctgtagaagtcaccattgttgtgcacgacgacatcattccgtggcgttatccagctaagcgcgaactgcaatttggagaatggcagcgcaatgacattcttgcaggtatcttcgagccagccacgatcgacattgatctggctatcttgctgacaaaagcaagagaacatagcgttgccttggtaggtccagcggcggaggaactctttgatccggttcctgaacaggatctatttgaggcgctaaatgaaaccttaacgctatggaactcgccgcccgactgggctggcgatgagcgaaatgtagtgcttacgttgtcccgcatttggtacagcgcagtaaccggcaaaatcgcgccgaaggatgtcgctgccgactgggcaatggagcgcctgccggcccagtatcagcccgtcatacttgaagctagacaggcttatcttggacaagaagaagatcgcttggcctcgcgcgcagatcagttggaagaatttgtccactacgtgaaaggcgagatcaccaaggtagtcggcaaataatgtctaacaattcgttcaagccgacgccgcttcgcggcgcggcttaactcaagcgttagatgcactaagcacataattgctcacagccaaactatcaggtcaagtctgcttttattatttttaagcgtgcataataagccctacacaaattgggagatatatcatgaaaggctggctttttcttgttatcgcaatagttggcgaagtaatcgcaacatccgcattaaaatctagcgagggctttactaagctgatccggtggatgaccttttgaatgacctttaatagattatattactaattaattggggaccctagaggtccccttttttattttaaaaattttttcacaaaacggtttacaagcatacgttggccgattcattaatgcagctggcacgacaggtttcccgactggaaagcgggcagtgagcgcaacgcaattaatgtgagttagctcactcattaggcaccccaggctttacactttatgcttccggctcgtatgttgtgtggaattgtgagcggataacaatttcacacaggaaacagctatgaccatgattacgccaagcttgctattgacgacagctatggttcactgtccaccaaccaaaactgtgctcagtaccgccaatatttctcccttgaggggtacaaagaggtgtccctagaagagatccacgctgtgtaaaaattttacaaaaaggtattgactttccctacagggtgtgtaataatttaattacaggcgggggcaaccccgcctgttctgcagaggaggaatatagccatggaagtgaaaatcttcaacacccaggatgttcaggattttctgcgtgttgcaagcggtctggaacaagagggtggtaatccgcgtgttaaacaaattattcatcgtgttctgagcgacctgtataaagcaattgaagatctgaatatcaccagcgacgaatattgggcaggcgttgcatatctgaatcagctgggtgcaaatcaagaagcaggtctgctgagtccgggtctgggttttgatcattatctggatatgcgtatggatgcagaagatgcagcactgggtattgaaaatgcaacaccgcgtaccattgaaggtccgctgtatgttgcgggtgcaccggaaagcgttggttatgcacgcatggatgatggtagcgatccgaatggtcataccctgattctgcatggcaccatttttgatgcagatggtaaaccgctgccgaatgcaaaagttgaaatttggcatgcaaacaccaaaggcttttatagccattttgatccgaccggtgaacagcaggcctttaatatgcgtcgtagcattattaccgatgagaatggtcagtatcgtgttcgtaccattctgcctgccggttatggttgtcctccggaaggtccgacccagcaactgctgaaccaactgggtcgtcatggtaatcgtccggcacatattcattattttgttagcgcagatggtcaccgtaaactgaccacccagattaatgttgccggtgatccgtatacctatgatgattttgcatatgccacccgtgaaggtctggttgttgatgcagttgaacataccgatccggaagcaattaaagccaatgatgtggaaggtccttttgccgaaatggtgtttgatctgaaactgacccgtctggttgatggtgttgataatcaggttgtggatcgtccgcgtctggcagtttaatacaccaaaatggttcaaaattatcaggcgagtgatcatgatcactggcctgtttttatttcagggaagggtggagacaattacgtggataatcagatcatccaagaaaccgtggataaaattctgagcgttctgccgaatcaggcaggtcagctggcacgtctggtgcgtctgatgcaatttgcatgcgatccgaccattaccgttattggcaaatataaccatggtaaaagccgtctgctgaatgaactgattggcaccgatatctttagcgttgcagataaacgtgaaaccattcagctggccgaacataaacaggatcaggttcgttggctggatgcacctggtctggatgccgatgttgcagcagttgatgatcgtcatgcatttgaagcagtttggacccaggcagatattcgtctgtttgttcatagcgttcgtgaaggtgaactggatgcaaccgaacaccatctgctgcaacagctgattgaagatgccgatcatagccgtcgtcagaccattctggttctgacccagattgatcagattccggatcagaccatcctgacacagattaaaaccagcattgcacagcaggttccgaaactggatatttgggcagttagcgcaacccgtcatcgtcagggcattgaaaacggtaaaaccctgctgatcgaaaaaagcggtattggtgcactgcgccataccctggaacaggcactggcacaggtgccgagcgcacgtacctatgaaaaaaatcgtctgctgtcagatctgcaccatcagctgaaacaactgctgctggatcagaaacatgttctgcaacaactgcaacagacacagcaacagcagctgcatgattttgataccggtctgattaacattctggacaaaattcgtgttgatctggaaccgattgtgaatattgatggtcaggatcaagcactgaatccggatagctttgcaaccatgtttaaaaacaccgcagcaaaacagcagcgtgccaaagttcagattgcatatagccgtgcatgcattgaaatcaacagccatctgattcgccatggtgttgttggtctgcctgcggaacagcagaccaccattaaaagcattgataccgtgattgttgccgtgtttggtatcagcgttaaatttcgtgatcagctgcgtgccctgttttataccgataccgaacgtcagcgtctgcaacgtgaatttcgtttctattttgaaaaaagtgccggtcgcatgattctggcagcaaaaattgaacagaccatgcgtcagcagggctgtattcagaatgccatgatggcactgcaacaaatggaaagcgcagcataaaaacacggacgccgcaaacggcgtccgaatttcttggtcgaccgttaaatctatcaccgcaagggataaatatctaacaccgtgcgtgttgactattttacctctggcggtgataatggttgcatgtactaatctagataaggaatatagccatgaccgcaccgattcaggatctgcgtgatgcaattgccctgctgcaacagcatgataatcagtatctggaaaccgatcatccggttgatccgaatgcagaactggcaggcgtttatcgtcatattggtgccggtggcaccgttaaacgtccgacccgtattggtccggcaatgatgtttaataacattaaaggttatccgcacagccgtattctggttggtatgcatgcaagccgtcagcgtgcagcactgctgctgggttgtgaagcaagtcagctggcactggaagttggtaaagcagttaaaaaaccggttgcaccggtggttgttccggcaagcagcgcaccgtgtcaagagcagatttttctggcagatgatccggattttgatctgcgtaccctgctgcctgcacataccaataccccgattgatgcaggtccgtttttttgtctgggtctggccctggcaagcgatccggtggatgcaagcctgaccgatgttaccattcatcgtctgtgtgttcagggtcgtgatgaactgagcatgttcctggcagcaggtcgccatattgaagtttttcgtcagaaagcagaagcagcaggtaaaccgctgccgattaccattaatatgggtctggacccagcaatctatattggcgcatgttttgaagcaccgaccaccccgtttggttataatgaactgggtgttgccggtgcactgcgtcagcgtccggttgaactggttcagggtgttagcgttccggaaaaagcaattgcacgtgccgaaattgttattgaaggtgaactgctgcctggtgttcgtgttcgtgaagatcagcataccaattcaggtcatgcaatgccggaatttccgggttattgtggtggtgcaaatccgagcctgccggttattaaagttaaagccgttaccatgcgcaataacgcaattctgcaaaccctggttggtccgggtgaagaacataccaccctggcaggtctgccgaccgaagcaagcatttggaatgcagttgaagcagcaattccgggttttctgcaaaatgtttatgcccataccgcaggcggtggtaaatttctgggtattctgcaagtgaaaaaacgtcagcctgccgatgaaggtcgtcagggtcaggcagccctgctggcgctggcaacctatagcgaactgaaaaatatcattctggtggatgaggatgtggacatttttgatagtgatgatattctgtgggcaatgaccacccgtatgcagggtgatgttagcattaccaccattccgggtattcgcggtcatcagctggacccgagccagacaccggaatattcaccgagcattcgtggtaatggtattagctgcaaaaccatctttgattgtaccgttccgtgggcactgaaaagccattttgaacgtgcaccgtttgcagatgttgatccgcgtccgtttgcacctgaatattttgcacgtctggaaaaaaatcagggcagcgcaaaataagctaataacaggcctgctggtaatcgcaggaatttttatttggatggatccgcctacctagcttccaagaaagatatcctaacagcacaagagcggaaagatgttttgttctacatccagaacaacctctgctaaaattcctgaaaaattttgcaaaaagttgttgactttatctacaaggtgtggtataataatcttaacaacagcaggacgctcccgggttgaggaaaacctaatgaaatatagcctgtgcaccattagctttcgtcaccagctgattagctttaccgatattgttcagtttgcctatgaaaacggctttgaaggtattgaactgtggggcacccatgcacagaatctgtatatgcaagaatatgaaaccaccgaacgtgaactgaattgcctgaaagataaaaccctggaaattaccatgatcagcgattatctggatattagcctgagcgcagattttgaaaaaaccatcgaaaaatgtgaacagctggcaattctggccaattggtttaaaacgaacaaaattcgtacctttgccggtcagaaaggtagtgcagattttagccagcaagaacgtcaagagtatgtgaatcgtattcgcatgatttgtgaactgtttgcccagcataatatgtatgttctgctggaaacccatccgaataccctgaccgataccctgccgagcaccctggaactgctgggtgaagttgatcatccgaatctgaaaatcaacctggattttctgcatatctgggaaagcggtgcagatccggttgatagctttcagcagctgcgtccgtggattcagcattatcactttaaaaacattagcagcgcagactatctgcatgtgtttgaaccgaataatgtttatgcagcagcaggtaatcgtaccggtatggttccgctgtttgaaggcattgttaactatgatgaaatcatccaagaagtgcgcgataccgatcattttgcaagcctggaatggtttggtcataacgcaaaagatattctgaaagccgaaatgaaagtgctgaccaatcgtaatctggaagttgttaccagctaaatgcatgcgcgccgcgttcgcgcggcgcttttttttggtaccgagctcgaattcactggccgtcgttttacaacgtcgtgactgggaaaaccctggcgttacccaacttaatcgccttgcagcacatccccctttcgccagctggcgtaatagcgaagaggcccgcaccgatcgcccttcccaacagttgcgcagcctgaatggcgaatggcgcctgatgcggtattttctccttacgcatctgtgcggtatttcacaccgcatatggtgcactctcagtacaatctgctctgatgccgcatagttaagccagccccgacacccgccaacacccgctgacgaattc

SEQ ID NO: 27 - DNA, 10249 bp, Escherichia coli
  misc_feature (1)..(10249): DNA sequence of the plasmid pMG70
gttgacagtaagacgggtaagcctgttgatgataccgctgccttactgggtgcattagccagtctgaatgacctgtcacgggataatccgaagtggtcagactggaaaatcagagggcaggaactgctgaacagcaaaaagtcagatagcaccacatagcagacccgccataaaacgccctgagaagcccgtgacgggcttttcttgtattatgggtagtttccttgcatgaatccataaaaggcgcctgtagtgccatttacccccattcactgccagagccgtgagcgcagcgaactgaatgtcacgaaaaagacagcgactcaggtgcctgatggtcggagacaaaaggaatattcagcgatttgcccgagcttgcgagggtgctacttaagcctttagggttttaaggtctgttttgtagaggagcaaacagcgtttgcgacatccttttgtaatactgcggaactgactaaagtagtgagttatacacagggctgggatctattctttttatctttttttattctttctttattctataaattataaccacttgaatataaacaaaaaaaacacacaaaggtctagcggaatttacagagggtctagcagaatttacaagttttccagcaaaggtctagcagaatttacagatacccacaactcaaaggaaaaggactagtaattatcattgactagcccatctcaattggtatagtgattaaaatcacctagaccaattgagatgtatgtctgaattagttgttttcaaagcaaatgaactagcgattagtcgctatgacttaacggagcatgaaaccaagctaattttatgctgtgtggcactactcaaccccacgattgaaaaccctacaaggaaagaacggacggtatcgttcacttataaccaatacgctcagatgatgaacatcagtagggaaaatgcttatggtgtattagctaaagcaaccagagagctgatgacgagaactgtggaaatcaggaatcctttggttaaaggctttgagattttccagtggacaaactatgccaagttctcaagcgaaaaattagaattagtttttagtgaagagatattgccttatcttttccagttaaaaaaattcataaaatataatctggaacatgttaagtcttttgaaaacaaatactctatgaggatttatgagtggttattaaaagaactaacacaaaagaaaactcacaaggcaaatatagagattagccttgatgaatttaagttcatgttaatgcttgaaaataactaccatgagtttaaaaggcttaaccaatgggttttgaaaccaataagtaaagatttaaacacttacagcaatatgaaattggtggttgataagcgaggccgcccgactgatacgttgattttccaagttgaactagatagacaaatggatctcgtaaccgaacttgagaacaaccagataaaaatgaatggtgacaaaataccaacaaccattacatcagattcctacctacgtaacggactaagaaaaacactacacgatgctttaactgcaaaaattcagctcaccagttttgaggcaaaatttttgagtgacatgcaaagtaagcatgatctcaatggttcgttctcatggctcacgcaaaaacaacgaaccacactagagaacatactggctaaatacggaaggatctgaggttcttatggctcttgtatctatcagtgaagcatcaagactaacaaacaaaagtagaacaactgttcaccgttagatatcaaagggaaaactgtccatatgcacagatgaaaacggtgtaaaaaagatagatacatcagagcttttacgagtttttggtgcatttaaagctgttcaccatgaacagatcgacaatgtaacagatgaacagcatgtaacacctaatagaacaggtgaaaccagtaaaacaaagcaactagaacatgaaattgaacacctgagacaacttgttacagctcaacagtcacacatagacagcctgaaacaggcgatgctgcttatcgaatcaaagctgccgacaacacgggagccagtgacgcctcccgtggggaaaaaatcatggcaattctggaagaaatagcgctttcagccggcaaacctgaagccggatctgcgattctgataacaaactagcaacaccagaacagcccgtttgcgggcagcaaaacccgttatgcttgtaaaccgttttgtgaaaaaatttttaaaataaaaaaggggacctctagggtccccaattaattagtaatataatctattaaaggtcattcaaaaggtcatccaccggatcaattcccctgctcgcgcaggctgggtgccaagctctcgggtaacatcaaggcccgatccttggagcccttgccctcccgcacgatgatcgtgccgtgatcgaaatccagatccttgacccgcagttgcaaaccctcactgatccgcatgcccgttccatacagaagctgggcgaacaaacgatgctcgccttccagaaaaccgaggatgcgaaccacttcatccggggtcagcaccaccggcaagcgccgcgacggccgaggtcttccgatctcctgaagccagggcagatccgtgcacagcaccttgccgtagaagaacagcaaggccgccaatgcctgacgatgcgtggagaccgaaaccttgcgctcgttcgccagccaggacagaaatgcctcgacttcgctgctgcccaaggttgccgggtgacgcacaccgtggaaacggatgaaggcacgaacccagtggacataagcctgttcggttcgtaagctgtaatgcaagtagcgtatgcgctcacgcaactggtccagaaccttgaccgaacgcagcggtggtaacggcgcagtggcggttttcatggcttgttatgactgtttttttggggtacagtctatgcctcgggcatccaagcagcaagcgcgttacgccgtgggtcgatgtttgatgttatggagcagcaacgatgttacgcagcagggcagtcgccctaaaacaaagttaaacatcatgagggaagcggtgatcgccgaagtatcgactcaactatcagaggtagttggcgtcatcgagcgccatctcgaaccgacgttgctggccgtacatttgtacggctccgcagtggatggcggcctgaagccacacagtgatattgatttgctggttacggtgaccgtaaggcttgatgaaacaacgcggcgagctttgatcaacgaccttttggaaacttcggcttcccctggagagagcgagattctccgcgctgtagaagtcaccattgttgtgcacgacgacatcattccgtggcgttatccagctaagcgcgaactgcaatttggagaatggcagcgcaatgacattcttgcaggtatcttcgagccagccacgatcgacattgatctggctatcttgctgacaaaagcaagagaacatagcgttgccttggtaggtccagcggcggaggaactctttgatccggttcctgaacaggatctatttgaggcgctaaatgaaaccttaacgctatggaactcgccgcccgactgggctggcgatgagcgaaatgtagtgcttacgttgtcccgcatttggtacagcgcagtaaccggcaaaatcgcgccgaaggatgtcgctgccgactgggcaatggagcgcctgccggcccagtatcagcccgtcatacttgaagctagacaggcttatcttggacaagaagaagatcgcttggcctcgcgcgcagatcagttggaagaatttgtccactacgtgaaaggcgagatcaccaaggtagtcggcaaataatgtctaacaattcgttcaagccgacgccgcttcgcggcgcggcttaactcaagcgttagatgcactaagcacataattgctcacagccaaactatcaggtcaagtctgcttttattatttttaagcgtgcataataagccctacacaaattgggagatatatcatgaaaggctggctttttcttgttatcgcaatagttggcgaagtaatcgcaacatccgcattaaaatctagcgagggctttactaagctgatccggtggatgaccttttgaatgacctttaatagattatattactaattaattggggaccctagaggtccccttttttattttaaaaattttttcacaaaacggtttacaagcatacgttggccgattcattaatgcagctggcacgacaggtttcccgactggaaagcgggcagtgagcgcaacgcaattaatgtgagttagctcactcattaggcaccccaggctttacactttatgcttccggctcgtatgttgtgtggaattgtgagcggataacaatttcacacaggaaacagctatgaccatgattacgccaagcttgctattgacgacagctatggttcactgtccaccaaccaaaactgtgctcagtaccgccaatatttctcccttgaggggtacaaagaggtgtccctagaagagatccacgctgtgtaaaaattttacaaaaaggtattgactttccctacagggtgtgtaataatttaattacaggcgggggcaaccccgcctgttctgcagaggaggaatatagccatggaagtgaaaatcttcaacacccaggatgttcaggattttctgcgtgttgcaagcggtctggaacaagagggtggtaatccgcgtgttaaacaaattattcatcgtgttctgagcgacctgtataaagcaattgaagatctgaatatcaccagcgacgaatattgggcaggcgttgcatatctgaatcagctgggtgcaaatcaagaagcaggtctgctgagtccgggtctgggttttgatcattatctggatatgcgtatggatgcagaagatgcagcactgggtattgaaaatgcaacaccgcgtaccattgaaggtccgctgtatgttgcgggtgcaccggaaagcgttggttatgcacgcatggatgatggtagcgatccgaatggtcataccctgattctgcatggcaccatttttgatgcagatggtaaaccgctgccgaatgcaaaagttgaaatttggcatgcaaacaccaaaggcttttatagccattttgatccgaccggtgaacagcaggcctttaatatgcgtcgtagcattattaccgatgagaatggtcagtatcgtgttcgtaccattctgcctgccggttatggttgtcctccggaaggtccgacccagcaactgctgaaccaactgggtcgtcatggtaatcgtccggcacatattcattattttgttagcgcagatggtcaccgtaaactgaccacccagattaatgttgccggtgatccgtatacctatgatgattttgcatatgccacccgtgaaggtctggttgttgatgcagttgaacataccgatccggaagcaattaaagccaatgatgtggaaggtccttttgccgaaatggtgtttgatctgaaactgacccgtctggttgatggtgttgataatcaggttgtggatcgtccgcgtctggcagtttaatacaccaaaatggttcaaaattatcaggcgagtgatcatgatcactggcctgtttttatttcagggaagggtggagacaattacgtggataatcagatcatccaagaaaccgtggataaaattctgagcgttctgccgaatcaggcaggtcagctggcacgtctggtgcgtctgatgcaatttgcatgcgatccgaccattaccgttattggcaaatataaccatggtaaaagccgtctgctgaatgaactgattggcaccgatatctttagcgttgcagataaacgtgaaaccattcagctggccgaacataaacaggatcaggttcgttggctggatgcacctggtctggatgccgatgttgcagcagttgatgatcgtcatgcatttgaagcagtttggacccaggcagatattcgtctgtttgttcatagcgttcgtgaaggtgaactggatgcaaccgaacaccatctgctgcaacagctgattgaagatgccgatcatagccgtcgtcagaccattctggttctgacccagattgatcagattccggatcagaccatcctgacacagattaaaaccagcattgcacagcaggttccgaaactggatatttgggcagttagcgcaacccgtcatcgtcagggcattgaaaacggtaaaaccctgctgatcgaaaaaagcggtattggtgcactgcgccataccctggaacaggcactggcacaggtgccgagcgcacgtacctatgaaaaaaatcgtctgctgtcagatctgcaccatcagctgaaacaactgctgctggatcagaaacatgttctgcaacaactgcaacagacacagcaacagcagctgcatgattttgataccggtctgattaacattctggacaaaattcgtgttgatctggaaccgattgtgaatattgatggtcaggatcaagcactgaatccggatagctttgcaaccatgtttaaaaacaccgcagcaaaacagcagcgtgccaaagttcagattgcatatagccgtgcatgcattgaaatcaacagccatctgattcgccatggtgttgttggtctgcctgcggaacagcagaccaccattaaaagcattgataccgtgattgttgccgtgtttggtatcagcgttaaatttcgtgatcagctgcgtgccctgttttataccgataccgaacgtcagcgtctgcaacgtgaatttcgtttctattttgaaaaaagtgccggtcgcatgattctggcagcaaaaattgaacagaccatgcgtcagcagggctgtattcagaatgccatgatggcactgcaacaaatggaaagcgcagcataaaaacacggacgccgcaaacggcgtccgaatttcttggtcgaccgttaaatctatcaccgcaagggataaatatctaacaccgtgcgtgttgactattttacctctggcggtgataatggttgcatgtactaatctagataaggaatatagccatgaccgcaccgattcaggatctgcgtgatgcaattgccctgctgcaacagcatgataatcagtatctggaaaccgatcatccggttgatccgaatgcagaactggcaggcgtttatcgtcatattggtgccggtggcaccgttaaacgtccgacccgtattggtccggcaatgatgtttaataacattaaaggttatccgcacagccgtattctggttggtatgcatgcaagccgtcagcgtgcagcactgctgctgggttgtgaagcaagtcagctggcactggaagttggtaaagcagttaaaaaaccggttgcaccggtggttgttccggcaagcagcgcaccgtgtcaagagcagatttttctggcagatgatccggattttgatctgcgtaccctgctgcctgcacataccaataccccgattgatgcaggtccgtttttttgtctgggtctggccctggcaagcgatccggtggatgcaagcctgaccgatgttaccattcatcgtctgtgtgttcagggtcgtgatgaactgagcatgttcctggcagcaggtcgccatattgaagtttttcgtcagaaagcagaagcagcaggtaaaccgctgccgattaccattaatatgggtctggacccagcaatctatattggcgcatgttttgaagcaccgaccaccccgtttggttataatgaactgggtgttgccggtgcactgcgtcagcgtccggttgaactggttcagggtgttagcgttccggaaaaagcaattgcacgtgccgaaattgttattgaaggtgaactgctgcctggtgttcgtgttcgtgaagatcagcataccaattcaggtcatgcaatgccggaatttccgggttattgtggtggtgcaaatccgagcctgccggttattaaagttaaagccgttaccatgcgcaataacgcaattctgcaaaccctggttggtccgggtgaagaacataccaccctggcaggtctgccgaccgaagcaagcatttggaatgcagttgaagcagcaattccgggttttctgcaaaatgtttatgcccataccgcaggcggtggtaaatttctgggtattctgcaagtgaaaaaacgtcagcctgccgatgaaggtcgtcagggtcaggcagccctgctggcgctggcaacctatagcgaactgaaaaatatcattctggtggatgaggatgtggacatttttgatagtgatgatattctgtgggcaatgaccacccgtatgcagggtgatgttagcattaccaccattccgggtattcgcggtcatcagctggacccgagccagacaccggaatattcaccgagcattcgtggtaatggtattagctgcaaaaccatctttgattgtaccgttccgtgggcactgaaaagccattttgaacgtgcaccgtttgcagatgttgatccgcgtccgtttgcacctgaatattttgcacgtctggaaaaaaatcagggcagcgcaaaataagctaataacaggcctgctggtaatcgcaggaatttttatttggatggatccgcctacctagcttccaagaaagatatcctaacagcacaagagcggaaagatgttttgttctacatccagaacaacctctgctaaaattcctgaaaaattttgcaaaaagttgttgactttatctacaaggtgtggtataataatcttaacaacagcaggacgctcccgggttgaggaaaacctaatgccgagcaaactggcaattagcagcatgagcctgggtcgttgttttgcaggtcatagcctggatagtaaactggatgcagcacagcgttatggttatctgggtattgaactgttttatgaggatctggttgatgttgcagaacatctgagcaatgaacgtccgagtccggaaggtccgtttgttgaagcacagattgcagcagcacgtcatattctgcaaatgtgtcaggcacgtggtctggaagttgtttgtctgcaaccgtttatgcattatgatggtctgaatgatcgtgccgaacatgaacgtcgtctggaaaaactggcactgtggattgaactggcacatgaactgcataccgatattattcagattccggcaaattttctgcctgcaaatcaggttagcgataatctggatctgattgttagcgatctgtgtaaagttgcagatattggtgcacaggcactgcctccgattcgttttgcatatgaaagcctgtgttggagcacccgtgttgatctgtgggaacgttgttgggatattgttcagcgtgtggatcgtccgaattttggtatttgtctggatacctttaacatcctgggtcgcatttatgcagatccgaccagcccgagcggtcgtaccccgaatgcaaaagaagcagttcgtaaaagcattgccaatctggttagccgtgtggatgttagcaaagttttttatgttcaggttgtggatgccgaacgtctgagtaaaccgctgctgcctggtcatccgtattataacccggaacagcctgcacgtatgagctggtcacgtaattgtcgtctgttctatggtgaaaccgaatatggtgcatatctgccggttaaagaagttgcacgcgcactgtttcatggtattggttttgaaggttgggttagcctggaactgtttaatcgtcgtatgagcgaagaaggtccggaagttcctgaagaactggccatgcgtggtgcaattagctgggcaaaactggttcaggatctgcgtattccggttgaaggtccgctggttaccatgcctcgtgttagcgcaagcctgtaaatgcatgcgcgccgcgttcgcgcggcgcttttttttggtaccgagctcgaattcactggccgtcgttttacaacgtcgtgactgggaaaaccctggcgttacccaacttaatcgccttgcagcacatccccctttcgccagctggcgtaatagcgaagaggcccgcaccgatcgcccttcccaacagttgcgcagcctgaatggcgaatggcgcctgatgcggtattttctccttacgcatctgtgcggtatttcacaccgcatatggtgcactctcagtacaatctgctctgatgccgcatagttaagccagccccgacacccgccaacacccgctgacgaattc

SEQ ID NO: 28 - DNA, 7623 bp, Escherichia coli
  misc_feature (1)..(7623): DNA sequence of the plasmid pCP32AMP
acatgaatggtcttcggtttccgtgtttcgtaaagtctggaaacgcggaagtcagcgccctgcaccattatgttccggatctgcatcgcaggatgctgctggctaccctgtggaacacctacatctgtattaacgaagcgctggcattgaccctgagtgatttttctctggtcccgccgcatccataccgccagttgtttaccctcacaacgttccagtaaccgggcatgttcatcatcagtaacccgtatcgtgagcatcctctctcgtttcatcggtatcattacccccatgaacagaaattcccccttacacggaggcatcaagtgaccaaacaggaaaaaaccgcccttaacatggcccgctttatcagaagccagacattaacgcttctggagaaactcaacgagctggacgcggatgaacaggcagacatctgtgaatcgcttcacgaccacgctgatgagctttaccgcagctgcctcgcgcgtttcggtgatgacggtgaaaacctctgacacatgcagctcccggagacggtcacagcttgtctgtaagcggatgccgggagcagacaagcccgtcagggcgcgtcagcgggtgttggcgggtgtcggggcgcagccatgacccagtcacgtagcgatagcggagtgtatactggcttaactatgcggcatcagagcagattgtactgagagtgcaccatatgcggtgtgaaataccgcacagatgcgtaaggagaaaataccgcatcaggcgctcttccgcttcctcgctcactgactcgctgcgctcggtcgttcggctgcggcgagcggtatcagctcactcaaaggcggtaatacggttatccacagaatcaggggataacgcaggaaagaacatgtgagcaaaaggccagcaaaaggccaggaaccgtaaaaaggccgcgttgctggcgtttttccataggctccgcccccctgacgagcatcacaaaaatcgacgctcaagtcagaggtggcgaaacccgacaggactataaagataccaggcgtttccccctggaagctccctcgtgcgctctcctgttccgaccctgccgcttaccggatacctgtccgcctttctcccttcgggaagcgtggcgctttctcatagctcacgctgtaggtatctcagttcggtgtaggtcgttcgctccaagctgggctgtgtgcacgaaccccccgttcagcccgaccgctgcgccttatccggtaactatcgtcttgagtccaacccggtaagacacgacttatcgccactggcagcagccactggtaacaggattagcagagcgaggtatgtaggcggtgctacagagttcttgaagtggtggcctaactacggctacactagaaggacagtatttggtatctgcgctctgctgaagccagttaccttcggaaaaagagttggtagctcttgatccggcaaacaaaccaccgctggtagcggtggtttttttgtttgcaagcagcagattacgcgcagaaaaaaaggatctcaagaagatcctttgatcttttctacggggtctgacgctcagtggaacgaaaactcacgttaagggattttggtcatgagattatcaaaaaggatcttcacctagatccttttaaattaaaaatgaagttttaaatcaatctaaagtatatatgagtaaacttggtctgacagttaccaatgcttaatcagtgaggcacctatctcagcgatctgtctatttcgttcatccatagttgcctgactccccgtcgtgtagataactacgatacgggagggcttaccatctggccccagtgctgcaatgataccgcgagacccacgctcaccggctccagatttatcagcaataaaccagccagccggaagggccgagcgcagaagtggtcctgcaactttatccgcctccatccagtctattaattgttgccgggaagctagagtaagtagttcgccagttaatagtttgcgcaacgttgttgccattgctgcaggcatcgtggtgtcacgctcgtcgtttggtatggcttcattcagctccggttcccaacgatcaaggcgagttacatgatcccccatgttgtgcaaaaaagcggttagctccttcggtcctccgatcgttgtcagaagtaagttggccgcagtgttatcactcatggttatggcagcactgcataattctcttactgtcatgccatccgtaagatgcttttctgtgactggtgagtactcaaccaagtcattctgagaatagtgtatgcggcgaccgagttgctcttgcccggcgtcaacacgggataataccgcgccacatagcagaactttaaaagtgctcatcattggaaaacgttcttcggggcgaaaactctcaaggatcttaccgctgttgagatccagttcgatgtaacccactcgtgcacccaactgatcttcagcatcttttactttcaccagcgtttctgggtgagcaaaaacaggaaggcaaaatgccgcaaaaaagggaataagggcgacacggaaatgttgaatactcatactcttcctttttcaatattattgaagcatttatcagggttattgtctcatgagcggatacatatttgaatgtatttagaaaaataaacaaataggggttccgcgcacatttccccgaaaagtgccacctgacgtctaagaaaccattattatcatgacattaacctataaaaataggcgtatcacgaggccctttcgtcttcaagaattctgaaccagtcctaaaacgagtaaataggaccggcaattcttcaagcaataaacaggaataccaattattaaaagataacttagtcagatcgtacaataaagctttgaagaaaaatgcgccttattcaatctttgctataaaaaatggcccaaaatctcacattggaagacatttgatgacctcatttctttcaatgaagggcctaacggagttgactaatgttgtgggaaattggagcgataagcgtgcttctgccgtggccaggacaacgtatactcatcagataacagcaatacctgatcactacttcgcactagtttctcggtactatgcatatgatccaatatcaaaggaaatgatagcattgaaggatgagactaatccaattgaggagtggcagcatatagaacagctaaagggtagtgctgaaggaagcatacgataccccgcatggaatgggataatatcacaggaggtactagactacctttcatcctacataaatagacgcatataagtacgcatttaagcataaacacgcactatgccgttcttctcatgtatatatatatacaggcaacacgcagatataggtgcgacgtgaacagtgagctgtatgtgcgcagctcgcgttgcattttcggaagcgctcgttttcggaaacgctttgaagttcctattccgaagttcctattctctagaaagtataggaacttcagagcgcttttgaaaaccaaaagcgctctgaagacgcactttcaaaaaaccaaaaacgcaccggactgtaacgagctactaaaatattgcgaataccgcttccacaaacattgctcaaaagtatctctttgctatatatctctgtgctatatccctatataacctacccatccacctttcgctccttgaacttgcatctaaactcgacctctacattttttatgtttatctctagtattactctttagacaaaaaaattgtagtaagaactattcatagagtgaatcgaaaacaatacgaaaatgtaaacatttcctatacgtagtatatagagacaaaatagaagaaaccgttcataattttctgaccaatgaagaatcatcaacgctatcactttctgttcacaaagtatgcgcaatccacatcggtatagaatataatcggggatgcctttatcttgaaaaaatgcacccgcagcttcgctagtaatcagtaaacgcgggaagtggagtcaggctttttttatggaagagaaaatagacaccaaagtagccttcttctaaccttaacggacctacagtgcaaaaagttatcaagagactgcattatagagcgcacaaaggagaaaaaaagtaatctaagatgctttgttagaaaaatagcgctctcgggatgcatttttgtagaacaaaaaagaagtatagattctttgttggtaaaatagcgctctcgcgttgcatttctgttctgtaaaaatgcagctcagattctttgtttgaaaaattagcgctctcgcgttgcatttttgttttacaaaaatgaagcacagattcttcgttggtaaaatagcgctttcgcgttgcatttctgttctgtaaaaatgcagctcagattctttgtttgaaaaattagcgctctcgcgttgcatttttgttctacaaaatgaagcacagatgcttcgttaacaaagatatgctattgaagtgcaagatggaaacgcagaaaatgaaccggggatgcgacgtgcaagattacctatgcaatagatgcaatagtttctccaggaaccgaaatacatacattgtcttccgtaaagcgctagactatatattattatacaggttcaaatatactatctgtttcagggaaaactcccaggttcggatgttcaaaattcaatgatgggtaacaagtacgatcgtaaatctgtaaaacagtttgtcggatattaggctgtatctcctcaaagcgtattcgaatatcattgagaagctgcagcgtcacatcggataataatgatggcagccattgtagaagtgccttttgcatttctagtctctttctcggtctagctagttttactacatcgcgaagatagaatcttagatcacactgcctttgctgagctggatcaatagagtaacaaaagagtggtaaggcctcgttaaaggacaaggacctgagcggaagtgtatcgtacagtagacggagtatactagtatagtctatagtccgtggaattctcatgtttgacagcttatcatcgataagcttttcaattcaattcatcattttttttttattcttttttttgatttcggtttctttgaaatttttttgattcggtaatctccgaacagaaggaagaacgaaggaaggagcacagacttagattggtatatatacgcatatgtagtgttgaagaaacatgaaattgcccagtattcttaacccaactgcacagaacaaaaacctgcaggaaacgaagataaatcatgtcgaaagctacatataaggaacgtgctgctactcatcctagtcctgttgctgccaagctatttaatatcatgcacgaaaagcaaacaaacttgtgtgcttcattggatgttcgtaccaccaaggaattactggagttagttgaagcattaggtcccaaaatttgtttactaaaaacacatgtggatatcttgactgatttttccatggagggcacagttaagccgctaaaggcattatccgccaagtacaattttttactcttcgaagacagaaaatttgctgacattggtaatacagtcaaattgcagtactctgcgggtgtatacagaatagcagaatgggcagacattacgaatgcacacggtgtggtgggcccaggtattgttagcggtttgaagcaggcggcagaagaagtaacaaaggaacctagaggccttttgatgttagcagaattgtcatgcaagggctccctatctactggagaatatactaagggtactgttgacattgcgaagagcgacaaagattttgttatcggctttattgctcaaagagacatgggtggaagagatgaaggttacgattggttgattatgacacccggtgtgggtttagatgacaagggagacgcattgggtcaacagtatagaaccgtggatgatgtggtctctacaggatctgacattattattgttggaagaggactatttgcaaagggaagggatgctaaggtagagggtgaacgttacagaaaagcaggctgggaagcatatttgagaagatgcggccagcaaaactaaaaaactgtattataagtaaatgcatgtatactaaactcacaaattagagcttcaatttaattatatcagttattacccgggaatctcggtcgtaatgacttgaaataattaacaaacaaaggagttacagttagaaattgtaggagagatctcgtttttcgcgacaatctggcgtttttcttgctaattccaggattaatccgttcatagtgtaaaaccccgtttacacattctgacggaagatatagattggaagtattgcattcactaagataagtatggcaacactggaacagacatgaattatcagaacgacgatttacgcatcaaagaaatcaaagagttacttcctcctgtcgcattgctggaaaaattccccgctactgaaaatgccgcgaatacggttgcccatgcccgaaaagcgatccataagatcctgaaaggtaatgatgatcgcctgttggttgtgattggcccatgctcaattcatgatcctgtcgcggcaaaagagtatgccactcgcttgctggcgctgcgtgaagagctgaaagatgagctggaaatcgtaatgcgcgtctattttgaaaagccgcgtaccacggtgggctggaaagggctgattaacgatccgcatatggataatagcttccagatcaacgacggtctgcgtatagcccgtaaattgctgcttgatattaacgacagcggtctgccagcggcaggtgagtttctcgatatgatcaccccacaatatctcgctgacctgatgagctggggcgcaattggcgcacgtaccaccgaatcgcaggtgcaccgcgaactggcatcagggctttcttgtccggtcggcttcaaaaatggcaccgacggtacgattaaagtggctatcgatgccattaatgccgccggtgcgccgcactgcttcctgtccgtaacgaaatgggggcattcggcgattgtgaataccagcggtaacggcgattgccatatcattctgcgcggcggtaaagagcctaactacagcgcgaagcacgttgctgaagtgaaagaagggctgaacaaagcaggcctgccagcacaggtgatgatcgatttcagccatgctaactcgtccaaacaattcaaaaagcagatggatgtttgtgctgacgtttgccagcagattgccggtggcgaaaaggccattattggcgtgatggtggaaagccatctggtggaaggcaatcagagcctcgagagcggggagccgctggcctacggtaagagcatcaccgatgcctgcatcggctgggaagataccgatgctctgttacgtcaactggcgaatgcagtaaaagcgcgtcgcgggtaaggtttaattgtcggatgcgccgtcagagtggcgtatccgatgaatcaccacaggcctgataagtcgcgcagcgtcgcatcaggcaatgtgctccattgttagcaacaaaaaagccgactcacttgcagtcggctttctcattttaaacgaatgacgtttacttcgctttaccctggtttgcaaccgccgctgctttcgct

SEQ ID NO: 29 - DNA, 7630 bp, Escherichia coli
  misc_feature (1)..(7630): DNA sequence of the plasmid pCP14
ctcgaggctattgacgacagctatggttcactgtccaccaaccaaaactgtgctcagtaccgccaatatttctcccttgaggggtacaaagaggtgtccctagaagagatccacgctgtgtaaaaattttacaaaaaggtattgactttccctacagggtgtgtaataatttaattacaggcgggggcaaccccgcctgttctagaggaggaggaatcgccatggagaggattgtcgttactctcggggaacgtagttacccaattaccatcgcatctggtttgtttaatgaaccagcttcattcttaccgctgaaatcgggcgagcaggtcatgttggtcaccaacgaaaccctggctcctctgtatctcgataaggtccgcggcgtacttgaacaggcgggtgttaacgtcgatagcgttatcctccctgacggcgagcagtataaaagcctggctgtactcgataccgtctttacggcgttgttacaaaagccgcatggtcgcgatactacgctggtggcgcttggcggcggcgtagtgggcgatctgaccggcttcgcggcggcgagttatcagcgcggtgttcgtttcattcaagtcccgacgacgttactgtcgcaggtcgattcctccgttggcggcaaaactgcggtcaaccatcccctcggtaaaaacatgattggcgcgttctaccagcctgcttcagtggtggtggatctcgactgtctgaaaacgcttcccccgcgtgagttagcgtcggggctggcagaagtcatcaaatacggcattattcttgacggtgcgtttttcaactggctggaagagaatctggatgcgttgttgcgtctggacggtccggcaatggcgtactgtattcgccgttgttgtgaactgaaggcagaagttgtcgccgccgacgagcgcgaaaccgggttacgtgctttactgaatctgggacacacctttggtcatgccattgaagctgaaatggggtatggcaattggttacatggtgaagcggtcgctgcgggtatggtgatggcggcgcggacgtcggaacgtctcgggcagtttagttctgccgaaacgcagcgtattataaccctgctcacgcgggctgggttaccggtcaatgggccgcgcgaaatgtccgcgcaggcgtatttaccgcatatgctgcgtgacaagaaagtccttgcgggagagatgcgcttaattcttccgttggcaattggtaagagtgaagttcgcagcggcgtttcgcacgagcttgttcttaacgccattgccgattgtcaatcagcgtaatcatcgttcatgcctgatgccgctatgtaggccggataaggcgttcacgccgcatccggcaaccgatgcctgatgcgacgcggtcgcgtcttatcaggcctacaggtcgatgccgatatgtacatcgtattcggcaattaatacatagcaacatgaatggtcttcggtttccgtgtttcgtaaagtctggaaacgcggaagtcagcgccctgcaccattatgttccggatctgcatcgcaggatgctgctggctaccctgtggaacacctacatctgtattaacgaagcgctggcattgaccctgagtgatttttctctggtcccgccgcatccataccgccagttgtttaccctcacaacgttccagtaaccgggcatgttcatcatcagtaacccgtatcgtgagcatcctctctcgtttcatcggtatcattacccccatgaacagaaattcccccttacacggaggcatcaagtgaccaaacaggaaaaaaccgcccttaacatggcccgctttatcagaagccagacattaacgcttctggagaaactcaacgagctggacgcggatgaacaggcagacatctgtgaatcgcttcacgaccacgctgatgagctttaccgcagctgcctcgcgcgtttcggtgatgacggtgaaaacctctgacacatgcagctcccggagacggtcacagcttgtctgtaagcggatgccgggagcagacaagcccgtcagggcgcgtcagcgggtgttggcgggtgtcggggcgcagccatgacccagtcacgtagcgatagcggagtgtatactggcttaactatgcggcatcagagcagattgtactgagagtgcaccatatgcggtgtgaaataccgcacagatgcgtaaggagaaaataccgcatcaggcgctcttccgcttcctcgctcactgactcgctgcgctcggtcgttcggctgcggcgagcggtatcagctcactcaaaggcggtaatacggttatccacagaatcaggggataacgcaggaaagaacatgtgagcaaaaggccagcaaaaggccaggaaccgtaaaaaggccgcgttgctggcgtttttccataggctccgcccccctgacgagcatcacaaaaatcgacgctcaagtcagaggtggcgaaacccgacaggactataaagataccaggcgtttccccctggaagctccctcgtgcgctctcctgttccgaccctgccgcttaccggatacctgtccgcctttctcccttcgggaagcgtggcgctttctcatagctcacgctgtaggtatctcagttcggtgtaggtcgttcgctccaagctgggctgtgtgcacgaaccccccgttcagcccgaccgctgcgccttatccggtaactatcgtcttgagtccaacccggtaagacacgacttatcgccactggcagcagccactggtaacaggattagcagagcgaggtatgtaggcggtgctacagagttcttgaagtggtggcctaactacggctacactagaaggacagtatttggtatctgcgctctgctgaagccagttaccttcggaaaaagagttggtagctcttgatccggcaaacaaaccaccgctggtagcggtggtttttttgtttgcaagcagcagattacgcgcagaaaaaaaggatctcaagaagatcctttgatcttttctacggggtctgacgctcagtggaacgaaaactcacgttaagggattttggtcatgagattatcaaaaaggatcttcacctagatccttttaaattaaaaatgaagttttaaatcaatctaaagtatatatgagtaaacttggtctgacagttaccaatgcttaatcagtgaggcacctatctcagcgatctgtctatttcgttcatccatagttgcctgactccccgtcgtgtagataactacgatacgggagggcttaccatctggccccagtgctgcaatgataccgcgagacccacgctcaccggctccagatttatcagcaataaaccagccagccggaagggccgagcgcagaagtggtcctgcaactttatccgcctccatccagtctattaattgttgccgggaagctagagtaagtagttcgccagttaatagtttgcgcaacgttgttgccattgctgcaggcatcgtggtgtcacgctcgtcgtttggtatggcttcattcagctccggttcccaacgatcaaggcgagttacatgatcccccatgttgtgcaaaaaagcggttagctccttcggtcctccgatcgttgtcagaagtaagttggccgcagtgttatcactcatggttatggcagcactgcataattctcttactgtcatgccatccgtaagatgcttttctgtgactggtgagtactcaaccaagtcattctgagaatagtgtatgcggcgaccgagttgctcttgcccggcgtcaacacgggataataccgcgccacatagcagaactttaaaagtgctcatcattggaaaacgttcttcggggcgaaaactctcaaggatcttaccgctgttgagatccagttcgatgtaacccactcgtgcacccaactgatcttcagcatcttttactttcaccagcgtttctgggtgagcaaaaacaggaaggcaaaatgccgcaaaaaagggaataagggcgacacggaaatgttgaatactcatactcttcctttttcaatattattgaagcatttatcagggttattgtctcatgagcggatacatatttgaatgtatttagaaaaataaacaaataggggttccgcgcacatttccccgaaaagtgccacctgacgtctaagaaaccattattatcatgacattaacctataaaaataggcgtatcacgaggccctttcgtcttcaagaattctgaaccagtcctaaaacgagtaaataggaccggcaattcttcaagcaataaacaggaataccaattattaaaagataacttagtcagatcgtacaataaagctttgaagaaaaatgcgccttattcaatctttgctataaaaaatggcccaaaatctcacattggaagacatttgatgacctcatttctttcaatgaagggcctaacggagttgactaatgttgtgggaaattggagcgataagcgtgcttctgccgtggccaggacaacgtatactcatcagataacagcaatacctgatcactacttcgcactagtttctcggtactatgcatatgatccaatatcaaaggaaatgatagcattgaaggatgagactaatccaattgaggagtggcagcatatagaacagctaaagggtagtgctgaaggaagcatacgataccccgcatggaatgggataatatcacaggaggtactagactacctttcatcctacataaatagacgcatataagtacgcatttaagcataaacacgcactatgccgttcttctcatgtatatatatatacaggcaacacgcagatataggtgcgacgtgaacagtgagctgtatgtgcgcagctcgcgttgcattttcggaagcgctcgttttcggaaacgctttgaagttcctattccgaagttcctattctctagaaagtataggaacttcagagcgcttttgaaaaccaaaagcgctctgaagacgcactttcaaaaaaccaaaaacgcaccggactgtaacgagctactaaaatattgcgaataccgcttccacaaacattgctcaaaagtatctctttgctatatatctctgtgctatatccctatataacctacccatccacctttcgctccttgaacttgcatctaaactcgacctctacattttttatgtttatctctagtattactctttagacaaaaaaattgtagtaagaactattcatagagtgaatcgaaaacaatacgaaaatgtaaacatttcctatacgtagtatatagagacaaaatagaagaaaccgttcataattttctgaccaatgaagaatcatcaacgctatcactttctgttcacaaagtatgcgcaatccacatcggtatagaatataatcggggatgcctttatcttgaaaaaatgcacccgcagcttcgctagtaatcagtaaacgcgggaagtggagtcaggctttttttatggaagagaaaatagacaccaaagtagccttcttctaaccttaacggacctacagtgcaaaaagttatcaagagactgcattatagagcgcacaaaggagaaaaaaagtaatctaagatgctttgttagaaaaatagcgctctcgggatgcatttttgtagaacaaaaaagaagtatagattctttgttggtaaaatagcgctctcgcgttgcatttctgttctgtaaaaatgcagctcagattctttgtttgaaaaattagcgctctcgcgttgcatttttgttttacaaaaatgaagcacagattcttcgttggtaaaatagcgctttcgcgttgcatttctgttctgtaaaaatgcagctcagattctttgtttgaaaaattagcgctctcgcgttgcatttttgttctacaaaatgaagcacagatgcttcgttaacaaagatatgctattgaagtgcaagatggaaacgcagaaaatgaaccggggatgcgacgtgcaagattacctatgcaatagatgcaatagtttctccaggaaccgaaatacatacattgtcttccgtaaagcgctagactatatattattatacaggttcaaatatactatctgtttcagggaaaactcccaggttcggatgttcaaaattcaatgatgggtaacaagtacgatcgtaaatctgtaaaacagtttgtcggatattaggctgtatctcctcaaagcgtattcgaatatcattgagaagctgcagcgtcacatcggataataatgatggcagccattgtagaagtgccttttgcatttctagtctctttctcggtctagctagttttactacatcgcgaagatagaatcttagatcacactgcctttgctgagctggatcaatagagtaacaaaagagtggtaaggcctcgttaaaggacaaggacctgagcggaagtgtatcgtacagtagacggagtatactagtatagtctatagtccgtggaattctcatgtttgacagcttatcatcgataagcttttcaattcaattcatcattttttttttattcttttttttgatttcggtttctttgaaatttttttgattcggtaatctccgaacagaaggaagaacgaaggaaggagcacagacttagattggtatatatacgcatatgtagtgttgaagaaacatgaaattgcccagtattcttaacccaactgcacagaacaaaaacctgcaggaaacgaagataaatcatgtcgaaagctacatataaggaacgtgctgctactcatcctagtcctgttgctgccaagctatttaatatcatgcacgaaaagcaaacaaacttgtgtgcttcattggatgttcgtaccaccaaggaattactggagttagttgaagcattaggtcccaaaatttgtttactaaaaacacatgtggatatcttgactgatttttccatggagggcacagttaagccgctaaaggcattatccgccaagtacaattttttactcttcgaagacagaaaatttgctgacattggtaatacagtcaaattgcagtactctgcgggtgtatacagaatagcagaatgggcagacattacgaatgcacacggtgtggtgggcccaggtattgttagcggtttgaagcaggcggcagaagaagtaacaaaggaacctagaggccttttgatgttagcagaattgtcatgcaagggctccctatctactggagaatatactaagggtactgttgacattgcgaagagcgacaaagattttgttatcggctttattgctcaaagagacatgggtggaagagatgaaggttacgattggttgattatgacacccggtgtgggtttagatgacaagggagacgcattgggtcaacagtatagaaccgtggatgatgtggtctctacaggatctgacattattattgttggaagaggactatttgcaaagggaagggatgctaaggtagagggtgaacgttacagaaaagcaggctgggaagcatatttgagaagatgcggccagcaaaactaaaaaactgtattataagtaaatgcatgtatactaaactcacaaattagagcttcaatttaattatatcagttattacccgggaatctcggtcgtaatga

SEQ ID NO: 30 - DNA, 10015 bp, Escherichia coli
  misc_feature (1)..(10015): DNA sequence of the plasmid pCP50
cttgaaataattaacaaacaaaggagttacagttagaaattgtaggagagatctcgtttttcgcgacaatctggcgtttttcttgctaattccaggattaatccgttcatagtgtaaaaccccgtttacacattctgacggaagatatagattggaagtattgcattcactaagataagtatggcaacactggaacagacatgaattatcagaacgacgatttacgcatcaaagaaatcaaagagttacttcctcctgtcgcattgctggaaaaattccccgctactgaaaatgccgcgaatacggttgcccatgcccgaaaagcgatccataagatcctgaaaggtaatgatgatcgcctgttggttgtgattggcccatgctcaattcatgatcctgtcgcggcaaaagagtatgccactcgcttgctggcgctgcgtgaagagctgaaagatgagctggaaatcgtaatgcgcgtctattttgaaaagccgcgtaccacggtgggctggaaagggctgattaacgatccgcatatggataatagcttccagatcaacgacggtctgcgtatagcccgtaaattgctgcttgatattaacgacagcggtctgccagcggcaggtgagtttctcgatatgatcaccccacaatatctcgctgacctgatgagctggggcgcaattggcgcacgtaccaccgaatcgcaggtgcaccgcgaactggcatcagggctttcttgtccggtcggcttcaaaaatggcaccgacggtacgattaaagtggctatcgatgccattaatgccgccggtgcgccgcactgcttcctgtccgtaacgaaatgggggcattcggcgattgtgaataccagcggtaacggcgattgccatatcattctgcgcggcggtaaagagcctaactacagcgcgaagcacgttgctgaagtgaaagaagggctgaacaaagcaggcctgccagcacaggtgatgatcgatttcagccatgctaactcgtccaaacaattcaaaaagcagatggatgtttgtgctgacgtttgccagcagattgccggtggcgaaaaggccattattggcgtgatggtggaaagccatctggtggaaggcaatcagagcctcgagagcggggagccgctggcctacggtaagagcatcaccgatgcctgcatcggctgggaagataccgatgctctgttacgtcaactggcgaatgcagtaaaagcgcgtcgcgggtaaggtttaattgtcggatgcgccgtcagagtggcgtatccgatgaatcaccacaggcctgataagtcgcgcagcgtcgcatcaggcaatgtgctccattgttagcaacaaaaaagccgactcacttgcagtcggctttctcattttaaacgaatgacgtttacttcgctttaccctggtttgcaaccgccgctgctttcgctacatgaatggtcttcggtttccgtgtttcgtaaagtctggaaacgcggaagtcagcgccctgcaccattatgttccggatctgcatcgcaggatgctgctggctaccctgtggaacacctacatctgtattaacgaagcgctggcattgaccctgagtgatttttctctggtcccgccgcatccataccgccagttgtttaccctcacaacgttccagtaaccgggcatgttcatcatcagtaacccgtatcgtgagcatcctctctcgtttcatcggtatcattacccccatgaacagaaattcccccttacacggaggcatcaagtgaccaaacaggaaaaaaccgcccttaacatggcccgctttatcagaagccagacattaacgcttctggagaaactcaacgagctggacgcggatgaacaggcagacatctgtgaatcgcttcacgaccacgctgatgagctttaccgcagctgcctcgcgcgtttcggtgatgacggtgaaaacctctgacacatgcagctcccggagacggtcacagcttgtctgtaagcggatgccgggagcagacaagcccgtcagggcgcgtcagcgggtgttggcgggtgtcggggcgcagccatgacccagtcacgtagcgatagcggagtgtatactggcttaactatgcggcatcagagcagattgtactgagagtgcaccatatgcggtgtgaaataccgcacagatgcgtaaggagaaaataccgcatcaggcgctcttccgcttcctcgctcactgactcgctgcgctcggtcgttcggctgcggcgagcggtatcagctcactcaaaggcggtaatacggttatccacagaatcaggggataacgcaggaaagaacatgtgagcaaaaggccagcaaaaggccaggaaccgtaaaaaggccgcgttgctggcgtttttccataggctccgcccccctgacgagcatcacaaaaatcgacgctcaagtcagaggtggcgaaacccgacaggactataaagataccaggcgtttccccctggaagctccctcgtgcgctctcctgttccgaccctgccgcttaccggatacctgtccgcctttctcccttcgggaagcgtggcgctttctcatagctcacgctgtaggtatctcagttcggtgtaggtcgttcgctccaagctgggctgtgtgcacgaaccccccgttcagcccgaccgctgcgccttatccggtaactatcgtcttgagtccaacccggtaagacacgacttatcgccactggcagcagccactggtaacaggattagcagagcgaggtatgtaggcggtgctacagagttcttgaagtggtggcctaactacggctacactagaaggacagtatttggtatctgcgctctgctgaagccagttaccttcggaaaaagagttggtagctcttgatccggcaaacaaaccaccgctggtagcggtggtttttttgtttgcaagcagcagattacgcgcagaaaaaaaggatctcaagaagatcctttgatcttttctacggggtctgacgctcagtggaacgaaaactcacgttaagggattttggtcatgagattatcaaaaaggatcttcacctagatccttttaaattaaaaatgaagttttaaatcaatctaaagtatatatgagtaaacttggtctgacagttaccaatgcttaatcagtgaggcacctatctcagcgatctgtctatttcgttcatccatagttgcctgactccccgtcgtgtagataactacgatacgggagggcttaccatctggccccagtgctgcaatgataccgcgagacccacgctcaccggctccagatttatcagcaataaaccagccagccggaagggccgagcgcagaagtggtcctgcaactttatccgcctccatccagtctattaattgttgccgggaagctagagtaagtagttcgccagttaatagtttgcgcaacgttgttgccattgctgcaggcatcgtggtgtcacgctcgtcgtttggtatggcttcattcagctccggttcccaacgatcaaggcgagttacatgatcccccatgttgtgcaaaaaagcggttagctccttcggtcctccgatcgttgtcagaagtaagttggccgcagtgttatcactcatggttatggcagcactgcataattctcttactgtcatgccatccgtaagatgcttttctgtgactggtgagtactcaaccaagtcattctgagaatagtgtatgcggcgaccgagttgctcttgcccggcgtcaacacgggataataccgcgccacatagcagaactttaaaagtgctcatcattggaaaacgttcttcggggcgaaaactctcaaggatcttaccgctgttgagatccagttcgatgtaacccactcgtgcacccaactgatcttcagcatcttttactttcaccagcgtttctgggtgagcaaaaacaggaaggcaaaatgccgcaaaaaagggaataagggcgacacggaaatgttgaatactcatactcttcctttttcaatattattgaagcatttatcagggttattgtctcatgagcggatacatatttgaatgtatttagaaaaataaacaaataggggttccgcgcacatttccccgaaaagtgccacctgacgtctaagaaaccattattatcatgacattaacctataaaaataggcgtatcacgaggccctttcgtcttcaagaattctgaaccagtcctaaaacgagtaaataggaccggcaattcttcaagcaataaacaggaataccaattattaaaagataacttagtcagatcgtacaataaagctttgaagaaaaatgcgccttattcaatctttgctataaaaaatggcccaaaatctcacattggaagacatttgatgacctcatttctttcaatgaagggcctaacggagttgactaatgttgtgggaaattggagcgataagcgtgcttctgccgtggccaggacaacgtatactcatcagataacagcaatacctgatcactacttcgcactagtttctcggtactatgcatatgatccaatatcaaaggaaatgatagcattgaaggatgagactaatccaattgaggagtggcagcatatagaacagctaaagggtagtgctgaaggaagcatacgataccccgcatggaatgggataatatcacaggaggtactagactacctttcatcctacataaatagacgcatataagtacgcatttaagcataaacacgcactatgccgttcttctcatgtatatatatatacaggcaacacgcagatataggtgcgacgtgaacagtgagctgtatgtgcgcagctcgcgttgcattttcggaagcgctcgttttcggaaacgctttgaagttcctattccgaagttcctattctctagaaagtataggaacttcagagcgcttttgaaaaccaaaagcgctctgaagacgcactttcaaaaaaccaaaaacgcaccggactgtaacgagctactaaaatattgcgaataccgcttccacaaacattgctcaaaagtatctctttgctatatatctctgtgctatatccctatataacctacccatccacctttcgctccttgaacttgcatctaaactcgacctctacattttttatgtttatctctagtattactctttagacaaaaaaattgtagtaagaactattcatagagtgaatcgaaaacaatacgaaaatgtaaacatttcctatacgtagtatatagagacaaaatagaagaaaccgttcataattttctgaccaatgaagaatcatcaacgctatcactttctgttcacaaagtatgcgcaatccacatcggtatagaatataatcggggatgcctttatcttgaaaaaatgcacccgcagcttcgctagtaatcagtaaacgcgggaagtggagtcaggctttttttatggaagagaaaatagacaccaaagtagccttcttctaaccttaacggacctacagtgcaaaaagttatcaagagactgcattatagagcgcacaaaggagaaaaaaagtaatctaagatgctttgttagaaaaatagcgctctcgggatgcatttttgtagaacaaaaaagaagtatagattctttgttggtaaaatagcgctctcgcgttgcatttctgttctgtaaaaatgcagctcagattctttgtttgaaaaattagcgctctcgcgttgcatttttgttttacaaaaatgaagcacagattcttcgttggtaaaatagcgctttcgcgttgcatttctgttctgtaaaaatgcagctcagattctttgtttgaaaaattagcgctctcgcgttgcatttttgttctacaaaatgaagcacagatgcttcgttaacaaagatatgctattgaagtgcaagatggaaacgcagaaaatgaaccggggatgcgacgtgcaagattacctatgcaatagatgcaatagtttctccaggaaccgaaatacatacattgtcttccgtaaagcgctagactatatattattatacaggttcaaatatactatctgtttcagggaaaactcccaggttcggatgttcaaaattcaatgatgggtaacaagtacgatcgtaaatctgtaaaacagtttgtcggatattaggctgtatctcctcaaagcgtattcgaatatcattgagaagctgcagcgtcacatcggataataatgatggcagccattgtagaagtgccttttgcatttctagtctctttctcggtctagctagttttactacatcgcgaagatagaatcttagatcacactgcctttgctgagctggatcaatagagtaacaaaagagtggtaaggcctcgttaaaggacaaggacctgagcggaagtgtatcgtacagtagacggagtatactagtatagtctatagtccgtggaattctcatgtttgacagcttatcatcgataagcttttcaattcaattcatcattttttttttattcttttttttgatttcggtttctttgaaatttttttgattcggtaatctccgaacagaaggaagaacgaaggaaggagcacagacttagattggtatatatacgcatatgtagtgttgaagaaacatgaaattgcccagtattcttaacccaactgcacagaacaaaaacctgcaggaaacgaagataaatcatgtcgaaagctacatataaggaacgtgctgctactcatcctagtcctgttgctgccaagctatttaatatcatgcacgaaaagcaaacaaacttgtgtgcttcattggatgttcgtaccaccaaggaattactggagttagttgaagcattaggtcccaaaatttgtttactaaaaacacatgtggatatcttgactgatttttccatggagggcacagttaagccgctaaaggcattatccgccaagtacaattttttactcttcgaagacagaaaatttgctgacattggtaatacagtcaaattgcagtactctgcgggtgtatacagaatagcagaatgggcagacattacgaatgcacacggtgtggtgggcccaggtattgttagcggtttgaagcaggcggcagaagaagtaacaaaggaacctagaggccttttgatgttagcagaattgtcatgcaagggctccctatctactggagaatatactaagggtactgttgacattgcgaagagcgacaaagattttgttatcggctttattgctcaaagagacatgggtggaagagatgaaggttacgattggttgattatgacacccggtgtgggtttagatgacaagggagacgcattgggtcaacagtatagaaccgtggatgatgtggtctctacaggatctgacattattattgttggaagaggactatttgcaaagggaagggatgctaaggtagagggtgaacgttacagaaaagcaggctgggaagcatatttgagaagatgcggccagcaaaactaaaaaactgtattataagtaaatgcatgtatactaaactcacaaattagagcttcaatttaattatatcagttattacccgggaatctcggtcgtaatgaaaggaaaagcgcaacggacgggcgagtagattgcgcaacatgcgagcatgatccagagatttctgaagcagcaaaaggatgttccatgtacatgacgcgcggcttgcggtaaattgttggcaaattttccggcgtagcccaaaacgcgctgtcgtcaagtcgttaagggcgtgcccttcatcatccgatctggagtcaaaatgtcctcacgtaaagagcttgccaatgctattcgtgcgctgagcatggacgcagtacagaaagccaaatccggtcacccgggtgcccctatgggtatggctgacattgccgaagtcctgtggcgtgatttcctgaaacacaacccgcagaatccgtcctgggctgaccgtgaccgcttcgtgctgtccaacggccacggctccatgctgatctacagcctgctgcacctcaccggttacgatctgccgatggaagaactgaaaaacttccgtcagctgcactctaaaactccgggccacccggaagtaggttataccgctggtgtggaaaccaccaccggtccgctgggtcagggtattgccaacgcagtcggtatggcgattgcagaaaaaacgctggcggcgcagtttaaccgtccaggtcacgacattgtcgaccactacacctacgccttcatgggcgacggctgcatgatggaaggcatctcccacgaagtttgctctctggcgggtacgctgaagctgggtaaactgattgcgttctacgatgacaacggtatctcaatcgatggtcacgttgaaggctggttcactgacgacaccgcaatgcgtttcgaagcttacggctggcacgttattcgcgacatcgacggtcatgacgcggcatccatcaaacgcgcagtagaagaagcgcgcgcagtgactgacaaaccgtccctgctgatgtgcaaaaccatcatcggtttcggttccccgaacaaagccggtacccacgactcccacggtgcgccgctgggcgacgctgaaattgccctgacccgcgaacagctgggctggaaatacgcgccgttcgaaatcccgtctgaaatctatgctcagtgggatgcgaaagaagcaggccaggcgaaagaatctgcatggaatgagaagtttgcggcttacgcgaaagcttatccgcaggaagcggctgaatttacccgccgtatgaaaggcgaaatgccgtctgacttcgacgccaaagcgaaagagtttatcgctaaactgcaggctaatccggcgaaaatcgccagccgtaaagcgtcgcagaatgctatcgaagcgttcggcccgctgttgcctgaattcctcggcggctctgctgacctggcaccgtctaacctgaccctgtggtctggttctaaagcaatcaacgaagatgctgcaggtaactacatccactacggtgttcgcgagttcggtatgaccgcgattgctaacggtatctccctgcacggtggtttcctgccgtacacctccaccttcctgatgttcgtggaatacgcacgtaacgccgtacgtatggctgcgctgatgaaacagcgtcaggtgatggtttacacccacgactccatcggtctgggcgaagatggcccgactcaccagccggttgagcaggtcgcttctctgcgcgtgaccccgaacatgtctacatggcgtccgtgtgaccaggttgaatccgcggtcgcgtggaaatacggcgttgagcgtcaggacggcccgactgcgcttatcctctcccgtcagaacctggcgcagcaggaacgaactgaagagcaactggcaaacatcgcgcgcggtggttatgtgctgaaagactgcgccggtcagccggaactgattttcatcgctaccggttcagaagttgaactggctgttgctgcctacgaaaaactgactgccgaaggcgtgaaagcgcgcgtggtgtccatgccgtctaccgacgcatttgacaagcaggatgctgcttaccgtgaatccgtactgccgaaagcggttactgcacgcgttgctgtagaagcgggtattgctgactactggtacaagtatgttggcctgaacggtgctatcgtcggtatgaccaccttcggtgaatctgctccggcagagctgctgtttgaagagttcggcttcactgttgataacgttgttgcgaaagcaaaagaactgctgtaattagcatttcgggtaaaaaggtcgcttcggcgaccttttttattaccttgatatgtccgtttgcggacaagcaatagataaagcgtgttgtagatcacaaatatttatatgcaataaatatcaattatgtaatatgcatcacgatatgcgtattgacatttgttgttataactataactcaatgttatataagaaattaa

SEQ ID NO: 31 - DNA, 9065 bp, Escherichia coli
  misc_feature (1)..(9065): DNA sequence of the plasmid pCP54
acatgaatggtcttcggtttccgtgtttcgtaaagtctggaaacgcggaagtcagcgccctgcaccattatgttccggatctgcatcgcaggatgctgctggctaccctgtggaacacctacatctgtattaacgaagcgctggcattgaccctgagtgatttttctctggtcccgccgcatccataccgccagttgtttaccctcacaacgttccagtaaccgggcatgttcatcatcagtaacccgtatcgtgagcatcctctctcgtttcatcggtatcattacccccatgaacagaaattcccccttacacggaggcatcaagtgaccaaacaggaaaaaaccgcccttaacatggcccgctttatcagaagccagacattaacgcttctggagaaactcaacgagctggacgcggatgaacaggcagacatctgtgaatcgcttcacgaccacgctgatgagctttaccgcagctgcctcgcgcgtttcggtgatgacggtgaaaacctctgacacatgcagctcccggagacggtcacagcttgtctgtaagcggatgccgggagcagacaagcccgtcagggcgcgtcagcgggtgttggcgggtgtcggggcgcagccatgacccagtcacgtagcgatagcggagtgtatactggcttaactatgcggcatcagagcagattgtactgagagtgcaccatatgcggtgtgaaataccgcacagatgcgtaaggagaaaataccgcatcaggcgctcttccgcttcctcgctcactgactcgctgcgctcggtcgttcggctgcggcgagcggtatcagctcactcaaaggcggtaatacggttatccacagaatcaggggataacgcaggaaagaacatgtgagcaaaaggccagcaaaaggccaggaaccgtaaaaaggccgcgttgctggcgtttttccataggctccgcccccctgacgagcatcacaaaaatcgacgctcaagtcagaggtggcgaaacccgacaggactataaagataccaggcgtttccccctggaagctccctcgtgcgctctcctgttccgaccctgccgcttaccggatacctgtccgcctttctcccttcgggaagcgtggcgctttctcatagctcacgctgtaggtatctcagttcggtgtaggtcgttcgctccaagctgggctgtgtgcacgaaccccccgttcagcccgaccgctgcgccttatccggtaactatcgtcttgagtccaacccggtaagacacgacttatcgccactggcagcagccactggtaacaggattagcagagcgaggtatgtaggcggtgctacagagttcttgaagtggtggcctaactacggctacactagaaggacagtatttggtatctgcgctctgctgaagccagttaccttcggaaaaagagttggtagctcttgatccggcaaacaaaccaccgctggtagcggtggtttttttgtttgcaagcagcagattacgcgcagaaaaaaaggatctcaagaagatcctttgatcttttctacggggtctgacgctcagtggaacgaaaactcacgttaagggattttggtcatgagattatcaaaaaggatcttcacctagatccttttaaattaaaaatgaagttttaaatcaatctaaagtatatatgagtaaacttggtctgagtggcggttttcatggcttgttatgactgtttttttggggtacagtctatgcctcgggcatccaagcagcaagcgcgttacgccgtgggtcgatgtttgatgttatggagcagcaacgatgttacgcagcagggcagtcgccctaaaacaaagttaaacatcatgagggaagcggtgatcgccgaagtatcgactcaactatcagaggtagttggcgtcatcgagcgccatctcgaaccgacgttgctggccgtacatttgtacggctccgcagtggatggcggcctgaagccacacagtgatattgatttgctggttacggtgaccgtaaggcttgatgaaacaacgcggcgagctttgatcaacgaccttttggaaacttcggcttcccctggagagagcgagattctccgcgctgtagaagtcaccattgttgtgcacgacgacatcattccgtggcgttatccagctaagcgcgaactgcaatttggagaatggcagcgcaatgacattcttgcaggtatcttcgagccagccacgatcgacattgatctggctatcttgctgacaaaagcaagagaacatagcgttgccttggtaggtccagcggcggaggaactctttgatccggttcctgaacaggatctatttgaggcgctaaatgaaaccttaacgctatggaactcgccgcccgactgggctggcgatgagcgaaatgtagtgcttacgttgtcccgcatttggtacagcgcagtaaccggcaaaatcgcgccgaaggatgtcgctgccgactgggcaatggagcgcctgccggcccagtatcagcccgtcatacttgaagctagacaggcttatcttggacaagaagaagatcgcttggcctcgcgcgcagatcagttggaagaatttgtccactacgtgaaaggcgagatcaccaaggtagtcggcaaataatgtctaacaattcgttcaagccgacgccgcttcgcggcgcggcttaactcaagcgttagatgcactaagcacataattgctcacagccaaactatcagaattctgaaccagtcctaaaacgagtaaataggaccggcaattcttcaagcaataaacaggaataccaattattaaaagataacttagtcagatcgtacaataaagctttgaagaaaaatgcgccttattcaatctttgctataaaaaatggcccaaaatctcacattggaagacatttgatgacctcatttctttcaatgaagggcctaacggagttgactaatgttgtgggaaattggagcgataagcgtgcttctgccgtggccaggacaacgtatactcatcagataacagcaatacctgatcactacttcgcactagtttctcggtactatgcatatgatccaatatcaaaggaaatgatagcattgaaggatgagactaatccaattgaggagtggcagcatatagaacagctaaagggtagtgctgaaggaagcatacgataccccgcatggaatgggataatatcacaggaggtactagactacctttcatcctacataaatagacgcatataagtacgcatttaagcataaacacgcactatgccgttcttctcatgtatatatatatacaggcaacacgcagatataggtgcgacgtgaacagtgagctgtatgtgcgcagctcgcgttgcattttcggaagcgctcgttttcggaaacgctttgaagttcctattccgaagttcctattctctagaaagtataggaacttcagagcgcttttgaaaaccaaaagcgctctgaagacgcactttcaaaaaaccaaaaacgcaccggactgtaacgagctactaaaatattgcgaataccgcttccacaaacattgctcaaaagtatctctttgctatatatctctgtgctatatccctatataacctacccatccacctttcgctccttgaacttgcatctaaactcgacctctacattttttatgtttatctctagtattactctttagacaaaaaaattgtagtaagaactattcatagagtgaatcgaaaacaatacgaaaatgtaaacatttcctatacgtagtatatagagacaaaatagaagaaaccgttcataattttctgaccaatgaagaatcatcaacgctatcactttctgttcacaaagtatgcgcaatccacatcggtatagaatataatcggggatgcctttatcttgaaaaaatgcacccgcagcttcgctagtaatcagtaaacgcgggaagtggagtcaggctttttttatggaagagaaaatagacaccaaagtagccttcttctaaccttaacggacctacagtgcaaaaagttatcaagagactgcattatagagcgcacaaaggagaaaaaaagtaatctaagatgctttgttagaaaaatagcgctctcgggatgcatttttgtagaacaaaaaagaagtatagattctttgttggtaaaatagcgctctcgcgttgcatttctgttctgtaaaaatgcagctcagattctttgtttgaaaaattagcgctctcgcgttgcatttttgttttacaaaaatgaagcacagattcttcgttggtaaaatagcgctttcgcgttgcatttctgttctgtaaaaatgcagctcagattctttgtttgaaaaattagcgctctcgcgttgcatttttgttctacaaaatgaagcacagatgcttcgttaacaaagatatgctattgaagtgcaagatggaaacgcagaaaatgaaccggggatgcgacgtgcaagattacctatgcaatagatgcaatagtttctccaggaaccgaaatacatacattgtcttccgtaaagcgctagactatatattattatacaggttcaaatatactatctgtttcagggaaaactcccaggttcggatgttcaaaattcaatgatgggtaacaagtacgatcgtaaatctgtaaaacagtttgtcggatattaggctgtatctcctcaaagcgtattcgaatatcattgagaagctgcagcgtcacatcggataataatgatggcagccattgtagaagtgccttttgcatttctagtctctttctcggtctagctagttttactacatcgcgaagatagaatcttagatcacactgcctttgctgagctggatcaatagagtaacaaaagagtggtaaggcctcgttaaaggacaaggacctgagcggaagtgtatcgtacagtagacggagtatactagtatagtctatagtccgtggaattctcatgtttgacagcttatcatcgataagcttttcaattcaattcatcattttttttttattcttttttttgatttcggtttctttgaaatttttttgattcggtaatctccgaacagaaggaagaacgaaggaaggagcacagacttagattggtatatatacgcatatgtagtgttgaagaaacatgaaattgcccagtattcttaacccaactgcacagaacaaaaacctgcaggaaacgaagataaatcatgtcgaaagctacatataaggaacgtgctgctactcatcctagtcctgttgctgccaagctatttaatatcatgcacgaaaagcaaacaaacttgtgtgcttcattggatgttcgtaccaccaaggaattactggagttagttgaagcattaggtcccaaaatttgtttactaaaaacacatgtggatatcttgactgatttttccatggagggcacagttaagccgctaaaggcattatccgccaagtacaattttttactcttcgaagacagaaaatttgctgacattggtaatacagtcaaattgcagtactctgcgggtgtatacagaatagcagaatgggcagacattacgaatgcacacggtgtggtgggcccaggtattgttagcggtttgaagcaggcggcagaagaagtaacaaaggaacctagaggccttttgatgttagcagaattgtcatgcaagggctccctatctactggagaatatactaagggtactgttgacattgcgaagagcgacaaagattttgttatcggctttattgctcaaagagacatgggtggaagagatgaaggttacgattggttgattatgacacccggtgtgggtttagatgacaagggagacgcattgggtcaacagtatagaaccgtggatgatgtggtctctacaggatctgacattattattgttggaagaggactatttgcaaagggaagggatgctaaggtagagggtgaacgttacagaaaagcaggctgggaagcatatttgagaagatgcggccagcaaaactaaaaaactgtattataagtaaatgcatgtatactaaactcacaaattagagcttcaatttaattatatcagttattacccgggaatctcggtcgtaatgacttgaaataattaacaaacaaaggagttacagttagaaattgtaggagagatctcgtttttcgcgacaatctggcgtttttcttgctaattccaggattaatccgttcatagtgtaaaaccccgtttacacattctgacggaagatatagattggaagtattgcattcactaagataagtatggcaacactggaacagacatgaattatcagaacgacgatttacgcatcaaagaaatcaaagagttacttcctcctgtcgcattgctggaaaaattccccgctactgaaaatgccgcgaatacggttgcccatgcccgaaaagcgatccataagatcctgaaaggtaatgatgatcgcctgttggttgtgattggcccatgctcaattcatgatcctgtcgcggcaaaagagtatgccactcgcttgctggcgctgcgtgaagagctgaaagatgagctggaaatcgtaatgcgcgtctattttgaaaagccgcgtaccacggtgggctggaaagggctgattaacgatccgcatatggataatagcttccagatcaacgacggtctgcgtatagcccgtaaattgctgcttgatattaacgacagcggtctgccagcggcaggtgagtttctcgatatgatcaccccacaatatctcgctgacctgatgagctggggcgcaattggcgcacgtaccaccgaatcgcaggtgcaccgcgaactggcatcagggctttcttgtccggtcggcttcaaaaatggcaccgacggtacgattaaagtggctatcgatgccattaatgccgccggtgcgccgcactgcttcctgtccgtaacgaaatgggggcattcggcgattgtgaataccagcggtaacggcgattgccatatcattctgcgcggcggtaaagagcctaactacagcgcgaagcacgttgctgaagtgaaagaagggctgaacaaagcaggcctgccagcacaggtgatgatcgatttcagccatgctaactcgtccaaacaattcaaaaagcagatggatgtttgtgctgacgtttgccagcagattgccggtggcgaaaaggccattattggcgtgatggtggaaagccatctggtggaaggcaatcagagcctcgagagcggggagccgctggcctacggtaagagcatcaccgatgcctgcatcggctgggaagataccgatgctctgttacgtcaactggcgaatgcagtaaaagcgcgtcgcgggtaaggtttaattgtcggatgcgccgtcagagtggcgtatccgatgaatcaccacaggcctgataagtcgcgcagcgtcgcatcaggcaatgtgctccattgttagcaacaaaaaagccgactcacttgcagtcggctttctcattttaaacgaatgacgtttacttcgctttaccctggtttgcaaccgccgctgctttcgctctcgaggctattgacgacagctatggttcactgtccaccaaccaaaactgtgctcagtaccgccaatatttctcccttgaggggtacaaagaggtgtccctagaagagatccacgctgtgtaaaaattttacaaaaaggtattgactttccctacagggtgtgtaataatttaattacaggcgggggcaaccccgcctgttctagaggaggaggaatcgccatggagaggattgtcgttactctcggggaacgtagttacccaattaccatcgcatctggtttgtttaatgaaccagcttcattcttaccgctgaaatcgggcgagcaggtcatgttggtcaccaacgaaaccctggctcctctgtatctcgataaggtccgcggcgtacttgaacaggcgggtgttaacgtcgatagcgttatcctccctgacggcgagcagtataaaagcctggctgtactcgataccgtctttacggcgttgttacaaaagccgcatggtcgcgatactacgctggtggcgcttggcggcggcgtagtgggcgatctgaccggcttcgcggcggcgagttatcagcgcggtgttcgtttcattcaagtcccgacgacgttactgtcgcaggtcgattcctccgttggcggcaaaactgcggtcaaccatcccctcggtaaaaacatgattggcgcgttctaccagcctgcttcagtggtggtggatctcgactgtctgaaaacgcttcccccgcgtgagttagcgtcggggctggcagaagtcatcaaatacggcattattcttgacggtgcgtttttcaactggctggaagagaatctggatgcgttgttgcgtctggacggtccggcaatggcgtactgtattcgccgttgttgtgaactgaaggcagaagttgtcgccgccgacgagcgcgaaaccgggttacgtgctttactgaatctgggacacacctttggtcatgccattgaagctgaaatggggtatggcaattggttacatggtgaagcggtcgctgcgggtatggtgatggcggcgcggacgtcggaacgtctcgggcagtttagttctgccgaaacgcagcgtattataaccctgctcacgcgggctgggttaccggtcaatgggccgcgcgaaatgtccgcgcaggcgtatttaccgcatatgctgcgtgacaagaaagtccttgcgggagagatgcgcttaattcttccgttggcaattggtaagagtgaagttcgcagcggcgtttcgcacgagcttgttcttaacgccattgccgattgtcaatcagcgtaatcatcgttcatgcctgatgccgctatgtaggccggataaggcgttcacgccgcatccggcaaccgatgcctgatgcgacgcggtcgcgtcttatcaggcctacaggtcgatgccgatatgtacatcgtattcggcaattaatacatagca

SEQ ID NO: 32 - DNA, 11475 bp, Escherichia coli
  misc_feature (1)..(11475): DNA sequence of the plasmid pCP55
acatgaatggtcttcggtttccgtgtttcgtaaagtctggaaacgcggaagtcagcgccctgcaccattatgttccggatctgcatcgcaggatgctgctggctaccctgtggaacacctacatctgtattaacgaagcgctggcattgaccctgagtgatttttctctggtcccgccgcatccataccgccagttgtttaccctcacaacgttccagtaaccgggcatgttcatcatcagtaacccgtatcgtgagcatcctctctcgtttcatcggtatcattacccccatgaacagaaattcccccttacacggaggcatcaagtgaccaaacaggaaaaaaccgcccttaacatggcccgctttatcagaagccagacattaacgcttctggagaaactcaacgagctggacgcggatgaacaggcagacatctgtgaatcgcttcacgaccacgctgatgagctttaccgcagctgcctcgcgcgtttcggtgatgacggtgaaaacctctgacacatgcagctcccggagacggtcacagcttgtctgtaagcggatgccgggagcagacaagcccgtcagggcgcgtcagcgggtgttggcgggtgtcggggcgcagccatgacccagtcacgtagcgatagcggagtgtatactggcttaactatgcggcatcagagcagattgtactgagagtgcaccatatgcggtgtgaaataccgcacagatgcgtaaggagaaaataccgcatcaggcgctcttccgcttcctcgctcactgactcgctgcgctcggtcgttcggctgcggcgagcggtatcagctcactcaaaggcggtaatacggttatccacagaatcaggggataacgcaggaaagaacatgtgagcaaaaggccagcaaaaggccaggaaccgtaaaaaggccgcgttgctggcgtttttccataggctccgcccccctgacgagcatcacaaaaatcgacgctcaagtcagaggtggcgaaacccgacaggactataaagataccaggcgtttccccctggaagctccctcgtgcgctctcctgttccgaccctgccgcttaccggatacctgtccgcctttctcccttcgggaagcgtggcgctttctcatagctcacgctgtaggtatctcagttcggtgtaggtcgttcgctccaagctgggctgtgtgcacgaaccccccgttcagcccgaccgctgcgccttatccggtaactatcgtcttgagtccaacccggtaagacacgacttatcgccactggcagcagccactggtaacaggattagcagagcgaggtatgtaggcggtgctacagagttcttgaagtggtggcctaactacggctacactagaaggacagtatttggtatctgcgctctgctgaagccagttaccttcggaaaaagagttggtagctcttgatccggcaaacaaaccaccgctggtagcggtggtttttttgtttgcaagcagcagattacgcgcagaaaaaaaggatctcaagaagatcctttgatcttttctacggggtctgacgctcagtggaacgaaaactcacgttaagggattttggtcatgagattatcaaaaaggatcttcacctagatccttttaaattaaaaatgaagttttaaatcaatctaaagtatatatgagtaaacttggtctgacagttaccaatgcttaatcagtgaggcacctatctcagcgatctgtctatttcgttcatccatagttgcctgactccccgtcgtgtagataactacgatacgggagggcttaccatctggccccagtgctgcaatgataccgcgagacccacgctcaccggctccagatttatcagcaataaaccagccagccggaagggccgagcgcagaagtggtcctgcaactttatccgcctccatccagtctattaattgttgccgggaagctagagtaagtagttcgccagttaatagtttgcgcaacgttgttgccattgctgcaggcatcgtggtgtcacgctcgtcgtttggtatggcttcattcagctccggttcccaacgatcaaggcgagttacatgatcccccatgttgtgcaaaaaagcggttagctccttcggtcctccgatcgttgtcagaagtaagttggccgcagtgttatcactcatggttatggcagcactgcataattctcttactgtcatgccatccgtaagatgcttttctgtgactggtgagtactcaaccaagtcattctgagaatagtgtatgcggcgaccgagttgctcttgcccggcgtcaacacgggataataccgcgccacatagcagaactttaaaagtgctcatcattggaaaacgttcttcggggcgaaaactctcaaggatcttaccgctgttgagatccagttcgatgtaacccactcgtgcacccaactgatcttcagcatcttttactttcaccagcgtttctgggtgagcaaaaacaggaaggcaaaatgccgcaaaaaagggaataagggcgacacggaaatgttgaatactcatactcttcctttttcaatattattgaagcatttatcagggttattgtctcatgagcggatacatatttgaatgtatttagaaaaataaacaaataggggttccgcgcacatttccccgaaaagtgccacctgacgtctaagaaaccattattatcatgacattaacctataaaaataggcgtatcacgaggccctttcgtcttcaagaattctgaaccagtcctaaaacgagtaaataggaccggcaattcttcaagcaataaacaggaataccaattattaaaagataacttagtcagatcgtacaataaagctttgaagaaaaatgcgccttattcaatctttgctataaaaaatggcccaaaatctcacattggaagacatttgatgacctcatttctttcaatgaagggcctaacggagttgactaatgttgtgggaaattggagcgataagcgtgcttctgccgtggccaggacaacgtatactcatcagataacagcaatacctgatcactacttcgcactagtttctcggtactatgcatatgatccaatatcaaaggaaatgatagcattgaaggatgagactaatccaattgaggagtggcagcatatagaacagctaaagggtagtgctgaaggaagcatacgataccccgcatggaatgggataatatcacaggaggtactagactacctttcatcctacataaatagacgcatataagtacgcatttaagcataaacacgcactatgccgttcttctcatgtatatatatatacaggcaacacgcagatataggtgcgacgtgaacagtgagctgtatgtgcgcagctcgcgttgcattttcggaagcgctcgttttcggaaacgctttgaagttcctattccgaagttcctattctctagaaagtataggaacttcagagcgcttttgaaaaccaaaagcgctctgaagacgcactttcaaaaaaccaaaaacgcaccggactgtaacgagctactaaaatattgcgaataccgcttccacaaacattgctcaaaagtatctctttgctatatatctctgtgctatatccctatataacctacccatccacctttcgctccttgaacttgcatctaaactcgacctctacattttttatgtttatctctagtattactctttagacaaaaaaattgtagtaagaactattcatagagtgaatcgaaaacaatacgaaaatgtaaacatttcctatacgtagtatatagagacaaaatagaagaaaccgttcataattttctgaccaatgaagaatcatcaacgctatcactttctgttcacaaagtatgcgcaatccacatcggtatagaatataatcggggatgcctttatcttgaaaaaatgcacccgcagcttcgctagtaatcagtaaacgcgggaagtggagtcaggctttttttatggaagagaaaatagacaccaaagtagccttcttctaaccttaacggacctacagtgcaaaaagttatcaagagactgcattatagagcgcacaaaggagaaaaaaagtaatctaagatgctttgttagaaaaatagcgctctcgggatgcatttttgtagaacaaaaaagaagtatagattctttgttggtaaaatagcgctctcgcgttgcatttctgttctgtaaaaatgcagctcagattctttgtttgaaaaattagcgctctcgcgttgcatttttgttttacaaaaatgaagcacagattcttcgttggtaaaatagcgctttcgcgttgcatttctgttctgtaaaaatgcagctcagattctttgtttgaaaaattagcgctctcgcgttgcatttttgttctacaaaatgaagcacagatgcttcgttaacaaagatatgctattgaagtgcaagatggaaacgcagaaaatgaaccggggatgcgacgtgcaagattacctatgcaatagatgcaatagtttctccaggaaccgaaatacatacattgtcttccgtaaagcgctagactatatattattatacaggttcaaatatactatctgtttcagggaaaactcccaggttcggatgttcaaaattcaatgatgggtaacaagtacgatcgtaaatctgtaaaacagtttgtcggatattaggctgtatctcctcaaagcgtattcgaatatcattgagaagctgcagcgtcacatcggataataatgatggcagccattgtagaagtgccttttgcatttctagtctctttctcggtctagctagttttactacatcgcgaagatagaatcttagatcacactgcctttgctgagctggatcaatagagtaacaaaagagtggtaaggcctcgttaaaggacaaggacctgagcggaagtgtatcgtacagtagacggagtatactagtatagtctatagtccgtggaattctcatgtttgacagcttatcatcgataagcttttcaattcaattcatcattttttttttattcttttttttgatttcggtttctttgaaatttttttgattcggtaatctccgaacagaaggaagaacgaaggaaggagcacagacttagattggtatatatacgcatatgtagtgttgaagaaacatgaaattgcccagtattcttaacccaactgcacagaacaaaaacctgcaggaaacgaagataaatcatgtcgaaagctacatataaggaacgtgctgctactcatcctagtcctgttgctgccaagctatttaatatcatgcacgaaaagcaaacaaacttgtgtgcttcattggatgttcgtaccaccaaggaattactggagttagttgaagcattaggtcccaaaatttgtttactaaaaacacatgtggatatcttgactgatttttccatggagggcacagttaagccgctaaaggcattatccgccaagtacaattttttactcttcgaagacagaaaatttgctgacattggtaatacagtcaaattgcagtactctgcgggtgtatacagaatagcagaatgggcagacattacgaatgcacacggtgtggtgggcccaggtattgttagcggtttgaagcaggcggcagaagaagtaacaaaggaacctagaggccttttgatgttagcagaattgtcatgcaagggctccctatctactggagaatatactaagggtactgttgacattgcgaagagcgacaaagattttgttatcggctttattgctcaaagagacatgggtggaagagatgaaggttacgattggttgattatgacacccggtgtgggtttagatgacaagggagacgcattgggtcaacagtatagaaccgtggatgatgtggtctctacaggatctgacattattattgttggaagaggactatttgcaaagggaagggatgctaaggtagagggtgaacgttacagaaaagcaggctgggaagcatatttgagaagatgcggccagcaaaactaaaaaactgtattataagtaaatgcatgtatactaaactcacaaattagagcttcaatttaattatatcagttattacccgggaatctcggtcgtaatgaaaggaaaagcgcaacggacgggcgagtagattgcgcaacatgcgagcatgatccagagatttctgaagcagcaaaaggatgttccatgtacatgacgcgcggcttgcggtaaattgttggcaaattttccggcgtagcccaaaacgcgctgtcgtcaagtcgttaagggcgtgcccttcatcatccgatctggagtcaaaatgtcctcacgtaaagagcttgccaatgctattcgtgcgctgagcatggacgcagtacagaaagccaaatccggtcacccgggtgcccctatgggtatggctgacattgccgaagtcctgtggcgtgatttcctgaaacacaacccgcagaatccgtcctgggctgaccgtgaccgcttcgtgctgtccaacggccacggctccatgctgatctacagcctgctgcacctcaccggttacgatctgccgatggaagaactgaaaaacttccgtcagctgcactctaaaactccgggccacccggaagtaggttataccgctggtgtggaaaccaccaccggtccgctgggtcagggtattgccaacgcagtcggtatggcgattgcagaaaaaacgctggcggcgcagtttaaccgtccaggtcacgacattgtcgaccactacacctacgccttcatgggcgacggctgcatgatggaaggcatctcccacgaagtttgctctctggcgggtacgctgaagctgggtaaactgattgcgttctacgatgacaacggtatctcaatcgatggtcacgttgaaggctggttcactgacgacaccgcaatgcgtttcgaagcttacggctggcacgttattcgcgacatcgacggtcatgacgcggcatccatcaaacgcgcagtagaagaagcgcgcgcagtgactgacaaaccgtccctgctgatgtgcaaaaccatcatcggtttcggttccccgaacaaagccggtacccacgactcccacggtgcgccgctgggcgacgctgaaattgccctgacccgcgaacagctgggctggaaatacgcgccgttcgaaatcccgtctgaaatctatgctcagtgggatgcgaaagaagcaggccaggcgaaagaatctgcatggaatgagaagtttgcggcttacgcgaaagcttatccgcaggaagcggctgaatttacccgccgtatgaaaggcgaaatgccgtctgacttcgacgccaaagcgaaagagtttatcgctaaactgcaggctaatccggcgaaaatcgccagccgtaaagcgtcgcagaatgctatcgaagcgttcggcccgctgttgcctgaattcctcggcggctctgctgacctggcaccgtctaacctgaccctgtggtctggttctaaagcaatcaacgaagatgctgcaggtaactacatccactacggtgttcgcgagttcggtatgaccgcgattgctaacggtatctccctgcacggtggtttcctgccgtacacctccaccttcctgatgttcgtggaatacgcacgtaacgccgtacgtatggctgcgctgatgaaacagcgtcaggtgatggtttacacccacgactccatcggtctgggcgaagatggcccgactcaccagccggttgagcaggtcgcttctctgcgcgtgaccccgaacatgtctacatggcgtccgtgtgaccaggttgaatccgcggtcgcgtggaaatacggcgttgagcgtcaggacggcccgactgcgcttatcctctcccgtcagaacctggcgcagcaggaacgaactgaagagcaactggcaaacatcgcgcgcggtggttatgtgctgaaagactgcgccggtcagccggaactgattttcatcgctaccggttcagaagttgaactggctgttgctgcctacgaaaaactgactgccgaaggcgtgaaagcgcgcgtggtgtccatgccgtctaccgacgcatttgacaagcaggatgctgcttaccgtgaatccgtactgccgaaagcggttactgcacgcgttgctgtagaagcgggtattgctgactactggtacaagtatgttggcctgaacggtgctatcgtcggtatgaccaccttcggtgaatctgctccggcagagctgctgtttgaagagttcggcttcactgttgataacgttgttgcgaaagcaaaagaactgctgtaattagcatttcgggtaaaaaggtcgcttcggcgaccttttttattaccttgatatgtccgtttgcggacaagcaatagataaagcgtgttgtagatcacaaatatttatatgcaataaatatcaattatgtaatatgcatcacgatatgcgtattgacatttgttgttataactataactcaatgttatataagaaattaacttgaaataattaacaaacaaaggagttacagttagaaattgtaggagagatctcgtttttcgcgacaatctggcgtttttcttgctaattccaggattaatccgttcatagtgtaaaaccccgtttacacattctgacggaagatatagattggaagtattgcattcactaagataagtatggcaacactggaacagacatgaattatcagaacgacgatttacgcatcaaagaaatcaaagagttacttcctcctgtcgcattgctggaaaaattccccgctactgaaaatgccgcgaatacggttgcccatgcccgaaaagcgatccataagatcctgaaaggtaatgatgatcgcctgttggttgtgattggcccatgctcaattcatgatcctgtcgcggcaaaagagtatgccactcgcttgctggcgctgcgtgaagagctgaaagatgagctggaaatcgtaatgcgcgtctattttgaaaagccgcgtaccacggtgggctggaaagggctgattaacgatccgcatatggataatagcttccagatcaacgacggtctgcgtatagcccgtaaattgctgcttgatattaacgacagcggtctgccagcggcaggtgagtttctcgatatgatcaccccacaatatctcgctgacctgatgagctggggcgcaattggcgcacgtaccaccgaatcgcaggtgcaccgcgaactggcatcagggctttcttgtccggtcggcttcaaaaatggcaccgacggtacgattaaagtggctatcgatgccattaatgccgccggtgcgccgcactgcttcctgtccgtaacgaaatgggggcattcggcgattgtgaataccagcggtaacggcgattgccatatcattctgcgcggcggtaaagagcctaactacagcgcgaagcacgttgctgaagtgaaagaagggctgaacaaagcaggcctgccagcacaggtgatgatcgatttcagccatgctaactcgtccaaacaattcaaaaagcagatggatgtttgtgctgacgtttgccagcagattgccggtggcgaaaaggccattattggcgtgatggtggaaagccatctggtggaaggcaatcagagcctcgagagcggggagccgctggcctacggtaagagcatcaccgatgcctgcatcggctgggaagataccgatgctctgttacgtcaactggcgaatgcagtaaaagcgcgtcgcgggtaaggtttaattgtcggatgcgccgtcagagtggcgtatccgatgaatcaccacaggcctgataagtcgcgcagcgtcgcatcaggcaatgtgctccattgttagcaacaaaaaagccgactcacttgcagtcggctttctcattttaaacgaatgacgtttacttcgctttaccctggtttgcaaccgccgctgctttcgctctcgaggctattgacgacagctatggttcactgtccaccaaccaaaactgtgctcagtaccgccaatatttctcccttgaggggtacaaagaggtgtccctagaagagatccacgctgtgtaaaaattttacaaaaaggtattgactttccctacagggtgtgtaataatttaattacaggcgggggcaaccccgcctgttctagaggaggaggaatcgccatggagaggattgtcgttactctcggggaacgtagttacccaattaccatcgcatctggtttgtttaatgaaccagcttcattcttaccgctgaaatcgggcgagcaggtcatgttggtcaccaacgaaaccctggctcctctgtatctcgataaggtccgcggcgtacttgaacaggcgggtgttaacgtcgatagcgttatcctccctgacggcgagcagtataaaagcctggctgtactcgataccgtctttacggcgttgttacaaaagccgcatggtcgcgatactacgctggtggcgcttggcggcggcgtagtgggcgatctgaccggcttcgcggcggcgagttatcagcgcggtgttcgtttcattcaagtcccgacgacgttactgtcgcaggtcgattcctccgttggcggcaaaactgcggtcaaccatcccctcggtaaaaacatgattggcgcgttctaccagcctgcttcagtggtggtggatctcgactgtctgaaaacgcttcccccgcgtgagttagcgtcggggctggcagaagtcatcaaatacggcattattcttgacggtgcgtttttcaactggctggaagagaatctggatgcgttgttgcgtctggacggtccggcaatggcgtactgtattcgccgttgttgtgaactgaaggcagaagttgtcgccgccgacgagcgcgaaaccgggttacgtgctttactgaatctgggacacacctttggtcatgccattgaagctgaaatggggtatggcaattggttacatggtgaagcggtcgctgcgggtatggtgatggcggcgcggacgtcggaacgtctcgggcagtttagttctgccgaaacgcagcgtattataaccctgctcacgcgggctgggttaccggtcaatgggccgcgcgaaatgtccgcgcaggcgtatttaccgcatatgctgcgtgacaagaaagtccttgcgggagagatgcgcttaattcttccgttggcaattggtaagagtgaagttcgcagcggcgtttcgcacgagcttgttcttaacgccattgccgattgtcaatcagcgtaatcatcgttcatgcctgatgccgctatgtaggccggataaggcgttcacgccgcatccggcaaccgatgcctgatgcgacgcggtcgcgtcttatcaggcctacaggtcgatgccgatatgtacatcgtattcggcaattaatacatagca

SEQ ID NO: 33 - DNA, 7769 bp, Escherichia coli
  misc_feature (1)..(7769): DNA sequence of the plasmid YEP24
gaattctgaaccagtcctaaaacgagtaaataggaccggcaattcttcaagcaataaacaggaataccaattattaaaagataacttagtcagatcgtacaataaagctttgaagaaaaatgcgccttattcaatctttgctataaaaaatggcccaaaatctcacattggaagacatttgatgacctcatttctttcaatgaagggcctaacggagttgactaatgttgtgggaaattggagcgataagcgtgcttctgccgtggccaggacaacgtatactcatcagataacagcaatacctgatcactacttcgcactagtttctcggtactatgcatatgatccaatatcaaaggaaatgatagcattgaaggatgagactaatccaattgaggagtggcagcatatagaacagctaaagggtagtgctgaaggaagcatacgataccccgcatggaatgggataatatcacaggaggtactagactacctttcatcctacataaatagacgcatataagtacgcatttaagcataaacacgcactatgccgttcttctcatgtatatatatatacaggcaacacgcagatataggtgcgacgtgaacagtgagctgtatgtgcgcagctcgcgttgcattttcggaagcgctcgttttcggaaacgctttgaagttcctattccgaagttcctattctctagaaagtataggaacttcagagcgcttttgaaaaccaaaagcgctctgaagacgcactttcaaaaaaccaaaaacgcaccggactgtaacgagctactaaaatattgcgaataccgcttccacaaacattgctcaaaagtatctctttgctatatatctctgtgctatatccctatataacctacccatccacctttcgctccttgaacttgcatctaaactcgacctctacattttttatgtttatctctagtattactctttagacaaaaaaattgtagtaagaactattcatagagtgaatcgaaaacaatacgaaaatgtaaacatttcctatacgtagtatatagagacaaaatagaagaaaccgttcataattttctgaccaatgaagaatcatcaacgctatcactttctgttcacaaagtatgcgcaatccacatcggtatagaatataatcggggatgcctttatcttgaaaaaatgcacccgcagcttcgctagtaatcagtaaacgcgggaagtggagtcaggctttttttatggaagagaaaatagacaccaaagtagccttcttctaaccttaacggacctacagtgcaaaaagttatcaagagactgcattatagagcgcacaaaggagaaaaaaagtaatctaagatgctttgttagaaaaatagcgctctcgggatgcatttttgtagaacaaaaaagaagtatagattctttgttggtaaaatagcgctctcgcgttgcatttctgttctgtaaaaatgcagctcagattctttgtttgaaaaattagcgctctcgcgttgcatttttgttttacaaaaatgaagcacagattcttcgttggtaaaatagcgctttcgcgttgcatttctgttctgtaaaaatgcagctcagattctttgtttgaaaaattagcgctctcgcgttgcatttttgttctacaaaatgaagcacagatgcttcgttaacaaagatatgctattgaagtgcaagatggaaacgcagaaaatgaaccggggatgcgacgtgcaagattacctatgcaatagatgcaatagtttctccaggaaccgaaatacatacattgtcttccgtaaagcgctagactatatattattatacaggttcaaatatactatctgtttcagggaaaactcccaggttcggatgttcaaaattcaatgatgggtaacaagtacgatcgtaaatctgtaaaacagtttgtcggatattaggctgtatctcctcaaagcgtattcgaatatcattgagaagctgcagcgtcacatcggataataatgatggcagccattgtagaagtgccttttgcatttctagtctctttctcggtctagctagttttactacatcgcgaagatagaatcttagatcacactgcctttgctgagctggatcaatagagtaacaaaagagtggtaaggcctcgttaaaggacaaggacctgagcggaagtgtatcgtacagtagacggagtatactagtatagtctatagtccgtggaattctcatgtttgacagcttatcatcgataagcttttcaattcaattcatcattttttttttattcttttttttgatttcggtttctttgaaatttttttgattcggtaatctccgaacagaaggaagaacgaaggaaggagcacagacttagattggtatatatacgcatatgtagtgttgaagaaacatgaaattgcccagtattcttaacccaactgcacagaacaaaaacctgcaggaaacgaagataaatcatgtcgaaagctacatataaggaacgtgctgctactcatcctagtcctgttgctgccaagctatttaatatcatgcacgaaaagcaaacaaacttgtgtgcttcattggatgttcgtaccaccaaggaattactggagttagttgaagcattaggtcccaaaatttgtttactaaaaacacatgtggatatcttgactgatttttccatggagggcacagttaagccgctaaaggcattatccgccaagtacaattttttactcttcgaagacagaaaatttgctgacattggtaatacagtcaaattgcagtactctgcgggtgtatacagaatagcagaatgggcagacattacgaatgcacacggtgtggtgggcccaggtattgttagcggtttgaagcaggcggcagaagaagtaacaaaggaacctagaggccttttgatgttagcagaattgtcatgcaagggctccctatctactggagaatatactaagggtactgttgacattgcgaagagcgacaaagattttgttatcggctttattgctcaaagagacatgggtggaagagatgaaggttacgattggttgattatgacacccggtgtgggtttagatgacaagggagacgcattgggtcaacagtatagaaccgtggatgatgtggtctctacaggatctgacattattattgttggaagaggactatttgcaaagggaagggatgctaaggtagagggtgaacgttacagaaaagcaggctgggaagcatatttgagaagatgcggccagcaaaactaaaaaactgtattataagtaaatgcatgtatactaaactcacaaattagagcttcaatttaattatatcagttattacccgggaatctcggtcgtaatgatttttataatgacgaaaaaaaaaaaattggaaagaaaaagctttaatgcggtagtttatcacagttaaattgctaacgcagtcaggcaccgtgtatgaaatctaacaatgcgctcatcgtcatcctcggcaccgtcaccctggatgctgtaggcataggcttggttatgccggtactgccgggcctcttgcgggatatcgtccattccgacagcatcgccagtcactatggcgtgctgctagcgctatatgcgttgatgcaatttctatgcgcacccgttctcggagcactgtccgaccgctttggccgccgcccagtcctgctcgcttcgctacttggagccactatcgactacgcgatcatggcgaccacacccgtcctgtggatcctctacgccggacgcatcgtggccggcatcaccggcgccacaggtgcggttgctggcgcctatatcgccgacatcaccgatggggaagatcgggctcgccacttcgggctcatgagcgcttgtttcggcgtgggtatggtggcaggccccgtggccgggggactgttgggcgccatctccttgcatgcaccattccttgcggcggcggtgctcaacggcctcaacctactactgggctgcttcctaatgcaggagtcgcataagggagagcgtcgaccgatgcccttgagagccttcaacccagtcagctccttccggtgggcgcggggcatgactatcgtcgccgcacttatgactgtcttctttatcatgcaactcgtaggacaggtgccggcagcgctctgggtcattttcggcgaggaccgctttcgctggagcgcgacgatgatcggcctgtcgcttgcggtattcggaatcttgcacgccctcgctcaagccttcgtcactggtcccgccaccaaacgtttcggcgagaagcaggccattatcgccggcatggcggccgacgcgctgggctacgtcttgctggcgttcgcgacgcgaggctggatggccttccccattatgattcttctcgcttccggcggcatcgggatgcccgcgttgcaggccatgctgtccaggcaggtagatgacgaccatcagggacagcttcaaggatcgctcgcggctcttaccagcctaacttcgatcactggaccgctgatcgtcacggcgatttatgccgcctcggcgagcacatggaacgggttggcatggattgtaggcgccgccctataccttgtctgcctccccgcgttgcgtcgcggtgcatggagccgggccacctcgacctgaatggaagccggcggcacctcgctaacggattcaccactccaagaattggagccaatcaattcttgcggagaactgtgaatgcgcaaaccaacccttggcagaacatatccatcgcgtccgccatctccagcagccgcacgcggcgcatctcgggcagcgttgggtcctggccacgggtgcgcatgatcgtgctcctgtcgttgaggacccggctaggctggcggggttgccttactggttagcagaatgaatcaccgatacgcgagcgaacgtgaagcgactgctgctgcaaaacgtctgcgacctgagcaacaacatgaatggtcttcggtttccgtgtttcgtaaagtctggaaacgcggaagtcagcgccctgcaccattatgttccggatctgcatcgcaggatgctgctggctaccctgtggaacacctacatctgtattaacgaagcgctggcattgaccctgagtgatttttctctggtcccgccgcatccataccgccagttgtttaccctcacaacgttccagtaaccgggcatgttcatcatcagtaacccgtatcgtgagcatcctctctcgtttcatcggtatcattacccccatgaacagaaattcccccttacacggaggcatcaagtgaccaaacaggaaaaaaccgcccttaacatggcccgctttatcagaagccagacattaacgcttctggagaaactcaacgagctggacgcggatgaacaggcagacatctgtgaatcgcttcacgaccacgctgatgagctttaccgcagctgcctcgcgcgtttcggtgatgacggtgaaaacctctgacacatgcagctcccggagacggtcacagcttgtctgtaagcggatgccgggagcagacaagcccgtcagggcgcgtcagcgggtgttggcgggtgtcggggcgcagccatgacccagtcacgtagcgatagcggagtgtatactggcttaactatgcggcatcagagcagattgtactgagagtgcaccatatgcggtgtgaaataccgcacagatgcgtaaggagaaaataccgcatcaggcgctcttccgcttcctcgctcactgactcgctgcgctcggtcgttcggctgcggcgagcggtatcagctcactcaaaggcggtaatacggttatccacagaatcaggggataacgcaggaaagaacatgtgagcaaaaggccagcaaaaggccaggaaccgtaaaaaggccgcgttgctggcgtttttccataggctccgcccccctgacgagcatcacaaaaatcgacgctcaagtcagaggtggcgaaacccgacaggactataaagataccaggcgtttccccctggaagctccctcgtgcgctctcctgttccgaccctgccgcttaccggatacctgtccgcctttctcccttcgggaagcgtggcgctttctcatagctcacgctgtaggtatctcagttcggtgtaggtcgttcgctccaagctgggctgtgtgcacgaaccccccgttcagcccgaccgctgcgccttatccggtaactatcgtcttgagtccaacccggtaagacacgacttatcgccactggcagcagccactggtaacaggattagcagagcgaggtatgtaggcggtgctacagagttcttgaagtggtggcctaactacggctacactagaaggacagtatttggtatctgcgctctgctgaagccagttaccttcggaaaaagagttggtagctcttgatccggcaaacaaaccaccgctggtagcggtggtttttttgtttgcaagcagcagattacgcgcagaaaaaaaggatctcaagaagatcctttgatcttttctacggggtctgacgctcagtggaacgaaaactcacgttaagggattttggtcatgagattatcaaaaaggatcttcacctagatccttttaaattaaaaatgaagttttaaatcaatctaaagtatatatgagtaaacttggtctgacagttaccaatgcttaatcagtgaggcacctatctcagcgatctgtctatttcgttcatccatagttgcctgactccccgtcgtgtagataactacgatacgggagggcttaccatctggccccagtgctgcaatgataccgcgagacccacgctcaccggctccagatttatcagcaataaaccagccagccggaagggccgagcgcagaagtggtcctgcaactttatccgcctccatccagtctattaattgttgccgggaagctagagtaagtagttcgccagttaatagtttgcgcaacgttgttgccattgctgcaggcatcgtggtgtcacgctcgtcgtttggtatggcttcattcagctccggttcccaacgatcaaggcgagttacatgatcccccatgttgtgcaaaaaagcggttagctccttcggtcctccgatcgttgtcagaagtaagttggccgcagtgttatcactcatggttatggcagcactgcataattctcttactgtcatgccatccgtaagatgcttttctgtgactggtgagtactcaaccaagtcattctgagaatagtgtatgcggcgaccgagttgctcttgcccggcgtcaacacgggataataccgcgccacatagcagaactttaaaagtgctcatcattggaaaacgttcttcggggcgaaaactctcaaggatcttaccgctgttgagatccagttcgatgtaacccactcgtgcacccaactgatcttcagcatcttttactttcaccagcgtttctgggtgagcaaaaacaggaaggcaaaatgccgcaaaaaagggaataagggcgacacggaaatgttgaatactcatactcttcctttttcaatattattgaagcatttatcagggttattgtctcatgagcggatacatatttgaatgtatttagaaaaataaacaaataggggttccgcgcacatttccccgaaaagtgccacctgacgtctaagaaaccattattatcatgacattaacctataaaaataggcgtatcacgaggccctttcgtcttcaa

SEQ ID NO: 34 - DNA, 2000 bp, Escherichia coli
  gene (1)..(2000): DNA sequence of the deleted aroE region
actacgtccgtcctctgaaatcttcagcggatggacatatcgtcaaagttctggaggggcaggtttgccctgcatgtggcgcaaatctggtattacgccagggacgctttggtatgtttattggttgcattaactaccctgaatgcgaacataccgaacttatcgataaaccggacgaaacagcaattacatgcccccaatgtcggacgggccatctggtccagcgccgctcccgttatggcaaaacatttcactcttgtgatcgctacccggagtgtcaatttgccattaacttcaaacccatagctggagaatgccctgagtgtcattatccgctactcatcgaaaagaaaaccgcgcagggtgtaaaacacttttgtgccagtaaacaatgtggaaagccggtttcggcggaataataacgtgaataataacctgcaaagagacgctatcgcagctgcgatagatgttctcaatgaagaacgtgtcatcgcctatccaacggaagccgttttcggtgttgggtgcgatcctgatagcgaaacagcagtgatgcgactgttggagttaaaacagcgtccggttgataaggggctgattttaatcgcagcaaattacgagcagcttaaaccctatattgatgacaccatgttgactgacgtgcagcgtgaaaccattttttcccgctggccaggtcctgtcacctttgtctttcccgcgcctgcgacaacaccgcgctggttgacgggccgctttgattcgcttgctgtacgagtcaccgaccatccgttggtggttgctttgtgccaggcttatggtaaaccgctggtttctaccagtgccaacttgagtggattgccaccttgtcgaacagtagacgaagttcgcgcacaatttggcgcggcgttcccggttgtgcctggtgaaacgggggggcgtttaaatccttcagaaatccgcgatgccctgacgggtgaactgtttcgacaggggtaacataatcaggccatccagtttccggacagggaagagtgggacgagaataaaaaatgtgtatgttttcccgctctcgtgaatggtatgcaactgacatgcgcgatctctggcgagagtctggcgtatcgctttactggagatacgccagaacagtggttagcgagttttcgtcagcatcgctgggacctggaagaagaagcggaaaacttaattcaggaacaaagtgaagatgatcaaggctgggtctggttaccctgatccagatattcgtccttccatttcacgtaattattcgcggaatagcgtaacccagccttctcttcatcacttaacgggcggatctgtttgacggggctaccgagatacagatatccgctctccagccgtttattttgtgggaccagactacccgcaccaatcatcacatcatcttctactattgcgccatcaagtaaaattgagcccatcccaaccaaaactcgattgccaatggtgcagccgtggagcatcaccttgtgaccaacagtgacatcttcgccaatggttaatgggttgccatctgggttgtacgaggatttatgagtgacatgcaacatactgccatcctggatattggtgcgtgctccgatctgtacataatgtacatctccacgaatcacaacgagcggccagatccccacatcatcagccagacgaacgtcaccaatcacgacactgctatcgtcgatcattacgcgctgaccgatttgtggaaaaagatcgcggtatgggcgtaaaacatcagacatacttacctcagcaataaatgatttactaatgactttgggggcattattggccttgtgcaagtcttttagtatgcaaaaaagcaccgttttgtgtgcgattgcagcaaaaagggtgaaaaaacaacaaacagaaaaaaagatcaaaaaaatacttgtgcaaaaaattgggatccctataatgcgcctccgttgagacgacaacgtgaaacacttcac

SEQ ID NO: 35 - DNA, 2460 bp, Escherichia coli
  gene (1)..(2460): DNA sequence of the integrated cassette  ack::P15aroB
gatcggcggcataaaacggatcgcataacgcgtcatcttgataacgcgattttcgacaaagaccggggcaaggcgtttttccagcggccacgtctttgagtaatgctgtccccggcgaaacaagctaaaaaaattaacagaacgattatccggcgttgacatgcttcacctcaacttcacatataaagattcaaaaatttgtgcaaattcacaactcagcgggacaacgttcaaaacattttgtcttccatacccactatcaggtatcctttagcagcctgaaggcctaagtagtacatattcattgagtcgtcaaattcatatacattatgccattggctgaaaattacgcaaaatggcatagactcaagatatttcttccatcatgcaaaaaaaaatttgcagtgcatgatgttaatcataaatgtcggtgtcatcatgcgctacgctctatggctccctgacgtttttttagccacgtatcaattataggtacttccctcgaggctattgacgacagctatggttcactgtccaccaaccaaaactgtgctcagtaccgccaatatttctcccttgaggggtacaaagaggtgtccctagaagagatccacgctgtgtaaaaattttacaaaaaggtattgactttccctacagggtgtgtaataatttaattacaggcgggggcaaccccgcctgttctagaggaggaggaatcgccatggagaggattgtcgttactctcggggaacgtagttacccaattaccatcgcatctggtttgtttaatgaaccagcttcattcttaccgctgaaatcgggcgagcaggtcatgttggtcaccaacgaaaccctggctcctctgtatctcgataaggtccgcggcgtacttgaacaggcgggtgttaacgtcgatagcgttatcctccctgacggcgagcagtataaaagcctggctgtactcgataccgtctttacggcgttgttacaaaagccgcatggtcgcgatactacgctggtggcgcttggcggcggcgtagtgggcgatctgaccggcttcgcggcggcgagttatcagcgcggtgttcgtttcattcaagtcccgacgacgttactgtcgcaggtcgattcctccgttggcggcaaaactgcggtcaaccatcccctcggtaaaaacatgattggcgcgttctaccagcctgcttcagtggtggtggatctcgactgtctgaaaacgcttcccccgcgtgagttagcgtcggggctggcagaagtcatcaaatacggcattattcttgacggtgcgtttttcaactggctggaagagaatctggatgcgttgttgcgtctggacggtccggcaatggcgtactgtattcgccgttgttgtgaactgaaggcagaagttgtcgccgccgacgagcgcgaaaccgggttacgtgctttactgaatctgggacacacctttggtcatgccattgaagctgaaatggggtatggcaattggttacatggtgaagcggtcgctgcgggtatggtgatggcggcgcggacgtcggaacgtctcgggcagtttagttctgccgaaacgcagcgtattataaccctgctcacgcgggctgggttaccggtcaatgggccgcgcgaaatgtccgcgcaggcgtatttaccgcatatgctgcgtgacaagaaagtccttgcgggagagatgcgcttaattcttccgttggcaattggtaagagtgaagttcgcagcggcgtttcgcacgagcttgttcttaacgccattgccgattgtcaatcagcgtaatcatcgttcatgcctgatgccgctatgtaggccggataaggcgttcacgccgcatccggcaaccgatgcctgatgcgacgcggtcgcgtcttatcaggcctacaggtcgatgccgatatgtacatcgtattcggcaattaatacatagcatttcacaccgccagctcagctggcggtgctgttttgtaacccgccaaatcggcggtaacgaaagaggataaaccgtgtcccgtattattatgctgatccctaccggaaccagcgtcggtctgaccagcgtcagccttggcgtgatccgtgcaatggaacgcaaaggcgttcgtctgagcgttttcaaacctatcgctcagccgcgtaccggtggcgatgcgcccgatcagactacgactatcgtgcgtgcgaactcttccaccacgacggccgctgaaccgctgaaaatgagctacgttgaaggtctgctttccagcaatcagaaagatgtgctgatggaagagatcgtcgcaaactaccacgctaacaccaaagacgctgaagtcgttctggttgaaggtctggtcccgacacgtaagcaccagtttgcccagtctctgaactacgaaatcgctaaaacgctgaatgcggaaatcgtcttcgttatgtctcagggcact

SEQ ID NO: 36 - DNA, 1000 bp, Escherichia coli
  gene (1)..(1000): DNA sequence of the  poxB region
gcggcccggctccgtatatggattgggtagagcaggaagtgaaagcgctcggcgtgacgcgtttctttaaagagaaattcttcaccccagtagcggaagcagcgaccagcggtctgaaattcaccaaactgcaaccggcacgagaattttacgccccggttggcaccacgctactggaggcgctggaaagcaataacgttccggttgtcgccgcctgccgtgcgggtgtttgcggctgctgtaagacaaaagtggtttccggtgaatatacggtgagcagcacaatgacgctgaccgacgccgaaatcgctgaaggttacgtactggcctgctcctgccatccgcagggggatttggttctcgcataatcgccttatgcccgatgatattcctttcatcgggctatttaaccgttagtgcctcctttctctcccatcccttccccctccgtcagatgaactaaacttgttaccgttatcacattcaggagatggagaaccaaagggtggcatttcccgtcataataaggacatgccatgattgatttacgcagtgataccgttacccgaccgagccgcgccatgctcgaagcaatgatggccgccccggttggggacgacgtttacggagacgaccctaccgttaatgctctgcaggactacgccgcagagctttccggtaaagaagccgccatttttctgccgaccggcactcaggccaacctggtcgctctgctcagtcactgcgaacgtggcgaagagtatattgtcggtcaggccgcgcataactatctgtttgaagccggtggcgcagcggtgctgggcagtattcagccgcaacccatcgacgcggctgccgacggcacgctaccgctggataaagtggcgatgaaaatcaaacccgacgatatccatttcgcccgcaccaaattactcagtctggaaaacacccacaacggcaaagtgctgccgcgtgaatacctgaaagaagcatgggaatt

SEQ ID NO: 37 - DNA, 3392 bp, Escherichia coli
  gene (1)..(3392): DNA sequence of the integrated cassette  poxB::tktA
gcggcccggctccgtatatggattgggtagagcaggaagtgaaagcgctcggcgtgacgcgtttctttaaagagaaattcttcaccccagtagcggaagcagcgaccagcggtctgaaattcaccaaactgcaaccggcacgagaattttacgccccggttggcaccacgctactggaggcgctggaaagcaataacgttccggttgtcgccgcctgccgtgcgggtgtttgcggctgctgtaagacaaaagtggtttccggtgaatatacggtgagcagcacaatgacgctgaccgacgccgaaatcgctgaaggttacgtactggcctgctcctgccatccgcagggggatttggttctcgcataatcgccttatgcccgatgatattcctttcatcgggctatttaaccgttagtgcctcctttctctcccatcccttccccctccgtcagatgaactaaacttgttaccgttatcacattcaggagatggagaaccaaggaaaagcgcaacggacgggcgagtagattgcgcaacatgcgagcatgatccagagatttctgaagcagcaaaaggatgttccatgtacatgacgcgcggcttgcggtaaattgttggcaaattttccggcgtagcccaaaacgcgctgtcgtcaagtcgttaagggcgtgcccttcatcatccgatctggagtcaaaatgtcctcacgtaaagagcttgccaatgctattcgtgcgctgagcatggacgcagtacagaaagccaaatccggtcacccgggtgcccctatgggtatggctgacattgccgaagtcctgtggcgtgatttcctgaaacacaacccgcagaatccgtcctgggctgaccgtgaccgcttcgtgctgtccaacggccacggctccatgctgatctacagcctgctgcacctcaccggttacgatctgccgatggaagaactgaaaaacttccgtcagctgcactctaaaactccgggccacccggaagtaggttataccgctggtgtggaaaccaccaccggtccgctgggtcagggtattgccaacgcagtcggtatggcgattgcagaaaaaacgctggcggcgcagtttaaccgtccaggtcacgacattgtcgaccactacacctacgccttcatgggcgacggctgcatgatggaaggcatctcccacgaagtttgctctctggcgggtacgctgaagctgggtaaactgattgcgttctacgatgacaacggtatctcaatcgatggtcacgttgaaggctggttcactgacgacaccgcaatgcgtttcgaagcttacggctggcacgttattcgcgacatcgacggtcatgacgcggcatccatcaaacgcgcagtagaagaagcgcgcgcagtgactgacaaaccgtccctgctgatgtgcaaaaccatcatcggtttcggttccccgaacaaagccggtacccacgactcccacggtgcgccgctgggcgacgctgaaattgccctgacccgcgaacagctgggctggaaatacgcgccgttcgaaatcccgtctgaaatctatgctcagtgggatgcgaaagaagcaggccaggcgaaagaatctgcatggaatgagaagtttgcggcttacgcgaaagcttatccgcaggaagcggctgaatttacccgccgtatgaaaggcgaaatgccgtctgacttcgacgccaaagcgaaagagtttatcgctaaactgcaggctaatccggcgaaaatcgccagccgtaaagcgtcgcagaatgctatcgaagcgttcggcccgctgttgcctgaattcctcggcggctctgctgacctggcaccgtctaacctgaccctgtggtctggttctaaagcaatcaacgaagatgctgcaggtaactacatccactacggtgttcgcgagttcggtatgaccgcgattgctaacggtatctccctgcacggtggtttcctgccgtacacctccaccttcctgatgttcgtggaatacgcacgtaacgccgtacgtatggctgcgctgatgaaacagcgtcaggtgatggtttacacccacgactccatcggtctgggcgaagatggcccgactcaccagccggttgagcaggtcgcttctctgcgcgtgaccccgaacatgtctacatggcgtccgtgtgaccaggttgaatccgcggtcgcgtggaaatacggcgttgagcgtcaggacggcccgactgcgcttatcctctcccgtcagaacctggcgcagcaggaacgaactgaagagcaactggcaaacatcgcgcgcggtggttatgtgctgaaagactgcgccggtcagccggaactgattttcatcgctaccggttcagaagttgaactggctgttgctgcctacgaaaaactgactgccgaaggcgtgaaagcgcgcgtggtgtccatgccgtctaccgacgcatttgacaagcaggatgctgcttaccgtgaatccgtactgccgaaagcggttactgcacgcgttgctgtagaagcgggtattgctgactactggtacaagtatgttggcctgaacggtgctatcgtcggtatgaccaccttcggtgaatctgctccggcagagctgctgtttgaagagttcggcttcactgttgataacgttgttgcgaaagcaaaagaactgctgtaattagcatttcgggtaaaaaggtcgcttcggcgaccttttttattaccttgatatgtccgtttgcggacaagcaatagataaagcgtgttgtagatcacaaatatttatatgcaataaatatcaattatgtaatatgcatcacgatatgcgtattgacatttgttgttataactataactcaatgttatataagaaattaaaaagggtggcatttcccgtcataataaggacatgccatgattgatttacgcagtgataccgttacccgaccgagccgcgccatgctcgaagcaatgatggccgccccggttggggacgacgtttacggagacgaccctaccgttaatgctctgcaggactacgccgcagagctttccggtaaagaagccgccatttttctgccgaccggcactcaggccaacctggtcgctctgctcagtcactgcgaacgtggcgaagagtatattgtcggtcaggccgcgcataactatctgtttgaagccggtggcgcagcggtgctgggcagtattcagccgcaacccatcgacgcggctgccgacggcacgctaccgctggataaagtggcgatgaaaatcaaacccgacgatatccatttcgcccgcaccaaattactcagtctggaaaacacccacaacggcaaagtgctgccgcgtgaatacctgaaagaagcatgggaatt

SEQ ID NO: 38 - DNA, 1045 bp, Escherichia coli
  gene (1)..(1045): DNA sequence of the  ptsHI region
gaagatgaaagctttaccaacaagaatattgtggttattctaccatcatcgggtgagcgttatttaagcaccgcattgtttgccgatctcttcactgagaaagaattgcaacagtaatgccagcttgttaaaaatgcgtaaaaaagcacctttttaggtgcttttttgtggcctgcttcaaactttcgcccctcctggcattgattcagcctgtcggaactggtatttaaccagactaattattttgatgcgcgaaattaatcgttacaggaaaagccaaagctgaatcgattttatgatttggttcaattcttcctttagcggcataatgtttaatgacgtacgaaacgtcagcggtcaacacccgccagcaatggactgtattgcgctcttcgtgcgtcgcgtctgttaaaaactggcgctaacaatacaggctaaagtcgaaccgccaggctagactttagttccacaacactaaacctataagttggggaaatacaatgttccagcaagaagttaccattaccgctccgacaatctgctaatccacgagatgcggcccaatttactgcttaggagaagatcatgggtttgttcgataaactgaaatctctggtttccgacgacaagaaggataccggaactattgagatcattgctccgctctctggcgagatcgtcaatatcgaagacgtgccggatgtcgtttttgcggaaaaaatcgttggtgatggtattgctatcaaaccaacgggtaacaaaatggtcgcgccagtagacggcaccattggtaaaatctttgaaaccaaccacgcattctctatcgaatctgatagcggcgttgaactgttcgtccacttcggtatcgacaccgttgaactgaaaggcgaaggcttcaagcgtattgctgaagaaggtcagcgcgtgaaagttggcgatactgtcattgaatttgatctgccgctgctggaagagaaagccaagtctaccctgactccggttgttatctccaacatggacgaaatcaaagaactgatcaaactgt

SEQ ID NO: 39 - DNA, 4595 bp, Escherichia coli
  gene (1)..(4595): DNA sequence of the integrated cassette  tdc::glf-glk
ctgatttctttgtcgctgatcccttactggaactctgcagttatcgaccaggttgacctcggttcgctgtcgttaaccggtcatgacggtatcctgatcactgtctggctggggatttccatcatggttttctcctttaacttctcgccaatcgtctcttccttcgtggtttctaaacgtgaagagtatgagaaagacttcggtcgcgacttcaccgaacgtaaatgttcccaaatcatttctcgtgccagcatgctgatggttgcagtggtgatgttctttgcctttagctgcctgtttactctgtctccggccaacatggcggaagccaaagcgcagaatattccagtgctttcttatctggctaaccactttgcgtccatgaccggtaccaaaacaacgttcgcgattacactggaatatgcggcttccatcatcgcactcgtggctatcttcaaatctttcttcggtcactatctggggacgctggaaggcttgaatggtctgattctgaagttcggttataaaggtgacaaaaccaaagtgtcgctgggtaaactgaatactctcagcatgatcttcatcatgggctccacctgggttgttgcctacgccaacccgaacatcctcgacctgattgaagccatgggcgcaccgattatcgcatccctgctgtgcctgttgccgatgtatgccatccgtaaagcgccgtctctggcgaaataccgtggtcgtctggataacgtgtttgttaccgtgattggtctgctgaccatcctgaacatcgtatacaaactgttttaatccgtaactcaggatgagaaaagagatgaatgaatttccggttgttttggttattaactgtggttcgtcttcgattaagttttccgtactcgatgccagcgactgtgaagtattaatgtcaggtattgccgacggtattaactcggaaaatgcattcttatccgtaaatgggggagagccagcaccgctggctcaccacagctacgaaggtgcattgaaggcaattgcatttgaactggaaaaacggagtttaaatgacagcgtggccttaattggtgcaaaagtggctgtgactgtaaaaagaaatcgaaaaagaccgttttgtgtgaaaacggtctttttgtttccttttaaccaactgccataactcgaggcctacctagcttccaagaaagatatcctaacagcacaagagcggaaagatgttttgttctacatccagaacaacctctgctaaaattcctgaaaaattttgcaaaaagttgttgactttatctacaaggtgtggtataataatcttaacaacagcaggacgctctagagggagaggaatcgccatgagttctgaaagtagtcagggtctagtcacgcgactagccctaatcgctgctataggcggcttgcttttcggttacgattcagcggttatcgctgcaatcggtacaccggttgatatccattttattgcccctcgtcacctgtctgctacggctgcggcttccctttctgggatggtcgttgttgctgttttggtcggttgtgttaccggttctttgctgtctggctggattggtattcgcttcggtcgtcgcggcggattgttgatgagttccatttgtttcgtcgccgccggttttggtgctgcgttaaccgaaaaattatttggaaccggtggttcggctttacaaattttttgctttttccggtttcttgccggtttaggtatcggtgtcgtttcaaccttgaccccaacctatattgctgaaattgctccgccagacaaacgtggtcagatggtttctggtcagcagatggccattgtgacgggtgctttaaccggttatatctttacctggttactggctcatttcggttctatcgattgggttaatgccagtggttggtgctggtctccggcttcagaaggcctgatcggtattgccttcttattgctgctgttaaccgcaccggatacgccgcattggttggtgatgaagggacgtcattccgaggctagcaaaatccttgctcgtctggaaccgcaagccgatcctaatctgacgattcaaaagattaaagctggctttgataaagccatggacaaaagcagcgcaggtttgtttgcttttggtatcaccgttgtttttgccggtgtatccgttgctgccttccagcagttagtcggtattaacgccgtgctgtattatgcaccgcagatgttccagaatttaggttttggagctgatacggcattattgcagaccatctctatcggtgttgtgaacttcatcttcaccatgattgcttcccgtgttgttgaccgcttcggccgtaaacctctgcttatttggggtgctctcggtatggctgcaatgatggctgttttaggctgctgtttctggttcaaagtcggtggtgttttgcctttggcttctgtgcttctttatattgcagtctttggtatgtcatggggccctgtctgctgggttgttctgtcagaaatgttcccgagttccatcaagggcgcagctatgcctatcgctgttaccggacaatggttagctaatatcttggttaacttcctgtttaaggttgccgatggttctccagcattgaatcagactttcaaccacggtttctcctatctcgttttcgcagcattaagtatcttaggtggcttgattgttgctcgcttcgtgccggaaaccaaaggtcggagcctggatgaaatcgaggagatgtggcgctcccagaagtagttaaacttgctttggctgaatccttttgtcttttttagataagtcttaaccaattatactttttgtttacaacgatggtataaagcgggcggacttattttacctgttgggtagccttctgatttcagaaaggaattattatggaaattgttgcgattgacatcggtggaacgcatgcgcgtttctctattgcggaagtaagcaatggtcgggttctttctcttggagaagaaacaacttttaaaacggcagaacatgctagcttgcagttagcttgggaacgtttcggtgaaaaactgggtcgtcctctgccacgtgccgcagctattgcatgggctggcccggttcatggtgaagttttaaaacttaccaataacccttgggtattaagaccagctactctgaatgaaaagctggacatcgatacgcatgttctgatcaatgacttcggcgcggttgcccacgcggttgcgcatatggattcttcttatctggatcatatttgtggtcctgatgaagcgcttcctagcgatggtgttatcactattcttggtccgggaacgggcttgggtgttgcccatctgttgcggactgaaggccgttatttcgtcatcgaaactgaaggcggtcatatcgactttgctccgcttgacagacttgaagacaaaattctggcacgtttacgtgaacgtttccgccgcgtttctatcgaacgcattatttctggcccgggtcttggtaatatctacgaagcactggctgccattgaaggcgttccgttcagcttgctggatgatattaaattatggcagatggctttggaaggtaaagacaaccttgctgaagccgctttggatcgcttctgcttgagccttggcgctatcgctggtgatcttgctttggcacagggtcgaaccagtgttgttattggcggtggtgtcggtcttcgtatcgcttcccatttgccagaatctggtttccgtcagcgctttgtttcaaaaggacgctttgaacgcgtcatgtccaagattccggttaagttgattacttatccgcagcctggactgttgggtgcgcagctgcctatgccaacaaatattctgaagttgaataatattttttaatattatgaactgaatttaagaggctgccttccgataaaatcgggaggtggccttttttatattttttactaaaaaatgaagacaaaaaagtcttaagtaagaataatattattattaacttttgatatattttgtattagtggatccgccctcccgctggaaattgaagccatcgcagtacgtagtgcgtaaagcctcgtgagcgggacggtcgtaaggtcgttccgctccacttcactgaacggcaatccgagggtgtggatatgattagtgcattcgatattttcaaaattgggattggtccctccagttcgcataccgtggggccaatgaatgccggaaaaagttttattgatcggctggaaagtagcggcttattaaccgcgacgagccatattgtggtcgatctgtacgggtcgttgtcactgacgggcaaaggccatgccacggatgtcgccatcatcatgggactggcaggaaacagtccgcaggatgttgtcattgatgagatccctgcatttatagagttagtaacgcgcagcgggcggctgccagtggcatctggtgcgcatattgttgattttcctgtagcaaagaacattatcttccatcccgaaatgttgcctcgccatgagaacggaatgcggatcactgcctggaagggacaggaagagctattaagtaaaac

SEQ ID NO: 40 - DNA, 1069 bp, Escherichia coli
  gene (1)..(1069): DNA sequence of the  galP region
actttggtcgtgaacatttcccgtgggaaaaaaccgacaaagcgcagctgctgcgcgatgctgccggtctgaagtaatctttcttcacctgcgttcaaaggccagcctcgcgctggcctttttcttttggataggcgttcacgccgcatccggcaaaaaaaccgcccgcacaataacatcattcttcctgatcacgtttcaccgcagattatcatcacaactgaaaccgattacaccaaccacaacagacaaagatttgtaatattttcatattattattcggttttcacagttgttacatttcttttcagtaaagtcttaattgcagataacagcgtttaatctatgatgatataactcaattattttcatgcacttaaatcataactaagataaatgttagtgtaagcgattacactgatgtgatttgcttcacatctttttacgtcgtactcacctatcttaattcacaataaaaaataaccatattggagggcatcatgcctgacgctaaaaaacaggggcggtcaaacaaggcaatgacgtttgaaataggcgctcacgattaatctccccaagcttcctcccatcgcggaggaagccacctcttgcagtcatcttttcttcgctctatcctctgccgctatgaaaacatcccgtctccctatcgccatccaacaggccgttatgcgtcgcctgcgggaaaaactcgcccaggccaacctgaagctagggcgtaactacccggagccaaaactctcttacacccagcgcggaacctccgccggaacggcctggctggaaagctatgaaattcgcctcaatcccgttttgctgttggaaaacagtgaagcttttattgaagaagtggtaccgcacgaactggcacatttgctggtatggaaacatttcggccgcgtagcgccacatggcaaagagtggaagtggatgatggaaaacgtgctgggtgttcccgcccgtcgtacgcatcagttcgaactgcaatccgtgcgtcgcaacaccttcccctaccgctgcaagtgccaggagcatcagcttaccgtacgcc

SEQ ID NO: 41 - DNA, 6100 bp, Escherichia coli
  gene (1)..(6100): MYR352  adhE::P15-catAX , PR-aroY, P26-quiC
ttgattttcataggttaagcaaatcatcaccgcactgactatactctcgtattcgagcagatgatttactaaaaaagtttaacattatcaggagagcattagcttgctattgacgacagctatggttcactgtccaccaaccaaaactgtgctcagtaccgccaatatttctcccttgaggggtacaaagaggtgtccctagaagagatccacgctgtgtaaaaattttacaaaaaggtattgactttccctacagggtgtgtaataatttaattacaggcgggggcaaccccgcctgttctgcagaggaggaatatagccatggaagtgaaaatcttcaacacccaggatgttcaggattttctgcgtgttgcaagcggtctggaacaagagggtggtaatccgcgtgttaaacaaattattcatcgtgttctgagcgacctgtataaagcaattgaagatctgaatatcaccagcgacgaatattgggcaggcgttgcatatctgaatcagctgggtgcaaatcaagaagcaggtctgctgagtccgggtctgggttttgatcattatctggatatgcgtatggatgcagaagatgcagcactgggtattgaaaatgcaacaccgcgtaccattgaaggtccgctgtatgttgcgggtgcaccggaaagcgttggttatgcacgcatggatgatggtagcgatccgaatggtcataccctgattctgcatggcaccatttttgatgcagatggtaaaccgctgccgaatgcaaaagttgaaatttggcatgcaaacaccaaaggcttttatagccattttgatccgaccggtgaacagcaggcctttaatatgcgtcgtagcattattaccgatgagaatggtcagtatcgtgttcgtaccattctgcctgccggttatggttgtcctccggaaggtccgacccagcaactgctgaaccaactgggtcgtcatggtaatcgtccggcacatattcattattttgttagcgcagatggtcaccgtaaactgaccacccagattaatgttgccggtgatccgtatacctatgatgattttgcatatgccacccgtgaaggtctggttgttgatgcagttgaacataccgatccggaagcaattaaagccaatgatgtggaaggtccttttgccgaaatggtgtttgatctgaaactgacccgtctggttgatggtgttgataatcaggttgtggatcgtccgcgtctggcagtttaatacaccaaaatggttcaaaattatcaggcgagtgatcatgatcactggcctgtttttatttcagggaagggtggagacaattacgtggataatcagatcatccaagaaaccgtggataaaattctgagcgttctgccgaatcaggcaggtcagctggcacgtctggtgcgtctgatgcaatttgcatgcgatccgaccattaccgttattggcaaatataaccatggtaaaagccgtctgctgaatgaactgattggcaccgatatctttagcgttgcagataaacgtgaaaccattcagctggccgaacataaacaggatcaggttcgttggctggatgcacctggtctggatgccgatgttgcagcagttgatgatcgtcatgcatttgaagcagtttggacccaggcagatattcgtctgtttgttcatagcgttcgtgaaggtgaactggatgcaaccgaacaccatctgctgcaacagctgattgaagatgccgatcatagccgtcgtcagaccattctggttctgacccagattgatcagattccggatcagaccatcctgacacagattaaaaccagcattgcacagcaggttccgaaactggatatttgggcagttagcgcaacccgtcatcgtcagggcattgaaaacggtaaaaccctgctgatcgaaaaaagcggtattggtgcactgcgccataccctggaacaggcactggcacaggtgccgagcgcacgtacctatgaaaaaaatcgtctgctgtcagatctgcaccatcagctgaaacaactgctgctggatcagaaacatgttctgcaacaactgcaacagacacagcaacagcagctgcatgattttgataccggtctgattaacattctggacaaaattcgtgttgatctggaaccgattgtgaatattgatggtcaggatcaagcactgaatccggatagctttgcaaccatgtttaaaaacaccgcagcaaaacagcagcgtgccaaagttcagattgcatatagccgtgcatgcattgaaatcaacagccatctgattcgccatggtgttgttggtctgcctgcggaacagcagaccaccattaaaagcattgataccgtgattgttgccgtgtttggtatcagcgttaaatttcgtgatcagctgcgtgccctgttttataccgataccgaacgtcagcgtctgcaacgtgaatttcgtttctattttgaaaaaagtgccggtcgcatgattctggcagcaaaaattgaacagaccatgcgtcagcagggctgtattcagaatgccatgatggcactgcaacaaatggaaagcgcagcataaaaacacggacgccgcaaacggcgtccgaatttcttggtcgaccgttaaatctatcaccgcaagggataaatatctaacaccgtgcgtgttgactattttacctctggcggtgataatggttgcatgtactaatctagataaggaatatagccatgaccgcaccgattcaggatctgcgtgatgcaattgccctgctgcaacagcatgataatcagtatctggaaaccgatcatccggttgatccgaatgcagaactggcaggcgtttatcgtcatattggtgccggtggcaccgttaaacgtccgacccgtattggtccggcaatgatgtttaataacattaaaggttatccgcacagccgtattctggttggtatgcatgcaagccgtcagcgtgcagcactgctgctgggttgtgaagcaagtcagctggcactggaagttggtaaagcagttaaaaaaccggttgcaccggtggttgttccggcaagcagcgcaccgtgtcaagagcagatttttctggcagatgatccggattttgatctgcgtaccctgctgcctgcacataccaataccccgattgatgcaggtccgtttttttgtctgggtctggccctggcaagcgatccggtggatgcaagcctgaccgatgttaccattcatcgtctgtgtgttcagggtcgtgatgaactgagcatgttcctggcagcaggtcgccatattgaagtttttcgtcagaaagcagaagcagcaggtaaaccgctgccgattaccattaatatgggtctggacccagcaatctatattggcgcatgttttgaagcaccgaccaccccgtttggttataatgaactgggtgttgccggtgcactgcgtcagcgtccggttgaactggttcagggtgttagcgttccggaaaaagcaattgcacgtgccgaaattgttattgaaggtgaactgctgcctggtgttcgtgttcgtgaagatcagcataccaattcaggtcatgcaatgccggaatttccgggttattgtggtggtgcaaatccgagcctgccggttattaaagttaaagccgttaccatgcgcaataacgcaattctgcaaaccctggttggtccgggtgaagaacataccaccctggcaggtctgccgaccgaagcaagcatttggaatgcagttgaagcagcaattccgggttttctgcaaaatgtttatgcccataccgcaggcggtggtaaatttctgggtattctgcaagtgaaaaaacgtcagcctgccgatgaaggtcgtcagggtcaggcagccctgctggcgctggcaacctatagcgaactgaaaaatatcattctggtggatgaggatgtggacatttttgatagtgatgatattctgtgggcaatgaccacccgtatgcagggtgatgttagcattaccaccattccgggtattcgcggtcatcagctggacccgagccagacaccggaatattcaccgagcattcgtggtaatggtattagctgcaaaaccatctttgattgtaccgttccgtgggcactgaaaagccattttgaacgtgcaccgtttgcagatgttgatccgcgtccgtttgcacctgaatattttgcacgtctggaaaaaaatcagggcagcgcaaaataagctaataacaggcctgctggtaatcgcaggaatttttatttggatggatccgcctacctagcttccaagaaagatatcctaacagcacaagagcggaaagatgttttgttctacatccagaacaacctctgctaaaattcctgaaaaattttgcaaaaagttgttgactttatctacaaggtgtggtataataatcttaacaacagcaggacgctcccgggttgaggaaaacctaatgaaactgaccagcctgcgtgttagcctgctggcactgggtctggttaccagcggttttgcagcagcagaaacctataccgttgatcgttatcaggatgatagcgaaaaaggtagcctgcgttgggcaattgaacagagcaatgcaaatagcgcacaagaaaaccagattctgattcaggcagttggtaaagcaccgtatgttatcaaagttgataaaccgctgcctccgattaaaagcagcgttaaaatcattggcaccgagtgggataaaaccggtgaatttattgcaattgatggcagcaactatatcaaaggcgaaggtgaaaaagcatgtccgggtgcaaatccgggtcagtatggcaccaatgttcgtaccatgaccctgcctggtctggttctgcaagatgttaatggtgttaccctgaaaggtctggatgttcatcgtttttgtattggtgttctggttaatcgcagcagcaataacctgattcagcataatcgtatcagcaacaattatggtggtgccggtgttatgattaccggtgatgatggtaaaggtaatccgaccagcaccaccaccaataataacaaagttctggataacgtgttcatcgataatggtgatggtctggaactgacccgtggtgcagcatttaatctgattgcaaataacctgtttaccagcacaaaagccaatccggaaccgagccagggtattgaaattctgtggggtaatgataatgccgtggtgggtaacaaattcgaaaactattcagatggcctgcaaatcaattggggtaaacgtaactatatcgcctataacgaactgaccaataacagcctgggtttcaatctgacaggtgatggtaacattttcgacagcaataaagtgcatggtaaccgtattggtattgccattcgtagtgaaaaagatgccaatgcacgtattaccctgaccaaaaatcagatttgggataacggcaaagatatcaaacgttgtgaagccggtggtagctgtgttccgaatcagcgtctgggtgcaattgtttttggtgttccggcactggaacatgaaggttttgttggtagccgtggcggtggtgttgttattgaaccggcaaaactgcaaaaaacctgcacccagccgaaccagcagaattgtaatgcaattcctaatcagggtattcaggcaccgaaactgacagttagcaaaaaacagctgaccgttgaagttaaaggcacccctaatcagcgttataatgtggaattttttggcaatcgtaatgccagcagcagcgaagcagaacagtatctgggtagcattgttgttgttaccgatcatcagggtctggcaaaagcaaattgggctccgaaagttagcatgccgagcgttaccgcaaatgtgacagatcatctgggtgcgaccagcgaactgagcagcgcagttaaaatgcgttaaatgcatgcgcgccgcgttcgcgcggcgcttttttttggtactcagtagcgctgtctggcaacataaacggccccttctgggcaatgccgatcagttaaggattagttgaccgatccttaaactgaggcactataacggcttc

SEQ ID NO: 42 - DNA, 594 bp, Klebsiella pneumoniae
  gene (1)..(594): Nucleotide sequence of Klebsiella pneumoniae kpdB gene.
atgaaactgattattgggatgacgggggccaccggggcaccgcttggggtggcattgctgcaggcgctgcgcgatatgccggaggtggaaacccatctggtgatgtcgaaatgggccaaaaccaccatcgagctggaaacgccctggacggcgcgcgaagtggccgcgctggcggacttttcccacagcccggcagaccaggccgccaccatctcatccggttcatttcgtaccgacggcatgatcgttattccctgcagtatgaaaacgcttgcaggcattcgcgcgggttatgccgaagggctggtgggccgcgcggcggacgtggtgctcaaagaggggcgcaagctggtgttggtcccgcgggaaatgccgctcagcacgatccatctggagaacatgctggcgctgtcccgcatgggcgtggcgatggtcccgccgatgccagcttactacaaccacccggagacggttgacgatatcaccaatcatatcgtcacccgggtgctggatcagtttggcctcgactatcacaaagcgcgccgctggaacggcttgcgcacggcagaacaatttgcacaggagatcgaataa

SEQ ID NO: 43 - protein, 197 aa, Klebsiella pneumoniae
  PEPTIDE (1)..(197): Amino acid sequence of KpdB protein of Klebsiella pneumoniae
MKLIIGMTGATGAPLGVALLQALRDMPEVETHLVMSKWAKTTIELETPWTAREVAALADFSHSPADQAATISSGSFRTDGMIVIPCSMKTLAGIRAGYAEGLVGRAADVVLKEGRKLVLVPREMPLSTIHLENMLALSRMGVAMVPPMPAYYNHPETVDDITNHIVTRVLDQFGLDYHKARRWNGLRTAEQFAQEIE

SEQ ID NO: 44 - DNA, 570 bp, Escherichia coli
  gene (1)..(570): Nucleotide sequence of Escherichia coli  ubiX gene
atgaaacgactcattgtaggcatcagcggtgccagcggcgcgatttatggcgtgcgcttattacaggttctgcgcgatgtcgcagatatcgaaacgcatctggtgatgagccaggcggcgcgccagaccttatccctcgaaacgggtttttccctgcgcgaagtgcaggcattagctgatgtcacgcacgatgcgcgcgatattgccgccagcatctcttccggttctttccagacgctggggatggttattttaccctgttcaatcaaaaccctttccggcattgtccatagctacaccgatggtttactgacccgtgcggcagatgtggtgctgaaagagcgtcgcccgttggtgctctgcgtgcgtgaaacaccattgcacttaggccatctgcgtttaatgactcaggcagcagaaatcggtgcggtgattatgcctcccgttccggcgttttatcatcgcccacagtcccttgatgatgtgataaatcagacggttaatcgtgttcttgaccagtttgcgataacccttcctgaagatctctttgcccgctggcagggcgcataa

SEQ ID NO: 45 - protein, 189 aa, Escherichia coli
  PEPTIDE (1)..(189)
MKRLIVGISGASGAIYGVRLLQVLRDVADIETHLVMSQAARQTLSLETGFSLREVQALADVTHDARDIAASISSGSFQTLGMVILPCSIKTLSGIVHSYTDGLLTRAADVVLKERRPLVLCVRETPLHLGHLRLMTQAAEIGAVIMPPVPAFYHRPQSLDDVINQTVNRVLDQFAITLPEDLFARWQGA

SEQ ID NO: 46 - DNA, 594 bp, Escherichia coli
  gene (1)..(594): Nucleotide sequence of Escherichia coli Wstrain elw  gene
atgaaactgatcgtcgggatgacaggggctaccggtgcgcctcttggtgtggcattactgcaagcgctgcgggagatgccgaatgtcgagactcatctggtgatgtcgaagtgggcgaaaaccaccattgaactggaaacgccttacagcgctcgcgatgttgctgccctcgcagacttcagccataacccggcggatcaggcggcgatcatctcatccggttcttttcgtaccgacggcatgatcgttattccgtgcagtatgaaaacgctcgccggtatccgcgctggttacgccgatggcctggtagggcgcgcggcggacgtcgtgctcaaagaaggccgcaaactggtgctggtgccgcgtgaaatgccgcttagcaccatccatctcgaaaatatgctcgcactttcacgcatgggcgtggcgatggtgccgccgatgcctgccttttataaccatcccgaaacggtagatgacattgtccaccatgtggtagcccgcgtgctggatcaatttggcctcgaacatccccacgccaggcgctggcaaggattgccgcaggcccggaatttttctcaggagaatgaataa

SEQ ID NO: 47 - protein, 197 aa, Escherichia coli
  PEPTIDE (1)..(197): Amino acid sequence of Elw protein of Escherichia coli W strain
MKLIVGMTGATGAPLGVALLQALREMPNVETHLVMSKWAKTTIELETPYSARDVAALADFSHNPADQAAIISSGSFRTDGMIVIPCSMKTLAGIRAGYADGLVGRAADVVLKEGRKLVLVPREMPLSTIHLENMLALSRMGVAMVPPMPAFYNHPETVDDIVHHVVARVLDQFGLEHPHARRWQGLPQARNFSQENE

SEQ ID NO: 48 - DNA, 579 bp, Klebsiella oxytoca
  gene (1)..(579): Nucleotide sequence of Klebsiella oxytoca kox gene
atgacggcacgcatcatcattggtatcagcggcgcatccgggtttcagtacggcgttaaggcgctggagctactgcgcccgcatcccgttgaagtccacctggtcgtctctaaaggcgcggaaaaaacctgcgagctggagacggatcaccgcctggacgaggtgatggcgctggccgacgtggtgcatcccatcgcgaatcttggggcggctatctccagcggttcgtttaaaacgctgggaatgttgatcgcgccgtgttcaatgcgttctttaggcgccatcgcccactgcctgaccgacaacctgctcacccgcgctgcggacgtggtgctgaaagagcgtcgccgcctggtgctgctggcccgggaaacaccgctgaaccttggccatatccgcaatatggccgccgtaaccgaaatgggcggaattatctttccgccggtcccggcactttaccagcgtccgcaaacggcggacgacatcgttacccatagcgtcaatcgcgcgctcgatctgtttgacctgcaggtcaacaacatcccccgctggggtgaaggcgagctacgttttaattaa

SEQ ID NO: 49 - protein, 192 aa, Klebsiella oxytoca
  PEPTIDE (1)..(192): Amino acid sequence of Kox protein of Klebsiella oxytoca.
MTARIIIGISGASGFQYGVKALELLRPHPVEVHLVVSKGAEKTCELETDHRLDEVMALADVVHPIANLGAAISSGSFKTLGMLIAPCSMRSLGAIAHCLTDNLLTRAADVVLKERRRLVLLARETPLNLGHIRNMAAVTEMGGIIFPPVPALYQRPQTADDIVTHSVNRALDLFDLQVNNIPRWGEGELRFN

SEQ ID NO: 50 - DNA, 564 bp, Lactobacillus plantarum
  gene (1)..(564): Nucleotide sequence of Lactobacillus plantarum lpl gene
atgaaacgaattgttgtgggaatcacgggagcgtccggtacgatttacgcggtcgacttattagaaaagttacatcagcggccagatgttgaagttcatctggtaatgagtgcgtgggctaaaaaaaacttggagttagagactgattactcgctcgcgcagctgacggcgctcgcggatgctacttatcgggctaatgaccaaggcgcagcgattgccagcggttcgtttttgaatgacggaatggtcattgtcccagctagtatgaagacggtagcagggattgcgtacggcttcggtgataatttaatatcgcgggctgctgatgtcacgattaaagaacaacgtaaacttgtgattgttccacgtgaaacaccgttaagcgtgattcatttagaaaatctaacgaagttggcaaaactcggtgcccaaattattccaccgattcccgcgttttataatcatccgcaatccattcaggatctggtcaatcatcaaaccatgaaaattttagatgcgtttcatattcataatgaaactgatcgccgttgggagggggattaa

SEQ ID NO: 51 - protein, 187 aa, Lactobacillus plantarum
  PEPTIDE (1)..(187): Amino acid sequence of Lpl protein of Lactobacillus plantarum
MKRIVVGITGASGTIYAVDLLEKLHQRPDVEVHLVMSAWAKKNLELETDYSLAQLTALADATYRANDQGAAIASGSFLNDGMVIVPASMKTVAGIAYGFGDNLISRAADVTIKEQRKLVIVPRETPLSVIHLENLTKLAKLGAQIIPPIPAFYNHPQSIQDLVNHQTMKILDAFHIHNETDRRWEGD

SEQ ID NO: 52 - DNA, 200 bp, Escherichia coli
  promoter (1)..(200): Nucleotide sequence of Pgi promoter
agcggggcggttgtcaacgatggggtcatgcggatttttcatccactcctggcggtcagtagttcagctaataaatgcttcactgcgctaagggtttacactcaacattacgctaacggcactaaaaccatcacatttttctgtgactggcgctacaatcttccaaagtcacaattctcatgcagaggaggaatatagcc

SEQ ID NO: 53 - DNA, 3537 bp, Saccharomyces cerevisiae
  gene (1)..(3537): Nucleotide sequence of Saccharomyces cerevisiae pyc gene
atgtcgcaaagaaaattcgccggcttgagagataacttcaatctcttgggtgaaaagaacaaaatattggtggctaatagaggagaaattccaatcagaatttttcgtaccgctcatgaactgtctatgcagacggtagctatatattctcatgaagatcgtctttcaacgcacaaacaaaaggctgacgaagcatacgtcataggtgaagtaggccaatatacccccgtcggcgcttatttggccattgacgaaatcatttccattgcccaaaaacaccaggtagatttcatccatccaggttatgggttcttgtctgaaaattcggaatttgccgacaaagtagtgaaggccggtatcacttggattggccctccagctgaagttattgactccgtgggtgataaggtctcagctagaaacctggcagcaaaagctaatgtgcccaccgttcctggtacaccaggtcctatagaaactgtagaggaagcacttgacttcgtcaatgaatacggctacccggtgatcattaaggccgcctttggtggtggtggtagaggtatgagagtcgttagagaaggtgacgacgtggcagatgcctttcaacgtgctacctccgaagcccgtactgccttcggtaatggtacctgctttgtggaaagattcttggacaagccaaagcatattgaagttcaattgttggccgataaccacggaaacgtggttcatcttttcgaaagagactgttccgtgcagagaagacaccaaaaggttgtcgaagtggccccagcaaagactttaccccgtgaagtccgtgacgccattttgacagatgcagttaaattggccaaagagtgtggctacagaaatgcgggtactgctgaattcttggttgataaccaaaatagacactatttcattgaaattaatccaagaatccaagtggaacataccatcacagaagaaattaccggtatagatattgtggcggctcagatccaaattgcggcaggtgcctctctaccccagctgggcctattccaggacaaaattacgactcgtggctttgccattcagtgccgtattaccacggaagaccctgctaagaacttccaaccagataccggtagaatagaagtgtaccgttctgcaggtggtaatggtgttagactggatggtggtaacgcctatgcaggaacaataatctcacctcattacgactcaatgctggtcaaatgctcatgctccggttccacctacgaaatcgttcgtagaaaaatgattcgtgcattaatcgagttcagaattagaggtgtcaagaccaacattcccttcctattgactcttttgaccaatccagtatttattgagggtacatactggacgacttttattgacgacaccccacaactgttccaaatggtttcatcacaaaacagagcccaaaaacttttacattacctcgccgacgtggcagtcaatggttcatctatcaagggtcaaattggcttgccaaaattaaaatcaaatccaagtgtcccccatttgcacgatgctcagggcaatgtcatcaacgttacaaagtctgcaccaccatccggatggaggcaagtgctactagaaaaggggccagctgaatttgccagacaagttagacagttcaatggtactttattgatggacaccacctggagagacgctcatcaatctctacttgcaacaagagtcagaacccacgatttggctacaatcgctccaacaaccgcacatgcccttgcaggtcgtttcgccttagaatgttggggtggtgccacattcgatgttgcaatgagatttttgcatgaggatccatgggaacgtttgagaaaattaagatctctggtgcctaatattccattccaaatgttattgcgtggtgccaatggtgtggcttattcttcattgcctgacaatgctattgaccatttcgtcaagcaagccaaggataatggtgttgatatatttagagtctttgatgccttaaatgacttggaacaattgaaggtcggtgtagatgctgtgaagaaggcaggtggtgttgtagaagccactgtttgtttctctggggatatgcttcagccaggcaagaaatacaatttggattactacttggaaattgctgaaaaaattgtccaaatgggcactcatatcctgggtatcaaagatatggcaggtaccatgaagccagcagctgccaaactactgattggatctttgagggctaagtaccctgatctcccaatacatgttcacactcacgattctgcaggtactgctgttgcatcaatgactgcgtgtgctctggcgggcgccgatgtcgttgatgttgccatcaactcaatgtctggtttaacttcacaaccatcaatcaatgctctgttggcttcattagaaggtaatattgacactggtattaacgttgagcatgtccgtgaactagatgcatattgggcagagatgagattgttatactcttgtttcgaggctgacttgaagggcccagatccagaagtttatcaacatgaaatcccaggtggtcaattgacaaacttgttgtttcaagcccaacaattgggtcttggagaacaatgggccgaaacaaaaagagcttacagagaagccaattatttattgggtgatattgtcaaagttaccccaacttcgaaggtcgttggtgatctggcacaatttatggtctccaataaattaacttccgatgatgtgagacgcctggctaattctttggatttccctgactctgttatggatttcttcgaaggcttaatcggccaaccatatggtgggttcccagaaccatttagatcagacgttttaaggaacaagagaagaaagttgacttgtcgtccaggcctggaactagagccatttgatctcgaaaaaattagagaagacttgcagaatagatttggtgatgttgatgagtgcgacgttgcttcttataacatgtacccaagagtttatgaagacttccaaaagatgagagaaacgtatggtgatttatctgtattgccaacaagaagctttttgtctccactagagactgacgaagaaattgaagttgtaatcgaacaaggtaaaacgctaattatcaagctacaggctgtgggtgatttgaacaaaaagaccggtgaaagagaagtttactttgatttgaatggtgaaatgagaaaaattcgtgttgctgacagatcacaaaaagtggaaactgttactaaatccaaagcagacatgcatgatccattacacattggtgcaccaatggcaggtgtcattgttgaagttaaagttcataaaggatcactaataaagaagggccaacctgtagccgtattaagcgccatgaaaatggaaatgattatatcttctccatccgatggacaagttaaagaagtgtttgtctctgatggtgaaaatgtggactcttctgatttattagttctattagaagaccaagttcctgttgaaactaaggcatga

SEQ ID NO: 54 - protein, 1178 aa, Escherichia coli
  PEPTIDE (1)..(1178): Amino acid sequence of Pyc protein of Saccharomyces cerevisiae
MSQRKFAGLRDNFNLLGEKNKILVANRGEIPIRIFRTAHELSMQTVAIYSHEDRLSTHKQKADEAYVIGEVGQYTPVGAYLAIDEIISIAQKHQVDFIHPGYGFLSENSEFADKVVKAGITWIGPPAEVIDSVGDKVSARNLAAKANVPTVPGTPGPIETVEEALDFVNEYGYPVIIKAAFGGGGRGMRVVREGDDVADAFQRATSEARTAFGNGTCFVERFLDKPKHIEVQLLADNHGNVVHLFERDCSVQRRHQKVVEVAPAKTLPREVRDAILTDAVKLAKECGYRNAGTAEFLVDNQNRHYFIEINPRIQVEHTITEEITGIDIVAAQIQIAAGASLPQLGLFQDKITTRGFAIQCRITTEDPAKNFQPDTGRIEVYRSAGGNGVRLDGGNAYAGTIISPHYDSMLVKCSCSGSTYEIVRRKMIRALIEFRIRGVKTNIPFLLTLLTNPVFIEGTYWTTFIDDTPQLFQMVSSQNRAQKLLHYLADVAVNGSSIKGQIGLPKLKSNPSVPHLHDAQGNVINVTKSAPPSGWRQVLLEKGPAEFARQVRQFNGTLLMDTTWRDAHQSLLATRVRTHDLATIAPTTAHALAGRFALECWGGATFDVAMRFLHEDPWERLRKLRSLVPNIPFQMLLRGANGVAYSSLPDNAIDHFVKQAKDNGVDIFRVFDALNDLEQLKVGVDAVKKAGGVVEATVCFSGDMLQPGKKYNLDYYLEIAEKIVQMGTHILGIKDMAGTMKPAAAKLLIGSLRAKYPDLPIHVHTHDSAGTAVASMTACALAGADVVDVAINSMSGLTSQPSINALLASLEGNIDTGINVEHVRELDAYWAEMRLLYSCFEADLKGPDPEVYQHEIPGGQLTNLLFQAQQLGLGEQWAETKRAYREANYLLGDIVKVTPTSKVVGDLAQFMVSNKLTSDDVRRLANSLDFPDSVMDFFEGLIGQPYGGFPEPFRSDVLRNKRRKLTCRPGLELEPFDLEKIREDLQNRFGDVDECDVASYNMYPRVYEDFQKMRETYGDLSVLPTRSFLSPLETDEEIEVVIEQGKTLIIKLQAVGDLNKKTGEREVYFDLNGEMRKIRVADRSQKVETVTKSKADMHDPLHIGAPMAGVIVEVKVHKGSLIKKGQPVAVLSAMKMEMIISSPSDGQVKEVFVSDGENVDSSDLLVLLEDQVPVETKA

SEQ ID NO: 55 - DNA, 6273 bp, Escherichia coli
  misc_feature (1)..(6273): DNA sequence of the plasmid pCAT350
tgaatgacctttaatagattatattactaattaattggggaccctagaggtccccttttttattttaaaaattttttcacaaaacggtttacaagcatacgttggccgattcattaatgcagctggcacgacaggtttcccgactggaaagcgggcagtgagcgcaacgcaattaatgtgagttagctcactcattaggcaccccaggctttacactttatgcttccggctcgtatgttgtgtggaattgtgagcggataacaatttcacacaggaaacagctatgaccatgattacgccaagcttgcatgcctgcaggtcgactctagaggatccccgggtaccgagctcgaattcactggccgtcgttttacaacgtcgtgactgggaaaaccctggcgttacccaacttaatcgccttgcagcacatccccctttcgccagctggcgtaatagcgaagaggcccgcaccgatcgcccttcccaacagttgcgcagcctgaatggcgaatggcgcctgatgcggtattttctccttacgcatctgtgcggtatttcacaccgcatatggtgcactctcagtacaatctgctctgatgccgcatagttaagccagccccgacacccgccaacacccgctgacgaattcgttgacagtaagacgggtaagcctgttgatgataccgctgccttactgggtgcattagccagtctgaatgacctgtcacgggataatccgaagtggtcagactggaaaatcagagggcaggaactgctgaacagcaaaaagtcagatagcaccacatagcagacccgccataaaacgccctgagaagcccgtgacgggcttttcttgtattatgggtagtttccttgcatgaatccataaaaggcgcctgtagtgccatttacccccattcactgccagagccgtgagcgcagcgaactgaatgtcacgaaaaagacagcgactcaggtgcctgatggtcggagacaaaaggaatattcagcgatttgcccgagcttgcgagggtgctacttaagcctttagggttttaaggtctgttttgtagaggagcaaacagcgtttgcgacatccttttgtaatactgcggaactgactaaagtagtgagttatacacagggctgggatctattctttttatctttttttattctttctttattctataaattataaccacttgaatataaacaaaaaaaacacacaaaggtctagcggaatttacagagggtctagcagaatttacaagttttccagcaaaggtctagcagaatttacagatacccacaactcaaaggaaaaggactagtaattatcattgactagcccatctcaattggtatagtgattaaaatcacctagaccaattgagatgtatgtctgaattagttgttttcaaagcaaatgaactagcgattagtcgctatgacttaacggagcatgaaaccaagctaattttatgctgtgtggcactactcaaccccacgattgaaaaccctacaaggaaagaacggacggtatcgttcacttataaccaatacgctcagatgatgaacatcagtagggaaaatgcttatggtgtattagctaaagcaaccagagagctgatgacgagaactgtggaaatcaggaatcctttggttaaaggctttgagattttccagtggacaaactatgccaagttctcaagcgaaaaattagaattagtttttagtgaagagatattgccttatcttttccagttaaaaaaattcataaaatataatctggaacatgttaagtcttttgaaaacaaatactctatgaggatttatgagtggttattaaaagaactaacacaaaagaaaactcacaaggcaaatatagagattagccttgatgaatttaagttcatgttaatgcttgaaaataactaccatgagtttaaaaggcttaaccaatgggttttgaaaccaataagtaaagatttaaacacttacagcaatatgaaattggtggttgataagcgaggccgcccgactgatacgttgattttccaagttgaactagatagacaaatggatctcgtaaccgaacttgagaacaaccagataaaaatgaatggtgacaaaataccaacaaccattacatcagattcctacctacgtaacggactaagaaaaacactacacgatgctttaactgcaaaaattcagctcaccagttttgaggcaaaatttttgagtgacatgcaaagtaagcatgatctcaatggttcgttctcatggctcacgcaaaaacaacgaaccacactagagaacatactggctaaatacggaaggatctgaggttcttatggcaaacacggacgccgcaaacggcgtccgaatttcttggtcgaccgttaaatctatcaccgcaagggataaatatctaacaccgtgcgtgttgactattttacctctggcggtgataatggttgcatgtactaatctagataaggaatatagccatggaagtgaaaatcttcaacacccaggatgttcaggattttctgcgtgttgcaagcggtctggaacaagagggtggtaatccgcgtgttaaacaaattattcatcgtgttctgagcgacctgtataaagcaattgaagatctgaatatcaccagcgacgaatattgggcaggcgttgcatatctgaatcagctgggtgcaaatcaagaagcaggtctgctgagtccgggtctgggttttgatcattatctggatatgcgtatggatgcagaagatgcagcactgggtattgaaaatgcaacaccgcgtaccattgaaggtccgctgtatgttgcgggtgcaccggaaagcgttggttatgcacgcatggatgatggtagcgatccgaatggtcataccctgattctgcatggcaccatttttgatgcagatggtaaaccgctgccgaatgcaaaagttgaaatttggcatgcaaacaccaaaggcttttatagccattttgatccgaccggtgaacagcaggcctttaatatgcgtcgtagcattattaccgatgagaatggtcagtatcgtgttcgtaccattctgcctgccggttatggttgtcctccggaaggtccgacccagcaactgctgaaccaactgggtcgtcatggtaatcgtccggcacatattcattattttgttagcgcagatggtcaccgtaaactgaccacccagattaatgttgccggtgatccgtatacctatgatgattttgcatatgccacccgtgaaggtctggttgttgatgcagttgaacataccgatccggaagcaattaaagccaatgatgtggaaggtccttttgccgaaatggtgtttgatctgaaactgacccgtctggttgatggtgttgataatcaggttgtggatcgtccgcgtctggcagtttaatacaccaaaatggttcaaaattatcaggcgagtgatcatgatcactggcctgtttttatttcagggaagggtggagacaattacgtggataatcagatcatccaagaaaccgtggataaaattctgagcgttctgccgaatcaggcaggtcagctggcacgtctggtgcgtctgatgcaatttgcatgcgatccgaccattaccgttattggcaaatataaccatggtaaaagccgtctgctgaatgaactgattggcaccgatatctttagcgttgcagataaacgtgaaaccattcagctggccgaacataaacaggatcaggttcgttggctggatgcacctggtctggatgccgatgttgcagcagttgatgatcgtcatgcatttgaagcagtttggacccaggcagatattcgtctgtttgttcatagcgttcgtgaaggtgaactggatgcaaccgaacaccatctgctgcaacagctgattgaagatgccgatcatagccgtcgtcagaccattctggttctgacccagattgatcagattccggatcagaccatcctgacacagattaaaaccagcattgcacagcaggttccgaaactggatatttgggcagttagcgcaacccgtcatcgtcagggcattgaaaacggtaaaaccctgctgatcgaaaaaagcggtattggtgcactgcgccataccctggaacaggcactggcacaggtgccgagcgcacgtacctatgaaaaaaatcgtctgctgtcagatctgcaccatcagctgaaacaactgctgctggatcagaaacatgttctgcaacaactgcaacagacacagcaacagcagctgcatgattttgataccggtctgattaacattctggacaaaattcgtgttgatctggaaccgattgtgaatattgatggtcaggatcaagcactgaatccggatagctttgcaaccatgtttaaaaacaccgcagcaaaacagcagcgtgccaaagttcagattgcatatagccgtgcatgcattgaaatcaacagccatctgattcgccatggtgttgttggtctgcctgcggaacagcagaccaccattaaaagcattgataccgtgattgttgccgtgtttggtatcagcgttaaatttcgtgatcagctgcgtgccctgttttataccgataccgaacgtcagcgtctgcaacgtgaatttcgtttctattttgaaaaaagtgccggtcgcatgattctggcagcaaaaattgaacagaccatgcgtcagcagggctgtattcagaatgccatgatggcactgcaacaaatggaaagcgcagcataagtctgacaggtgccggatttcatatccggcacttactttccttaactcttcgccttaacgcaaaatctcacactgatgatcctgaatttcctcggctgaagcacggttaagcgtcagtagatttcgttgtgtcgccagcaatacaaatgatggacataagcctgttcggttcgtaagctgtaatgcaagtagcgtatgcgctcacgcaactggtccagaaccttgaccgaacgcagcggtggtaacggcgcagtggcggttttcatggcttgttatgactgtttttttggggtacagtctatgcctcgggcatccaagcagcaagcgcgttacgccgtgggtcgatgtttgatgttatggagcagcaacgatgttacgcagcagggcagtcgccctaaaacaaagttaaacatcatgagggaagcggtgatcgccgaagtatcgactcaactatcagaggtagttggcgtcatcgagcgccatctcgaaccgacgttgctggccgtacatttgtacggctccgcagtggatggcggcctgaagccacacagtgatattgatttgctggttacggtgaccgtaaggcttgatgaaacaacgcggcgagctttgatcaacgaccttttggaaacttcggcttcccctggagagagcgagattctccgcgctgtagaagtcaccattgttgtgcacgacgacatcattccgtggcgttatccagctaagcgcgaactgcaatttggagaatggcagcgcaatgacattcttgcaggtatcttcgagccagccacgatcgacattgatctggctatcttgctgacaaaagcaagagaacatagcgttgccttggtaggtccagcggcggaggaactctttgatccggttcctgaacaggatctatttgaggcgctaaatgaaaccttaacgctatggaactcgccgcccgactgggctggcgatgagcgaaatgtagtgcttacgttgtcccgcatttggtacagcgcagtaaccggcaaaatcgcgccgaaggatgtcgctgccgactgggcaatggagcgcctgccggcccagtatcagcccgtcatacttgaagctagacaggcttatcttggacaagaagaagatcgcttggcctcgcgcgcagatcagttggaagaatttgtccactacgtgaaaggcgagatcaccaaggtagtcggcaaataatgtctaacaattcgttcaagccgacgccgcttcgcggcgcggcttaactcaagcgttagatgcactaagcacataattgctcacagccaaactatcaggtcaagtctgcttttattatttttaagcgtgcataataagccctacacaaattgggagatatatcatgaaaggctggctttttcttgttatcgcaatagttggcgaagtaatcgcaacatccgcattaaaatctagcgagggctttactaagctgatccggtggatgaccttt

SEQ ID NO: 56 - DNA, 3943 bp, Escherichia coli
  misc_feature (1)..(3943): DNA sequence of the plasmid pCP165
tgaatgacctttaatagattatattactaattaattggggaccctagaggtccccttttttattttaaaaattttttcacaaaacggtttacaagcatacgttggccgattcattaatgcagctggcacgacaggtttcccgactggaaagcgggcagtgagcgcaacgcaattaatgtgagttagctcactcattaggcaccccaggctttacactttatgcttccggctcgtatgttgtgtggaattgtgagcggataacaatttcacacaggaaacagctatgaccatgattacgccaagcttgcatgcctgcaggtcgactctagaggatccccgggtaccgagctcgaattcactggccgtcgttttacaacgtcgtgactgggaaaaccctggcgttacccaacttaatcgccttgcagcacatccccctttcgccagctggcgtaatagcgaagaggcccgcaccgatcgcccttcccaacagttgcgcagcctgaatggcgaatggcgcctgatgcggtattttctccttacgcatctgtgcggtatttcacaccgcatatggtgcactctcagtacaatctgctctgatgccgcatagttaagccagccccgacacccgccaacacccgctgacgaattcgttgacagtaagacgggtaagcctgttgatgataccgctgccttactgggtgcattagccagtctgaatgacctgtcacgggataatccgaagtggtcagactggaaaatcagagggcaggaactgctgaacagcaaaaagtcagatagcaccacatagcagacccgccataaaacgccctgagaagcccgtgacgggcttttcttgtattatgggtagtttccttgcatgaatccataaaaggcgcctgtagtgccatttacccccattcactgccagagccgtgagcgcagcgaactgaatgtcacgaaaaagacagcgactcaggtgcctgatggtcggagacaaaaggaatattcagcgatttgcccgagcttgcgagggtgctacttaagcctttagggttttaaggtctgttttgtagaggagcaaacagcgtttgcgacatccttttgtaatactgcggaactgactaaagtagtgagttatacacagggctgggatctattctttttatctttttttattctttctttattctataaattataaccacttgaatataaacaaaaaaaacacacaaaggtctagcggaatttacagagggtctagcagaatttacaagttttccagcaaaggtctagcagaatttacagatacccacaactcaaaggaaaaggactagtaattatcattgactagcccatctcaattggtatagtgattaaaatcacctagaccaattgagatgtatgtctgaattagttgttttcaaagcaaatgaactagcgattagtcgctatgacttaacggagcatgaaaccaagctaattttatgctgtgtggcactactcaaccccacgattgaaaaccctacaaggaaagaacggacggtatcgttcacttataaccaatacgctcagatgatgaacatcagtagggaaaatgcttatggtgtattagctaaagcaaccagagagctgatgacgagaactgtggaaatcaggaatcctttggttaaaggctttgagattttccagtggacaaactatgccaagttctcaagcgaaaaattagaattagtttttagtgaagagatattgccttatcttttccagttaaaaaaattcataaaatataatctggaacatgttaagtcttttgaaaacaaatactctatgaggatttatgagtggttattaaaagaactaacacaaaagaaaactcacaaggcaaatatagagattagccttgatgaatttaagttcatgttaatgcttgaaaataactaccatgagtttaaaaggcttaaccaatgggttttgaaaccaataagtaaagatttaaacacttacagcaatatgaaattggtggttgataagcgaggccgcccgactgatacgttgattttccaagttgaactagatagacaaatggatctcgtaaccgaacttgagaacaaccagataaaaatgaatggtgacaaaataccaacaaccattacatcagattcctacctacgtaacggactaagaaaaacactacacgatgctttaactgcaaaaattcagctcaccagttttgaggcaaaatttttgagtgacatgcaaagtaagcatgatctcaatggttcgttctcatggctcacgcaaaaacaacgaaccacactagagaacatactggctaaatacggaaggatctgaggttcttatggcaaacacggacgccgcaaacggcgtccgaatttcttggtcgaccgttaaatctatcaccgcaagggataaatatctaacaccgtgcgtgttgactattttacctctggcggtgataatggttgcatgtactaatctagataaggaatatagccttagatttgactgaaatcgtacagtaaaaagcgtacaataaaggctccacgaaagtggggccttttttagcgcgagagccttttttgtcagctatctatatggacataagcctgttcggttcgtaagctgtaatgcaagtagcgtatgcgctcacgcaactggtccagaaccttgaccgaacgcagcggtggtaacggcgcagtggcggttttcatggcttgttatgactgtttttttggggtacagtctatgcctcgggcatccaagcagcaagcgcgttacgccgtgggtcgatgtttgatgttatggagcagcaacgatgttacgcagcagggcagtcgccctaaaacaaagttaaacatcatgagggaagcggtgatcgccgaagtatcgactcaactatcagaggtagttggcgtcatcgagcgccatctcgaaccgacgttgctggccgtacatttgtacggctccgcagtggatggcggcctgaagccacacagtgatattgatttgctggttacggtgaccgtaaggcttgatgaaacaacgcggcgagctttgatcaacgaccttttggaaacttcggcttcccctggagagagcgagattctccgcgctgtagaagtcaccattgttgtgcacgacgacatcattccgtggcgttatccagctaagcgcgaactgcaatttggagaatggcagcgcaatgacattcttgcaggtatcttcgagccagccacgatcgacattgatctggctatcttgctgacaaaagcaagagaacatagcgttgccttggtaggtccagcggcggaggaactctttgatccggttcctgaacaggatctatttgaggcgctaaatgaaaccttaacgctatggaactcgccgcccgactgggctggcgatgagcgaaatgtagtgcttacgttgtcccgcatttggtacagcgcagtaaccggcaaaatcgcgccgaaggatgtcgctgccgactgggcaatggagcgcctgccggcccagtatcagcccgtcatacttgaagctagacaggcttatcttggacaagaagaagatcgcttggcctcgcgcgcagatcagttggaagaatttgtccactacgtgaaaggcgagatcaccaaggtagtcggcaaataatgtctaacaattcgttcaagccgacgccgcttcgcggcgcggcttaactcaagcgttagatgcactaagcacataattgctcacagccaaactatcaggtcaagtctgcttttattatttttaagcgtgcataataagccctacacaaattgggagatatatcatgaaaggctggctttttcttgttatcgcaatagttggcgaagtaatcgcaacatccgcattaaaatctagcgagggctttactaagctgatccggtggatgaccttt

SEQ ID NO: 57 - DNA, 10863 bp, Escherichia coli
  misc_feature (1)..(10863): DNA sequence of the plasmid pCP140
tggacataagcctgttcggttcgtaagctgtaatgcaagtagcgtatgcgctcacgcaactggtccagaaccttgaccgaacgcagcggtggtaacggcgcagtggcggttttcatggcttgttatgactgtttttttggggtacagtctatgcctcgggcatccaagcagcaagcgcgttacgccgtgggtcgatgtttgatgttatggagcagcaacgatgttacgcagcagggcagtcgccctaaaacaaagttaaacatcatgagggaagcggtgatcgccgaagtatcgactcaactatcagaggtagttggcgtcatcgagcgccatctcgaaccgacgttgctggccgtacatttgtacggctccgcagtggatggcggcctgaagccacacagtgatattgatttgctggttacggtgaccgtaaggcttgatgaaacaacgcggcgagctttgatcaacgaccttttggaaacttcggcttcccctggagagagcgagattctccgcgctgtagaagtcaccattgttgtgcacgacgacatcattccgtggcgttatccagctaagcgcgaactgcaatttggagaatggcagcgcaatgacattcttgcaggtatcttcgagccagccacgatcgacattgatctggctatcttgctgacaaaagcaagagaacatagcgttgccttggtaggtccagcggcggaggaactctttgatccggttcctgaacaggatctatttgaggcgctaaatgaaaccttaacgctatggaactcgccgcccgactgggctggcgatgagcgaaatgtagtgcttacgttgtcccgcatttggtacagcgcagtaaccggcaaaatcgcgccgaaggatgtcgctgccgactgggcaatggagcgcctgccggcccagtatcagcccgtcatacttgaagctagacaggcttatcttggacaagaagaagatcgcttggcctcgcgcgcagatcagttggaagaatttgtccactacgtgaaaggcgagatcaccaaggtagtcggcaaataatgtctaacaattcgttcaagccgacgccgcttcgcggcgcggcttaactcaagcgttagatgcactaagcacataattgctcacagccaaactatcaggtcaagtctgcttttattatttttaagcgtgcataataagccctacacaaattgggagatatatcatgaaaggctggctttttcttgttatcgcaatagttggcgaagtaatcgcaacatccgcattaaaatctagcgagggctttactaagctgatccggtggatgaccttttgaatgacctttaatagattatattactaattaattggggaccctagaggtccccttttttattttaaaaattttttcacaaaacggtttacaagcatacgttggccgattcattaatgcagctggcacgacaggtttcccgactggaaagcgggcagtgagcgcaacgcaattaatgtgagttagctcactcattaggcaccccaggctttacactttatgcttccggctcgtatgttgtgtggaattgtgagcggataacaatttcacacaggaaacagctatgaccatgattacgccatcgaccgttaaatctatcaccgcaagggataaatatctaacaccgtgcgtgttgactattttacctctggcggtgataatggttgcatgtactaatctagataaggaatatagccatggaagtgaaaatcttcaacacccaggatgttcaggattttctgcgtgttgcaagcggtctggaacaagagggtggtaatccgcgtgttaaacaaattattcatcgtgttctgagcgacctgtataaagcaattgaagatctgaatatcaccagcgacgaatattgggcaggcgttgcatatctgaatcagctgggtgcaaatcaagaagcaggtctgctgagtccgggtctgggttttgatcattatctggatatgcgtatggatgcagaagatgcagcactgggtattgaaaatgcaacaccgcgtaccattgaaggtccgctgtatgttgcgggtgcaccggaaagcgttggttatgcacgcatggatgatggtagcgatccgaatggtcataccctgattctgcatggcaccatttttgatgcagatggtaaaccgctgccgaatgcaaaagttgaaatttggcatgcaaacaccaaaggcttttatagccattttgatccgaccggtgaacagcaggcctttaatatgcgtcgtagcattattaccgatgagaatggtcagtatcgtgttcgtaccattctgcctgccggttatggttgtcctccggaaggtccgacccagcaactgctgaaccaactgggtcgtcatggtaatcgtccggcacatattcattattttgttagcgcagatggtcaccgtaaactgaccacccagattaatgttgccggtgatccgtatacctatgatgattttgcatatgccacccgtgaaggtctggttgttgatgcagttgaacataccgatccggaagcaattaaagccaatgatgtggaaggtccttttgccgaaatggtgtttgatctgaaactgacccgtctggttgatggtgttgataatcaggttgtggatcgtccgcgtctggcagtttaatacaccaaaatggttcaaaattatcaggcgagtgatcatgatcactggcctgtttttatttcagggaagggtggagacaattacgtggataatcagatcatccaagaaaccgtggataaaattctgagcgttctgccgaatcaggcaggtcagctggcacgtctggtgcgtctgatgcaatttgcatgcgatccgaccattaccgttattggcaaatataaccatggtaaaagccgtctgctgaatgaactgattggcaccgatatctttagcgttgcagataaacgtgaaaccattcagctggccgaacataaacaggatcaggttcgttggctggatgcacctggtctggatgccgatgttgcagcagttgatgatcgtcatgcatttgaagcagtttggacccaggcagatattcgtctgtttgttcatagcgttcgtgaaggtgaactggatgcaaccgaacaccatctgctgcaacagctgattgaagatgccgatcatagccgtcgtcagaccattctggttctgacccagattgatcagattccggatcagaccatcctgacacagattaaaaccagcattgcacagcaggttccgaaactggatatttgggcagttagcgcaacccgtcatcgtcagggcattgaaaacggtaaaaccctgctgatcgaaaaaagcggtattggtgcactgcgccataccctggaacaggcactggcacaggtgccgagcgcacgtacctatgaaaaaaatcgtctgctgtcagatctgcaccatcagctgaaacaactgctgctggatcagaaacatgttctgcaacaactgcaacagacacagcaacagcagctgcatgattttgataccggtctgattaacattctggacaaaattcgtgttgatctggaaccgattgtgaatattgatggtcaggatcaagcactgaatccggatagctttgcaaccatgtttaaaaacaccgcagcaaaacagcagcgtgccaaagttcagattgcatatagccgtgcatgcattgaaatcaacagccatctgattcgccatggtgttgttggtctgcctgcggaacagcagaccaccattaaaagcattgataccgtgattgttgccgtgtttggtatcagcgttaaatttcgtgatcagctgcgtgccctgttttataccgataccgaacgtcagcgtctgcaacgtgaatttcgtttctattttgaaaaaagtgccggtcgcatgattctggcagcaaaaattgaacagaccatgcgtcagcagggctgtattcagaatgccatgatggcactgcaacaaatggaaagcgcagcataaaaacacggacgccgcaaacggcgtccgaatttcttggtcgactctagaggatccccgggtaccgagctcgaattcactggccgtcgttttacaacgtcgtgactgggaaaaccctggcgttacccaacttaatcgccttgcagcacatccccctttcgccagctggcgtaatagcgaagaggcccgcaccgatcgcccttcccaacagttgcgcagcctgaatggcgaatggcgcctgatgcggtattttctccttacgcatctgtgcggtatttcacaccgcatatggtgcactctcagtacaatctgctctgatgccgcatagttaagccagccccgacacccgccaacacccgctgacgaattcgttgacagtaagacgggtaagcctgttgatgataccgctgccttactgggtgcattagccagtctgaatgacctgtcacgggataatccgaagtggtcagactggaaaatcagagggcaggaactgctgaacagcaaaaagtcagatagcaccacatagcagacccgccataaaacgccctgagaagcccgtgacgggcttttcttgtattatgggtagtttccttgcatgaatccataaaaggcgcctgtagtgccatttacccccattcactgccagagccgtgagcgcagcgaactgaatgtcacgaaaaagacagcgactcaggtgcctgatggtcggagacaaaaggaatattcagcgatttgcccgagcttgcgagggtgctacttaagcctttagggttttaaggtctgttttgtagaggagcaaacagcgtttgcgacatccttttgtaatactgcggaactgactaaagtagtgagttatacacagggctgggatctattctttttatctttttttattctttctttattctataaattataaccacttgaatataaacaaaaaaaacacacaaaggtctagcggaatttacagagggtctagcagaatttacaagttttccagcaaaggtctagcagaatttacagatacccacaactcaaaggaaaaggactagtaattatcattgactagcccatctcaattggtatagtgattaaaatcacctagaccaattgagatgtatgtctgaattagttgttttcaaagcaaatgaactagcgattagtcgctatgacttaacggagcatgaaaccaagctaattttatgctgtgtggcactactcaaccccacgattgaaaaccctacaaggaaagaacggacggtatcgttcacttataaccaatacgctcagatgatgaacatcagtagggaaaatgcttatggtgtattagctaaagcaaccagagagctgatgacgagaactgtggaaatcaggaatcctttggttaaaggctttgagattttccagtggacaaactatgccaagttctcaagcgaaaaattagaattagtttttagtgaagagatattgccttatcttttccagttaaaaaaattcataaaatataatctggaacatgttaagtcttttgaaaacaaatactctatgaggatttatgagtggttattaaaagaactaacacaaaagaaaactcacaaggcaaatatagagattagccttgatgaatttaagttcatgttaatgcttgaaaataactaccatgagtttaaaaggcttaaccaatgggttttgaaaccaataagtaaagatttaaacacttacagcaatatgaaattggtggttgataagcgaggccgcccgactgatacgttgattttccaagttgaactagatagacaaatggatctcgtaaccgaacttgagaacaaccagataaaaatgaatggtgacaaaataccaacaaccattacatcagattcctacctacgtaacggactaagaaaaacactacacgatgctttaactgcaaaaattcagctcaccagttttgaggcaaaatttttgagtgacatgcaaagtaagcatgatctcaatggttcgttctcatggctcacgcaaaaacaacgaaccacactagagaacatactggctaaatacggaaggatctgaggttcttatggcccggcgtagcccaaaacgcgctgtcgtcaagtcgttaagggcgtgcccttcatcatccgatctggagtcaaaatgtcctcacgtaaagagcttgccaatgctattcgtgcgctgagcatggacgcagtacagaaagccaaatccggtcacccgggtgcccctatgggtatggctgacattgccgaagtcctgtggcgtgatttcctgaaacacaacccgcagaatccgtcctgggctgaccgtgaccgcttcgtgctgtccaacggccacggctccatgctgatctacagcctgctgcacctcaccggttacgatctgccgatggaagaactgaaaaacttccgtcagctgcactctaaaactccgggccacccggaagtaggttataccgctggtgtggaaaccaccaccggtccgctgggtcagggtattgccaacgcagtcggtatggcgattgcagaaaaaacgctggcggcgcagtttaaccgtccaggtcacgacattgtcgaccactacacctacgccttcatgggcgacggctgcatgatggaaggcatctcccacgaagtttgctctctggcgggtacgctgaagctgggtaaactgattgcgttctacgatgacaacggtatctcaatcgatggtcacgttgaaggctggttcactgacgacaccgcaatgcgtttcgaagcttacggctggcacgttattcgcgacatcgacggtcatgacgcggcatccatcaaacgcgcagtagaagaagcgcgcgcagtgactgacaaaccgtccctgctgatgtgcaaaaccatcatcggtttcggttccccgaacaaagccggtacccacgactcccacggtgcgccgctgggcgacgctgaaattgccctgacccgcgaacagctgggctggaaatacgcgccgttcgaaatcccgtctgaaatctatgctcagtgggatgcgaaagaagcaggccaggcgaaagaatctgcatggaatgagaagtttgcggcttacgcgaaagcttatccgcaggaagcggctgaatttacccgccgtatgaaaggcgaaatgccgtctgacttcgacgccaaagcgaaagagtttatcgctaaactgcaggctaatccggcgaaaatcgccagccgtaaagcgtcgcagaatgctatcgaagcgttcggcccgctgttgcctgaattcctcggcggctctgctgacctggcaccgtctaacctgaccctgtggtctggttctaaagcaatcaacgaagatgctgcaggtaactacatccactacggtgttcgcgagttcggtatgaccgcgattgctaacggtatctccctgcacggtggtttcctgccgtacacctccaccttcctgatgttcgtggaatacgcacgtaacgccgtacgtatggctgcgctgatgaaacagcgtcaggtgatggtttacacccacgactccatcggtctgggcgaagatggcccgactcaccagccggttgagcaggtcgcttctctgcgcgtgaccccgaacatgtctacatggcgtccgtgtgaccaggttgaatccgcggtcgcgtggaaatacggcgttgagcgtcaggacggcccgactgcgcttatcctctcccgtcagaacctggcgcagcaggaacgaactgaagagcaactggcaaacatcgcgcgcggtggttatgtgctgaaagactgcgccggtcagccggaactgattttcatcgctaccggttcagaagttgaactggctgttgctgcctacgaaaaactgactgccgaaggcgtgaaagcgcgcgtggtgtccatgccgtctaccgacgcatttgacaagcaggatgctgcttaccgtgaatccgtactgccgaaagcggttactgcacgcgttgctgtagaagcgggtattgctgactactggtacaagtatgttggcctgaacggtgctatcgtcggtatgaccaccttcggtgaatctgctccggcagagctgctgtttgaagagttcggcttcactgttgataacgttgttgcgaaagcaaaagaactgctgtaattagcatttcgggtaaaaaggtcgcttcggcgaccttttttattaccttgatatgtccgtttgcggacaagcaatagataaagcgtgttgtagatcacaaatatttatatgcaataaatatcaattatgtaatatgcatcacgatatgcgtattgacatttgttgttataactataactcaatgttatataagaaattaactcgaggctattgacgacagctatggttcactgtccaccaaccaaaactgtgctcagtaccgccaatatttctcccttgaggggtacaaagaggtgtccctagaagagatccacgctgtgtaaaaattttacaaaaaggtattgactttccctacagggtgtgtaataatttaattacaggcgggggcaaccccgcctgttctagaggaggaggaatcgccatggagaggattgtcgttactctcggggaacgtagttacccaattaccatcgcatctggtttgtttaatgaaccagcttcattcttaccgctgaaatcgggcgagcaggtcatgttggtcaccaacgaaaccctggctcctctgtatctcgataaggtccgcggcgtacttgaacaggcgggtgttaacgtcgatagcgttatcctccctgacggcgagcagtataaaagcctggctgtactcgataccgtctttacggcgttgttacaaaagccgcatggtcgcgatactacgctggtggcgcttggcggcggcgtagtgggcgatctgaccggcttcgcggcggcgagttatcagcgcggtgttcgtttcattcaagtcccgacgacgttactgtcgcaggtcgattcctccgttggcggcaaaactgcggtcaaccatcccctcggtaaaaacatgattggcgcgttctaccagcctgcttcagtggtggtggatctcgactgtctgaaaacgcttcccccgcgtgagttagcgtcggggctggcagaagtcatcaaatacggcattattcttgacggtgcgtttttcaactggctggaagagaatctggatgcgttgttgcgtctggacggtccggcaatggcgtactgtattcgccgttgttgtgaactgaaggcagaagttgtcgccgccgacgagcgcgaaaccgggttacgtgctttactgaatctgggacacacctttggtcatgccattgaagctgaaatggggtatggcaattggttacatggtgaagcggtcgctgcgggtatggtgatggcggcgcggacgtcggaacgtctcgggcagtttagttctgccgaaacgcagcgtattataaccctgctcacgcgggctgggttaccggtcaatgggccgcgcgaaatgtccgcgcaggcgtatttaccgcatatgctgcgtgacaagaaagtccttgcgggagagatgcgcttaattcttccgttggcaattggtaagagtgaagttcgcagcggcgtttcgcacgagcttgttcttaacgccattgccgattgtcaatcagcgtaatcatcgttcatgcctgatgccgctatgtaggccggataaggcgttcacgccgcatccggcaaccgatgcctgatgcgacgcggtcgcgtcttatcaggcctacaggtcgatgccgatatgtacatcgtattcggcaattaatacatagcactcgaggcctacctagcttccaagaaagatatcctaacagcacaagagcggaaagatgttttgttctacatccagaacaacctctgctaaaattcctgaaaaattttgcaaaaagttgttgactttatctacaaggtgtggtataataatcttaacaacagcaggacgctctagaatgaaaaccgtaactgtaaaagatctcgtcattggtacgggcgcacctaaaatcatcgtctcgctgatggcgaaagatatcgccagcgtgaaatccgaagctctcgcctatcgtgaagcggactttgatattctggaatggcgtgtggaccactatgccgacctctccaatgtggagtctgtcatggcggcagcaaaaattctccgtgagaccatgccagaaaaaccgctgctgtttaccttccgcagtgccaaagaaggcggcgagcaggcgatttccaccgaggcttatattgcactcaatcgtgcagccatcgacagcggcctggttgatatgatcgatctggagttatttaccggtgatgatcaggttaaagaaaccgtcgcctacgcccacgcgcatgatgtgaaagtagtcatgtccaaccatgacttccataaaacgccggaagccgaagaaatcattgcccgtctgcgcaaaatgcaatccttcgacgccgatattcctaagattgcgctgatgccgcaaagtaccagcgatgtgctgacgttgcttgccgcgaccctggagatgcaggagcagtatgccgatcgtccaattatcacgatgtcgatggcaaaaactggcgtaatttctcgtctggctggtgaagtatttggctcggcggcaacttttggtgcggtaaaaaaagcgtctgcgccagggcaaatctcggtaaatgatttgcgcacggtattaactattttacaccaggcataagcaataatatttcggcgggaacaccctccccgccgaactaaaaaatatattcaatcgtatttaataaaaatatttcgtgagtctctgtgcgctaattctc

SEQ ID NO: 58 - DNA, 5500 bp, Escherichia coli
  gene (1)..(5500): Nucleotide sequence of  ppc::PR-pyc
cgaaccgacgtcactacaaccggtacgcgcacataaaggtcatatctctaacgccatccgtattcagggccagtcggggcactccagcgatccagcacgcggagttaacgctatcgaactaatgcacgacgccatcgggcatattttgcaattgcgcgataacctgaaagaacgttatcactacgaagcgtttaccgtgccataccctacgctcaacctcgggcatattcacggtggcgacgcttctaaccgtatttgcgcttgctgtgagttgcatatggatattcgtccgctgcctggcatgacactcaatgaacttaatggtttgctcaacgatgcattggctccggtgagcgaacgctggccgggtcgtctgacggtcgacgagctgcatccgccgatccctggctatgaatgcccaccgaatcatcaactggttgaagtggttgagaaattgctcggagcaaaaaccgaagtggtgaactactgtaccgaagcgccgtttattcaaacgttatgcccgacgctggtgttggggcctggctcaattaatcaggctcatcaacctgatgaatatctggaaacacggtttatcaagcccacccgcgaactgataacccaggtaattcaccatttttgctggcattaaaacgtaggccggataaggcgctcgcgccgcatccggcactgttgccaaactccagtgccgcaataatgtcggatgcgatacttgcgcatcttatccgacctacacctttggtgttacttggggcgattttttaacatttccataagttacgcttatttaaagcgtcgtgaatttaatgacgtaaattcctgctatttattcgttcgttaaatctatcaccgcaagggataaatatctaacaccgtgcgtgttgactattttacctctggcggtgataatggttgcatgtactaatctagataaggaatatagccatgtcgcaaagaaaattcgccggcttgagagataacttcaatctcttgggtgaaaagaacaaaatattggtggctaatagaggagaaattccaatcagaatttttcgtaccgctcatgaactgtctatgcagacggtagctatatattctcatgaagatcgtctttcaacgcacaaacaaaaggctgacgaagcatacgtcataggtgaagtaggccaatatacccccgtcggcgcttatttggccattgacgaaatcatttccattgcccaaaaacaccaggtagatttcatccatccaggttatgggttcttgtctgaaaattcggaatttgccgacaaagtagtgaaggccggtatcacttggattggccctccagctgaagttattgactccgtgggtgataaggtctcagctagaaacctggcagcaaaagctaatgtgcccaccgttcctggtacaccaggtcctatagaaactgtagaggaagcacttgacttcgtcaatgaatacggctacccggtgatcattaaggccgcctttggtggtggtggtagaggtatgagagtcgttagagaaggtgacgacgtggcagatgcctttcaacgtgctacctccgaagcccgtactgccttcggtaatggtacctgctttgtggaaagattcttggacaagccaaagcatattgaagttcaattgttggccgataaccacggaaacgtggttcatcttttcgaaagagactgttccgtgcagagaagacaccaaaaggttgtcgaagtggccccagcaaagactttaccccgtgaagtccgtgacgccattttgacagatgcagttaaattggccaaagagtgtggctacagaaatgcgggtactgctgaattcttggttgataaccaaaatagacactatttcattgaaattaatccaagaatccaagtggaacataccatcacagaagaaattaccggtatagatattgtggcggctcagatccaaattgcggcaggtgcctctctaccccagctgggcctattccaggacaaaattacgactcgtggctttgccattcagtgccgtattaccacggaagaccctgctaagaacttccaaccagataccggtagaatagaagtgtaccgttctgcaggtggtaatggtgttagactggatggtggtaacgcctatgcaggaacaataatctcacctcattacgactcaatgctggtcaaatgctcatgctccggttccacctacgaaatcgttcgtagaaaaatgattcgtgcattaatcgagttcagaattagaggtgtcaagaccaacattcccttcctattgactcttttgaccaatccagtatttattgagggtacatactggacgacttttattgacgacaccccacaactgttccaaatggtttcatcacaaaacagagcccaaaaacttttacattacctcgccgacgtggcagtcaatggttcatctatcaagggtcaaattggcttgccaaaattaaaatcaaatccaagtgtcccccatttgcacgatgctcagggcaatgtcatcaacgttacaaagtctgcaccaccatccggatggaggcaagtgctactagaaaaggggccagctgaatttgccagacaagttagacagttcaatggtactttattgatggacaccacctggagagacgctcatcaatctctacttgcaacaagagtcagaacccacgatttggctacaatcgctccaacaaccgcacatgcccttgcaggtcgtttcgccttagaatgttggggtggtgccacattcgatgttgcaatgagatttttgcatgaggatccatgggaacgtttgagaaaattaagatctctggtgcctaatattccattccaaatgttattgcgtggtgccaatggtgtggcttattcttcattgcctgacaatgctattgaccatttcgtcaagcaagccaaggataatggtgttgatatatttagagtctttgatgccttaaatgacttggaacaattgaaggtcggtgtagatgctgtgaagaaggcaggtggtgttgtagaagccactgtttgtttctctggggatatgcttcagccaggcaagaaatacaatttggattactacttggaaattgctgaaaaaattgtccaaatgggcactcatatcctgggtatcaaagatatggcaggtaccatgaagccagcagctgccaaactactgattggatctttgagggctaagtaccctgatctcccaatacatgttcacactcacgattctgcaggtactgctgttgcatcaatgactgcgtgtgctctggcgggcgccgatgtcgttgatgttgccatcaactcaatgtctggtttaacttcacaaccatcaatcaatgctctgttggcttcattagaaggtaatattgacactggtattaacgttgagcatgtccgtgaactagatgcatattgggcagagatgagattgttatactcttgtttcgaggctgacttgaagggcccagatccagaagtttatcaacatgaaatcccaggtggtcaattgacaaacttgttgtttcaagcccaacaattgggtcttggagaacaatgggccgaaacaaaaagagcttacagagaagccaattatttattgggtgatattgtcaaagttaccccaacttcgaaggtcgttggtgatctggcacaatttatggtctccaataaattaacttccgatgatgtgagacgcctggctaattctttggatttccctgactctgttatggatttcttcgaaggcttaatcggccaaccatatggtgggttcccagaaccatttagatcagacgttttaaggaacaagagaagaaagttgacttgtcgtccaggcctggaactagagccatttgatctcgaaaaaattagagaagacttgcagaatagatttggtgatgttgatgagtgcgacgttgcttcttataacatgtacccaagagtttatgaagacttccaaaagatgagagaaacgtatggtgatttatctgtattgccaacaagaagctttttgtctccactagagactgacgaagaaattgaagttgtaatcgaacaaggtaaaacgctaattatcaagctacaggctgtgggtgatttgaacaaaaagaccggtgaaagagaagtttactttgatttgaatggtgaaatgagaaaaattcgtgttgctgacagatcacaaaaagtggaaactgttactaaatccaaagcagacatgcatgatccattacacattggtgcaccaatggcaggtgtcattgttgaagttaaagttcataaaggatcactaataaagaagggccaacctgtagccgtattaagcgccatgaaaatggaaatgattatatcttctccatccgatggacaagttaaagaagtgtttgtctctgatggtgaaaatgtggactcttctgatttattagttctattagaagaccaagttcctgttgaaactaaggcatgatcttcctcttctgcaaaccctcgtgcttttgcgcgagggttttctgaaatacttctgttctaacaccctcgttttcaatatatttctgtctgcattttattcaaattctgaatataccttcagatatccttaaggaattgtcgttacattcggcgatattttttcaagacaggttcttactatgcattccacagaagtccaggctaaacctctttttagctggaaagccctgggttgggcactgctctacttttggtttttctctactctgctacaggccattatttacatcagtggttatagtggcactaacggcattcgcgactcgctgttattcagttcgctgtggttgatcccggtattcctctttccgaagcggattaaaattattgccgcagtaatcggcgtggtgctatgggcggcctctctggcggcgctgtgctactacgtcatctacggtcaggagttctcgcagagcgttctgtttgtgatgttcgaaaccaacaccaacgaagccagcgagtatttaagccagtatttcagcctgaaaattgtgcttatcgcgctggcctatacggcggtggcagttctgctgtggacacgcctgcgcccggtctatattccaaagccgtggcgttatgttgtctcttttgccctgctttatggcttgattctgcatccgatcgccatgaatacgtttatcaaaaacaagccgtttgagaaaacgttggataacctggcctcgcgtatggagcctgccgcaccgtggcaattcctgaccggctattatcagtatcgtcagcaactaaactcgctaacaaagttactgaatgaaaataatgccttgccgccactggctaatttcaaagatgaatcgggtaacgaaccgcgcactttagtgctggtgattggcgagtcgacccagcgcggacgcatgagtctgtacggttatccgcgtgaaaccacgccggagctggatgcgctgcataaaaccgatccg

SEQ ID NO: 59 - DNA, 200 bp, Escherichia coli
  promoter (1)..(200): Nucleotide sequence of acpP promoter
cacaaaatgctcatgttgcgcgcagtctgcgtggttatgagtaataattagtgcaaaatgatttgcgttattggggggtaaggcctcaaaataacgtaaaatcgtggtaagacctgccgggatttagttgcaaatttttcaacattttatacactacgaaaaccatcgcgaaagcgagttttgataggaaatttaagagt

SEQ ID NO: 60 - DNA, 200 bp, Escherichia coli
  promoter (1)..(200): Nuclotide sequence of rplU promoter
ttatggttaggaatatagggtgattgtactgaaaaaatggcacagataaacgttaccgtacaagttgtgttttttttcttcgtgtattgactgtagcacttgtcaaaggcgtgcgttttgcgtaatattcgcgccctattgtgaatatttatagcgcactctgaatcattgaaaaggtgtgcgcggaagcggagttttat

SEQ ID NO: 61 - DNA, 60 bp, Artificial Sequence
  Primer
  primer_bind (1)..(60): Sequence of DNA primer MS604
aacgccgtataatgggcgcagattaagaggctacagtgggcttacatggcgatagctaga

SEQ ID NO: 62 - DNA, 60 bp, Artificial Sequence
  Primer
  primer_bind (1)..(60): Sequence of DNA Primer MS605
tgtcggatcgataaatagggcaaaacaaacgcgcatcccggaaaacgattccgaagccca

SEQ ID NO: 63 - DNA, 60 bp, Artificial Sequence
  Primer
  primer_bind (1)..(60): Sequence of DNA Primer MS608
aaagtctgcctgcaagtctgacagggcaactatttgtgggcttacatggcgatagctaga

SEQ ID NO: 64 - DNA, 60 bp, Artificial Sequence
  Primer
  primer_bind (1)..(60): Sequence of DNA Primer MS609
ttgcaaaattgccctgaaacagggcaacagcggagtcccggaaaacgattccgaagccca

SEQ ID NO: 65 - DNA, 25 bp, Artificial Sequence
  Primer
  primer_bind (1)..(25): Sequence of DNA Primer MS461
ggctatattccttatctagattagt

SEQ ID NO: 66 - DNA, 25 bp, Artificial Sequence
  Primer
  primer_bind (1)..(25): Sequence of DNA Primer MS346
gtctgacaggtgccggatttcatat

SEQ ID NO: 67 - DNA, 45 bp, Artificial Sequence
  Primer
  primer_bind (1)..(45): Sequence of DNA Primer RP712
tctagataaggaatatagccatgaccgcaccgattcaggatctgc

SEQ ID NO: 68 - DNA, 45 bp, Artificial Sequence
  Primer
  primer_bind (1)..(45): Sequence of DNA Primer RP714
aaatccggcacctgtcagacttattttgcgctaccctggtttttt

SEQ ID NO: 69 - DNA, 60 bp, Artificial Sequence
  Primer
  primer_bind (1)..(60): Sequence of DNA Primer RP731
catgtactaatctagataaggaatatagccatgaaactgattattgggatgacgggggcc

SEQ ID NO: 70 - DNA, 60 bp, Artificial Sequence
  Primer
  primer_bind (1)..(60): Sequence of DNA Primer RP732
gccggatatgaaatccggcacctgtcagacttattcgatctcctgtgcaaattgttctgc

SEQ ID NO: 71 - DNA, 45 bp, Artificial Sequence
  Primer
  primer_bind (1)..(45): Sequenc of DNA Primer MS669
tctagataaggaatatagccatgaaacgactcattgtaggcatca

SEQ ID NO: 72 - DNA, 45 bp, Artificial Sequence
  Primer
  primer_bind (1)..(45): Sequence of DNA Primer MS666
accgaacaggcttatgtccagatagcaggtatagcggttgaatcg

SEQ ID NO: 73 - DNA, 24 bp, Artificial Sequence
  Primer
  primer_bind (1)..(24): Sequence of DNA Primer RP607
tggacataagcctgttcggttcgt

SEQ ID NO: 74 - DNA, 25 bp, Artificial Sequence
  Primer
  primer_bind (1)..(25): Sequence of DNA Primer RP621
ttagatttgactgaaatcgtacagt

SEQ ID NO: 75 - DNA, 45 bp, Artificial Sequence
  Primer
  primer_bind (1)..(45): Sequence of DNA Primer MS676
tctagataaggaatatagccatgaaactgatcgtcgggatgacag

SEQ ID NO: 76 - DNA, 45 bp, Artificial Sequence
  Primer
  primer_bind (1)..(45): Sequence of DNA Primer MS680
acgatttcagtcaaatctaattattcattctcctgagaaaaattc

SEQ ID NO: 77 - DNA, 45 bp, Artificial Sequence
  Primer
  primer_bind (1)..(45): Sequence of DNA Primer MS686
tctagataaggaatatagccatgacggcacgcatcatcattggta

SEQ ID NO: 78 - DNA, 45 bp, Artificial Sequence
  Primer
  primer_bind (1)..(45): Sequence of DNA Primer MS684
acgatttcagtcaaatctaattaattaaaacgtagctcgccttca

SEQ ID NO: 79 - DNA, 45 bp, Artificial Sequence
  Primer
  primer_bind (1)..(45): Sequence of DNA Primer MS692
tctagataaggaatatagccatgaaacgaattgttgtgggaatca

SEQ ID NO: 80 - DNA, 45 bp, Artificial Sequence
  Primer
  primer_bind (1)..(45): Sequence of DNA Primer MS691
acgatttcagtcaaatctaattaatccccctcccaacggcgatca

SEQ ID NO: 81 - DNA, 45 bp, Artificial Sequence; identical to SEQ ID NO: 80
  Primer
  primer_bind (1)..(45): Sequence of DNA Primer RP677

SEQ ID NO: 82 - DNA, 25 bp, Artificial Sequence
  Primer
  primer_bind (1)..(25): Sequence of DNA Primer RP671
ttaatcgccttgcagcacatccccc

SEQ ID NO: 83 - DNA, 24 bp, Artificial Sequence
  Primer
  primer_bind (1)..(24): Sequenc of DNA primer RP664
acgaaccgaacaggcttatgtcca

SEQ ID NO: 84 - DNA, 45 bp, Artificial Sequence
  Primer
  primer_bind (1)..(45): Sequence of DNA Primer RP702
gccgtcgttttacaacgtcggatccgcctacctagcttccaagaa

SEQ ID NO: 85 - DNA, 45 bp, Artificial Sequence
  Primer
  primer_bind (1)..(45): Sequence of DNA Primer RP783
cctacaatgagtcgtttcattaggttttcctcaacccgggagcgt

SEQ ID NO: 86 - DNA, 45 bp, Artificial Sequence
  Primer
  primer_bind (1)..(45): Sequence of DNA primer RP781
cccgggttgaggaaaacctaatgaaacgactcattgtaggcatca

SEQ ID NO: 87 - DNA, 45 bp, Artificial Sequence
  Primer
  primer_bind (1)..(45): Sequence of DNA Primer 780
atgtgctgcaaggcgattaagatagcaggtatagcggttgaatcg

SEQ ID NO: 88 - DNA, 45 bp, Artificial Sequence
  Primer
  primer_bind (1)..(45): Sequence of DNA Primer RP700
gccgtcgttttacaacgtcgagcggggcggttgtcaacgatgggg

SEQ ID NO: 89 - DNA, 45 bp, Artificial Sequence
  Primer
  misc_feature (1)..(45): Sequence of DNA Primer RP784
cctacaatgagtcgtttcatggctatattcctcctctgcatgaga

SEQ ID NO: 90 - DNA, 45 bp, Artificial Sequence
  Primer
  primer_bind (1)..(45): Sequenc of DNA Primer RP779
tgcagaggaggaatatagccatgaaacgactcattgtaggcatca

SEQ ID NO: 91 - DNA, 45 bp, Artificial Sequence
  Primer
  primer_bind (1)..(45): Sequence of DNA Primer MS1383
gatggggtgtctggggtaatatgtcgcaaagaaaattcgccggct

SEQ ID NO: 92 - DNA, 45 bp, Artificial Sequence
  Primer
  primer_bind (1)..(45): Sequence of DNA Primer MS1384
gggtttgcagaagaggaagatcatgccttagtttcaacaggaact

SEQ ID NO: 93 - DNA, 45 bp, Artificial Sequence
  Primer
  primer_bind (1)..(45): Sequence of DNA Primer MS1429
attcctgctatttattcgttcgttaaatctatcaccgcaagggat

SEQ ID NO: 94 - DNA, 45 bp, Artificial Sequence
  Primer
  primer_bind (1)..(45): Sequence of DNA Primer MS1430
gcgaattttctttgcgacatggctatattccttatctagattagt